European Patent Specification EP 3 738 971 B1, published July 17, 2024. Title: GENETICALLY ENCODED FLUORESCENT SENSORS FOR DETECTING LIGAND BIAS AND INTRACELLULAR SIGNALING THROUGH cAMP PATHWAYS. Applicant: Hughes, Thomas E. Tewson, Paul H. Quinn, Anne Marie. Application not yet assigned. The sequence listing filed with the application follows.

SEQUENCE LISTING (77 sequences)

SEQ ID NO: 1 - protein, 739 aa, Artificial Sequence
  Synthetic
MGSNNDRIPDKENTPLIEPHVPLRPANTITKVPSEKILRAGKILRNAILSRAPHMIRDRKYHLKTYRQCCVGTELVDWMMQQTPCVHSRTQAVGMWQVLLEDGVLNHVDQEHHFQDKYLFYRFLDDEHEDAPLPTEEEKKECDEELQDTMLLLSQMGPDAHMRMILRKPPGQRTVDDLEIIYEELLHIKALSHLSTTVKRELAGVLIFESHAKGGTVLFNQGEEGTSWYIILKGSVNVVIYGKGVVCTLHEGDDFGKLALVNDAPRAASIVLREDNCHFLRVDKEDFNRILRLVSHNVYIKADKQKNGIKANFKIRHNIEDGGVQLAYHYQQNTPIGDGPVLLPDNHYLSVQSILSKDPNEKRDHMVLLEFVTAAGITLGMDELYKGGTGGSMVSKGEELFTGVVPIQVELDGDVNGHKFSVSGEGEGDATYGKLTLKFICTTGKLPVPWPTLVTTLTYGVQCFSRYPDHMKQHDFFKSAMPEGYIQERTIFFKDDGNYKTRAEVKFEGDTLVNRIELKGIDFKEDGNILGHKLEYNFNNPDVEANTVRLKEHDQDVLVLEKVPAGNRASNQGNSQPQQKYTVMSGTPEKILEHFLETIRLEATLNEATDSVLNDFIMMHCVFMPNTQLCPALVAHYHAQPSQGTEQEKMDYALNNKRRVIRLVLQWAAMYGDLLQEDDVSMAFLEEFYVSVSDDARMIAALKEQLPELEKIVKQISEDAKAPQKKHKVLLQQFNTGDE

SEQ ID NO: 2 - protein, 1269 aa, Artificial Sequence
  Synthetic
MVAAHAAHSSSSAEWIACLDKRPLERSSEDVDIIFTRLKEVKAFEKFHPNLLHQICLCGYYENLEKGITLFRQGDIGTNWYAVLAGSLDVKVSETSSHQDAVTICTLGIGTAFGESILDNTPRHATIVTRESSELLRIEQKDFKALWEKYRQYMAGLLAPPYGVMETGSNNDRIPDKENTPLIEPHVPLRPANTITKVPSEKILRAGKILRNAILSRAPHMIRDRKYHLKTYRQCCVGTELVDWMMQQTPCVHSRTQAVGMWQVLLEDGVLNHVDQEHHFQDKYLFYRFLDDEHEDAPLPTEEEKKECDEELQDTMLLLSQMGPDAHMRMILRKPPGQRTVDDLEIIYEELLHIKALSHLSTTVKRELAGVLIFESHAKGGTVLFNQGEEGTSWYIILKGSVNVVIYGKGVVCTLHEGDDFGKLALVNDAPRAASIVLREDNCHFLRVDKEDFNRILRDVEALENVYIKADKQKNGIKANFKIRHNIEDGGVQLAYHYQQNTPIGDGPVLLPDNHYLSVQSILSKDPNEKRDHMVLLEFVTAAGITLGMDELYKGGTGGSMVSKGEELFTGVVPIQVELDGDVNGHKFSVSGEGEGDATYGKLTLKFICTTGKLPVPWPTLVTTLTYGVQCFSRYPDHMKQHDFFKSAMPEGYIQERTIFFKDDGNYKTRAEVKFEGDTLVNRIELKGIDFKEDGNILGHKLEYNTRKEDFNRILRDVEANTVRLKEHDQDVLVLEKVPAGNRASNQGNSQPQQKYTVMSGTPEKILEHFLETIRLEATLNEATDSVLNDFIMMHCVFMPNTQLCPALVAHYHAQPSQGTEQEKMDYALNNKRRVIRLVLQWAAMYGDLLQEDDVSMAFLEEFYVSVSDDARMIAALKEQLPELEKIVKQISEDAKAPQKKHKVLLQQFNTGDERAQKRQPIRGSDEVLFKVYCMDPTYTTIRVPVATSVKEVISAVADKLGSGEGLIIVKMSSGGEKVVLKPNDVSVFMTLTINGRLFACPREQFDSLTPLPEQEGPTVGTVGTFELMSSKDLAYQMTIYDWELFNCVHELELIYHTFGRHNFKKTTANLDLFLRRFNEIQFWVVTEICLCSQLSKRVQLLKKFIKIAAHCKEYKNLNSFFAIVMGLSNVAVSRLALTWEKLPSKFKKFYAEFESLMDPSRNHRAYRLTVAKLEPPLIPFMPLLIKDMTFTHEGNKTFIDNLVNFEKMRMIANTARTVRYYRSQPFNPDAAQANKNHQDVRSYVRQLNVIDNQRTLSQMSHRLEPRRP

SEQ ID NO: 3 - protein, 748 aa, Artificial Sequence
  Synthetic
MGSNNDRIPDKENTPLIEPHVPLRPANTITKVPSEKILRAGKILRNAILSRAPHMIRDRKYHLKTYRQCCVGTELVDWMMQQTPCVHSRTQAVGMWQVLLEDGVLNHVDQEHHFQDKYLFYRFLDDEHEDAPLPTEEEKKECDEELQDTMLLLSQMGPDAHMRMILRKPPGQRTVDDLEIIYEELLHIKALSHLSTTVKRELAGVLIFESHAKGGTVLFNQGEEGTSWYIILKGSVNVVIYGKGVVCTLHEGDDFGKLALVNDAPRAASIVLREDNCHFLRVDKEDFNRILRDVEALENVYIKADKQKNGIKANFKIRHNIEDGGVQLAYHYQQNTPIGDGPVLLPDNHYLSVQSILSKDPNEKRDHMVLLEFVTAAGITLGMDELYKGGTGGSMVSKGEELFTGVVPIQVELDGDVNGHKFSVSGEGEGDATYGKLTLKFICTTGKLPVPWPTLVTTLTYGVQCFSRYPDHMKQHDFFKSAMPEGYIQERTIFFKDDGNYKTRAEVKFEGDTLVNRIELKGIDFKEDGNILGHKLEYNTRKEDFNRILRDVEANTVRLKEHDQDVLVLEKVPAGNRASNQGNSQPQQKYTVMSGTPEKILEHFLETIRLEATLNEATDSVLNDFIMMHCVFMPNTQLCPALVAHYHAQPSQGTEQEKMDYALNNKRRVIRLVLQWAAMYGDLLQEDDVSMAFLEEFYVSVSDDARMIAALKEQLPELEKIVKQISEDAKAPQKKHKVLLQQFNTGDE

SEQ ID NO: 4 - protein, 1260 aa, Artificial Sequence
  Synthetic
MVAAHAAHSSSSAEWIACLDKRPLERSSEDVDIIFTRLKEVKAFEKFHPNLLHQICLCGYYENLEKGITLFRQGDIGTNWYAVLAGSLDVKVSETSSHQDAVTICTLGIGTAFGESILDNTPRHATIVTRESSELLRIEQKDFKALWEKYRQYMAGLLAPPYGVMETGSNNDRIPDKENTPLIEPHVPLRPANTITKVPSEKILRAGKILRNAILSRAPHMIRDRKYHLKTYRQCCVGTELVDWMMQQTPCVHSRTQAVGMWQVLLEDGVLNHVDQEHHFQDKYLFYRFLDDEHEDAPLPTEEEKKECDEELQDTMLLLSQMGPDAHMRMILRKPPGQRTVDDLEIIYEELLHIKALSHLSTTVKRELAGVLIFESHAKGGTVLFNQGEEGTSWYIILKGSVNVVIYGKGVVCTLHEGDDFGKLALVNDAPRAASIVLREDNCHFLRVDKEDFNRILRLVSHNVYIKADKQKNGIKANFKIRHNIEDGGVQLAYHYQQNTPIGDGPVLLPDNHYLSVQSILSKDPNEKRDHMVLLEFVTAAGITLGMDELYKGGTGGSMVSKGEELFTGVVPIQVELDGDVNGHKFSVSGEGEGDATYGKLTLKFICTTGKLPVPWPTLVTTLTYGVQCFSRYPDHMKQHDFFKSAMPEGYIQERTIFFKDDGNYKTRAEVKFEGDTLVNRIELKGIDFKEDGNILGHKLEYNFNNPDVEANTVRLKEHDQDVLVLEKVPAGNRASNQGNSQPQQKYTVMSGTPEKILEHFLETIRLEATLNEATDSVLNDFIMMHCVFMPNTQLCPALVAHYHAQPSQGTEQEKMDYALNNKRRVIRLVLQWAAMYGDLLQEDDVSMAFLEEFYVSVSDDARMIAALKEQLPELEKIVKQISEDAKAPQKKHKVLLQQFNTGDERAQKRQPIRGSDEVLFKVYCMDPTYTTIRVPVATSVKEVISAVADKLGSGEGLIIVKMSSGGEKVVLKPNDVSVFMTLTINGRLFACPREQFDSLTPLPEQEGPTVGTVGTFELMSSKDLAYQMTIYDWELFNCVHELELIYHTFGRHNFKKTTANLDLFLRRFNEIQFWVVTEICLCSQLSKRVQLLKKFIKIAAHCKEYKNLNSFFAIVMGLSNVAVSRLALTWEKLPSKFKKFYAEFESLMDPSRNHRAYRLTVAKLEPPLIPFMPLLIKDMTFTHEGNKTFIDNLVNFEKMRMIANTARTVRYYRSQPFNPDAAQANKNHQDVRSYVRQLNVIDNQRTLSQMSHRLEPRRP

SEQ ID NO: 5 - protein, 1256 aa, Artificial Sequence
  Synthetic
MVAAHAAHSSSSAEWIACLDKRPLERSSEDVDIIFTRLKEVKAFEKFHPNLLHQICLCGYYENLEKGITLFRQGDIGTNWYAVLAGSLDVKVSETSSHQDAVTICTLGIGTAFGESILDNTPRHATIVTRESSELLRIEQKDFKALWEKYRQYMAGLLAPPYGVMETGSNNDRIPDKENTPLIEPHVPLRPANTITKVPSEKILRAGKILRNAILSRAPHMIRDRKYHLKTYRQCCVGTELVDWMMQQTPCVHSRTQAVGMWQVLLEDGVLNHVDQEHHFQDKYLFYRFLDDEHEDAPLPTEEEKKECDEELQDTMLLLSQMGPDAHMRMILRKPPGQRTVDDLEIIYEELLHIKALSHLSTTVKRELAGVLIFESHAKGGTVLFNQGEEGTSWYIILKGSVNVVIYGKGVVCTLHEGDDFGKLALVNDAPRAASIVLREDNCHFLRVDKEDFNRILRDVLENVYIKADKQKNGIKANFKIRHNIEDGGVQLAYHYQQNTPIGDGPVLLPDNHYLSVQSILSKDPNEKRDHMVLLEFVTAAGITLGMDELYKGGTGGSMVSKGEELFTGVVPIQVELDGDVNGHKFSVSGEGEGDATYGKLTLKFICTTGKLPVPWPTLVTTLTYGVQCFSRYPDHMKQHDFFKSAMPEGYIQERTIFFKDDGNYKTRAEVKFEGDTLVNRIELKGIDFKEDGNILGHKLEYNTREANTVRLKEHDQDVLVLEKVPAGNRASNQGNSQPQQKYTVMSGTPEKILEHFLETIRLEATLNEATDSVLNDFIMMHCVFMPNTQLCPALVAHYHAQPSQGTEQEKMDYALNNKRRVIRLVLQWAAMYGDLLQEDDVSMAFLEEFYVSVSDDARMIAALKEQLPELEKIVKQISEDAKAPQKKHKVLLQQFNTGDERAQKRQPIRGSDEVLFKVYCMDPTYTTIRVPVATSVKEVISAVADKLGSGEGLIIVKMSSGGEKVVLKPNDVSVFMTLTINGRLFACPREQFDSLTPLPEQEGPTVGTVGTFELMSSKDLAYQMTIYDWELFNCVHELELIYHTFGRHNFKKTTANLDLFLRRFNEIQFWVVTEICLCSQLSKRVQLLKKFIKIAAHCKEYKNLNSFFAIVMGLSNVAVSRLALTWEKLPSKFKKFYAEFESLMDPSRNHRAYRLTVAKLEPPLIPFMPLLIKDMTFTHEGNKTFIDNLVNFEKMRMIANTARTVRYYRSQPFNPDAAQANKNHQDVRSYVRQLNVIDNQRTLSQMSHRLEPRRP

SEQ ID NO: 6 - protein, 535 aa, Artificial Sequence
  Synthetic
MGSNNDRIPDKENTPLIEPHVPLRPANTITKVPSEKILRAGKILRNAILSRAPHMIRDRKYHLKTYRQCCVGTELVDWMMQQTPCVHSRTQAVGMWQVLLEDGVLNHVDQEHHFQDKYLFYRFLDDEHEDAPLPTEEEKKECDEELQDTMLLLSQMGPDAHMRMILRKPPGQRTVDDLEIIYEELLHIKALSHLSTTVKRELAGVLIFESHAKGGTVLFNQGEEGTSWYIILKGSVNVVIYGKGVVCTLHEGDDFGKLALVNDAPRAASIVLREDNCHFLRVDKEDFNRILRRANVYIKADKQKNGIKANFKIRHNIEDGGVQLAYHYQQNTPIGDGPVLLPDNHYLSVQSILSKDPNEKRDHMVLLEFVTAAGITLGMDELYKGGTGGSMVSKGEELFTGVVPIQVELDGDVNGHKFSVSGEGEGDATYGKLTLKFICTTGKLPVPWPTLVTTLTYGVQCFSRYPDHMKQHDFFKSAMPEGYIQERTIFFKDDGNYKTRAEVKFEGDTLVNRIELKGIDFKEDGNILGHKLEYN

SEQ ID NO: 7 - protein, 1265 aa, Artificial Sequence
  Synthetic
MVAAHAAHSSSSAEWIACLDKRPLERSSEDVDIIFTRLKEVKAFEKFHPNLLHQICLCGYYENLEKGITLFRQGDIGTNWYAVLAGSLDVKVSETSSHQDAVTICTLGIGTAFGESILDNTPRHATIVTRESSELLRIEQKDFKALWEKYRQYMAGLLAPPYGVMETGSNNDRIPDKENTPLIEPHVPLRPANTITKVPSEKILRAGKILRNAILSRAPHMIRDRKYHLKTYRQCCVGTELVDWMMQQTPCVHSRTQAVGMWQVLLEDGVLNHVDQEHHFQDKYLFYRFLDDEHEDAPLPTEEEKKECDEELQDTMLLLSQMGPDAHMRMILRKPPGQRTVDDLEIIYEELLHIKALSHLSTTVKRELAGVLIFESHAKGGTVLFNQGEEGTSWYIILKGSVNVVIYGKGVVCTLHEGDDFGKLALVNDAPRAASIVLREDNCHFLRVDKEDFNRILRLENVYIKADKQKNGIKANFKIRHNIEDGGVQLAYHYQQNTPIGDGPVLLPDNHYLSVQSILSKDPNEKRDHMVLLEFVTAAGITLGMDELYKGGTGGSMVSKGEELFTGVVPIQVELDGDVNGHKFSVSGEGEGDATYGKLTLKFICTTGKLPVPWPTLVTTLTYGVQCFSRYPDHMKQHDFFKSAMPEGYIQERTIFFKDDGNYKTRAEVKFEGDTLVNRIELKGIDFKEDGNILGHKLEYNTRKEDFNRILRDVEANTVRLKEHDQDVLVLEKVPAGNRASNQGNSQPQQKYTVMSGTPEKILEHFLETIRLEATLNEATDSVLNDFIMMHCVFMPNTQLCPALVAHYHAQPSQGTEQEKMDYALNNKRRVIRLVLQWAAMYGDLLQEDDVSMAFLEEFYVSVSDDARMIAALKEQLPELEKIVKQISEDAKAPQKKHKVLLQQFNTGDERAQKRQPIRGSDEVLFKVYCMDPTYTTIRVPVATSVKEVISAVADKLGSGEGLIIVKMSSGGEKVVLKPNDVSVFMTLTINGRLFACPREQFDSLTPLPEQEGPTVGTVGTFELMSSKDLAYQMTIYDWELFNCVHELELIYHTFGRHNFKKTTANLDLFLRRFNEIQFWVVTEICLCSQLSKRVQLLKKFIKIAAHCKEYKNLNSFFAIVMGLSNVAVSRLALTWEKLPSKFKKFYAEFESLMDPSRNHRAYRLTVAKLEPPLIPFMPLLIKDMTFTHEGNKTFIDNLVNFEKMRMIANTARTVRYYRSQPFNPDAAQANKNHQDVRSYVRQLNVIDNQRTLSQMSHRLEPRRP

SEQ ID NO: 8 - protein, 1257 aa, Artificial Sequence
  Synthetic
MVAAHAAHSSSSAEWIACLDKRPLERSSEDVDIIFTRLKEVKAFEKFHPNLLHQICLCGYYENLEKGITLFRQGDIGTNWYAVLAGSLDVKVSETSSHQDAVTICTLGIGTAFGESILDNTPRHATIVTRESSELLRIEQKDFKALWEKYRQYMAGLLAPPYGVMETGSNNDRIPDKENTPLIEPHVPLRPANTITKVPSEKILRAGKILRNAILSRAPHMIRDRKYHLKTYRQCCVGTELVDWMMQQTPCVHSRTQAVGMWQVLLEDGVLNHVDQEHHFQDKYLFYRFLDDEHEDAPLPTEEEKKECDEELQDTMLLLSQMGPDAHMRMILRKPPGQRTVDDLEIIYEELLHIKALSHLSTTVKRELAGVLIFESHAKGGTVLFNQGEEGTSWYIILKGSVNVVIYGKGVVCTLHEGDDFGKLALVNDAPRAASIVLREDNCHFLRVDKEDFNRILRDVLENVYIKADKQKNGIKANFKIRHNIEDGGVQLAYHYQQNTPIGDGPVLLPDNHYLSVQSILSKDPNEKRDHMVLLEFVTAAGITLGMDELYKGGTGGSMVSKGEEVSSGGVPIQVELDGDVNGHKFSVSGEGEGDATYGKLTLKFICTTGKLPVPWPTLVTTLTYGVQCFSRYPDHMKQHDFFKSAMPEGYIQERTIFFKDDGNYKTRAEVKFEGDTLVNRIELKGIDFKEDGNILGHKLEYNTRVEANTVRLKEHDQDVLVLEKVPAGNRASNQGNSQPQQKYTVMSGTPEKILEHFLETIRLEATLNEATDSVLNDFIMMHCVFMPNTQLCPALVAHYHAQPSQGTEQEKMDYALNNKRRVIRLVLQWAAMYGDLLQEDDVSMAFLEEFYVSVSDDARMIAALKEQLPELEKIVKQISEDAKAPQKKHKVLLQQFNTGDERAQKRQPIRGSDEVLFKVYCMDPTYTTIRVPVATSVKEVISAVADKLGSGEGLIIVKMSSGGEKVVLKPNDVSVFMTLTINGRLFACPREQFDSLTPLPEQEGPTVGTVGTFELMSSKDLAYQMTIYDWELFNCVHELELIYHTFGRHNFKKTTANLDLFLRRFNEIQFWVVTEICLCSQLSKRVQLLKKFIKIAAHCKEYKNLNSFFAIVMGLSNVAVSRLALTWEKLPSKFKKFYAEFESLMDPSRNHRAYRLTVAKLEPPLIPFMPLLIKDMTFTHEGNKTFIDNLVNFEKMRMIANTARTVRYYRSQPFNPDAAQANKNHQDVRSYVRQLNVIDNQRTLSQMSHRLEPRRP

SEQ ID NO: 9 - protein, 1255 aa, Artificial Sequence
  Synthetic
MVAAHAAHSSSSAEWIACLDKRPLERSSEDVDIIFTRLKEVKAFEKFHPNLLHQICLCGYYENLEKGITLFRQGDIGTNWYAVLAGSLDVKVSETSSHQDAVTICTLGIGTAFGESILDNTPRHATIVTRESSELLRIEQKDFKALWEKYRQYMAGLLAPPYGVMETGSNNDRIPDKENTPLIEPHVPLRPANTITKVPSEKILRAGKILRNAILSRAPHMIRDRKYHLKTYRQCCVGTELVDWMMQQTPCVHSRTQAVGMWQVLLEDGVLNHVDQEHHFQDKYLFYRFLDDEHEDAPLPTEEEKKECDEELQDTMLLLSQMGPDAHMRMILRKPPGQRTVDDLEIIYEELLHIKALSHLSTTVKRELAGVLIFESHAKGGTVLFNQGEEGTSWYIILKGSVNVVIYGKGVVCTLHEGDDFGKLALVNDAPRAASIVLREDNCHFLRVDKEDFNRILRDVLENVYIKADKQKNGIKANFKIRHNIEDGGVQLAYHYQQNTPIGDGPVLLPDNHYLSVQSILSKDPNEKRDHMVLLEFVTAAGITLGMDELYKGGTGGSMVSKGEELFTGVVPIQVELDGDVNGHKFSVSGEGEGDATYGKLTLKFICTTGKLPVPWPTLVTTLTYGVQCFSRYPDHMKQHDFFKSAMPEGYIQERTIFFKDDGNYKTRAEVKFEGDTLVNRIELKGIDFKEDGNILGHKLEYNTRANTVRLKEHDQDVLVLEKVPAGNRASNQGNSQPQQKYTVMSGTPEKILEHFLETIRLEATLNEATDSVLNDFIMMHCVFMPNTQLCPALVAHYHAQPSQGTEQEKMDYALNNKRRVIRLVLQWAAMYGDLLQEDDVSMAFLEEFYVSVSDDARMIAALKEQLPELEKIVKQISEDAKAPQKKHKVLLQQFNTGDERAQKRQPIRGSDEVLFKVYCMDPTYTTIRVPVATSVKEVISAVADKLGSGEGLIIVKMSSGGEKVVLKPNDVSVFMTLTINGRLFACPREQFDSLTPLPEQEGPTVGTVGTFELMSSKDLAYQMTIYDWELFNCVHELELIYHTFGRHNFKKTTANLDLFLRRFNEIQFWVVTEICLCSQLSKRVQLLKKFIKIAAHCKEYKNLNSFFAIVMGLSNVAVSRLALTWEKLPSKFKKFYAEFESLMDPSRNHRAYRLTVAKLEPPLIPFMPLLIKDMTFTHEGNKTFIDNLVNFEKMRMIANTARTVRYYRSQPFNPDAAQANKNHQDVRSYVRQLNVIDNQRTLSQMSHRLEPRRP

SEQ ID NO: 10 - protein, 1260 aa, Artificial Sequence
  Synthetic
MVAAHAAHSSSSAEWIACLDKRPLERSSEDVDIIFTRLKEVKAFEKFHPNLLHQICLCGYYENLEKGITLFRQGDIGTNWYAVLAGSLDVKVSETSSHQDAVTICTLGIGTAFGESILDNTPRHATIVTRESSELLRIEQKDFKALWEKYRQYMAGLLAPPYGVMETGSNNDRIPDKENTPLIEPHVPLRPANTITKVPSEKILRAGKILRNAILSRAPHMIRDRKYHLKTYRQCCVGTELVDWMMQQTPCVHSRTQAVGMWQVLLEDGVLNHVDQEHHFQDKYLFYRFLDDEHEDAPLPTEEEKKECDEELQDTMLLLSQMGPDAHMRMILRKPPGQRTVDDLEIIYEELLHIKALSHLSTTVKRELAGVLIFESHAKGGTVLFNQGEEGTSWYIILKGSVNVVIYGKGVVCTLHEGDDFGKLALVNDAPRAASIVLREDNCHFLRVDKEDFNRILRLENVYIKADKQKNGIKANFKIRHNIEDGGVQLAYHYQQNTPIGDGPVLLPDNHYLSVQSILSKDPNEKRDHMVLLEFVTAAGITLGMDELYKGGTGGSMVSKGEELFTGVVPIQVELDGDVNGHKFSVSGEGEGDATYGKLTLKFICTTGKLPVPWPTLVTTLTYGVQCFSRYPDHMKQHDFFKSAMPEGYIQERTIFFKDDGNYKTRAEVKFEGDTLVNRIELKGIDFKEDGNILGHKLEYNTRRILRDVEANTVRLKEHDQDVLVLEKVPAGNRASNQGNSQPQQKYTVMSGTPEKILEHFLETIRLEATLNEATDSVLNDFIMMHCVFMPNTQLCPALVAHYHAQPSQGTEQEKMDYALNNKRRVIRLVLQWAAMYGDLLQEDDVSMAFLEEFYVSVSDDARMIAALKEQLPELEKIVKQISEDAKAPQKKHKVLLQQFNTGDERAQKRQPIRGSDEVLFKVYCMDPTYTTIRVPVATSVKEVISAVADKLGSGEGLIIVKMSSGGEKVVLKPNDVSVFMTLTINGRLFACPREQFDSLTPLPEQEGPTVGTVGTFELMSSKDLAYQMTIYDWELFNCVHELELIYHTFGRHNFKKTTANLDLFLRRFNEIQFWVVTEICLCSQLSKRVQLLKKFIKIAAHCKEYKNLNSFFAIVMGLSNVAVSRLALTWEKLPSKFKKFYAEFESLMDPSRNHRAYRLTVAKLEPPLIPFMPLLIKDMTFTHEGNKTFIDNLVNFEKMRMIANTARTVRYYRSQPFNPDAAQANKNHQDVRSYVRQLNVIDNQRTLSQMSHRLEPRRP

SEQ ID NO: 11 - protein, 1256 aa, Artificial Sequence; identical to SEQ ID NO: 5
  Synthetic

SEQ ID NO: 12 - protein, 1263 aa, Artificial Sequence
  Synthetic
MVAAHAAHSSSSAEWIACLDKRPLERSSEDVDIIFTRLKEVKAFEKFHPNLLHQICLCGYYENLEKGITLFRQGDIGTNWYAVLAGSLDVKVSETSSHQDAVTICTLGIGTAFGESILDNTPRHATIVTRESSELLRIEQKDFKALWEKYRQYMAGLLAPPYGVMETGSNNDRIPDKENTPLIEPHVPLRPANTITKVPSEKILRAGKILRNAILSRAPHMIRDRKYHLKTYRQCCVGTELVDWMMQQTPCVHSRTQAVGMWQVLLEDGVLNHVDQEHHFQDKYLFYRFLDDEHEDAPLPTEEEKKECDEELQDTMLLLSQMGPDAHMRMILRKPPGQRTVDDLEIIYEELLHIKALSHLSTTVKRELAGVLIFESHAKGGTVLFNQGEEGTSWYIILKGSVNVVIYGKGVVCTLHEGDDFGKLALVNDAPRAASIVLREDNCHFLRVDKEDFNRILRDLENVYIKADKQKNGIKANFKIRHNIEDGGVQLAYHYQQNTPIGDGPVLLPDNHYLSVQSILSKDPNEKRDHMVLLEFVTAAGITLGMDELYKGGTGGSMVSKGEELFTGVVPIQVELDGDVNGHKFSVSGEGEGDATYGKLTLKFICTTGKLPVPWPTLVTTLTYGVQCFSRYPDHMKQHDFFKSAMPEGYIQERTIFFKDDGNYKTRAEVKFEGDTLVNRIELKGIDFKEDGNILGHKLEYNTRFNRILRDVEANTVRLKEHDQDVLVLEKVPAGNRASNQGNSQPQQKYTVMSGTPEKILEHFLETIRLEATLNEATDSVLNDFIMMHCVFMPNTQLCPALVAHYHAQPSQGTEQEKMDYALNNKRRVIRLVLQWAAMYGDLLQEDDVSMAFLEEFYVSVSDDARMIAALKEQLPELEKIVKQISEDAKAPQKKHKVLLQQFNTGDERAQKRQPIRGSDEVLFKVYCMDPTYTTIRVPVATSVKEVISAVADKLGSGEGLIIVKMSSGGEKVVLKPNDVSVFMTLTINGRLFACPREQFDSLTPLPEQEGPTVGTVGTFELMSSKDLAYQMTIYDWELFNCVHELELIYHTFGRHNFKKTTANLDLFLRRFNEIQFWVVTEICLCSQLSKRVQLLKKFIKIAAHCKEYKNLNSFFAIVMGLSNVAVSRLALTWEKLPSKFKKFYAEFESLMDPSRNHRAYRLTVAKLEPPLIPFMPLLIKDMTFTHEGNKTFIDNLVNFEKMRMIANTARTVRYYRSQPFNPDAAQANKNHQDVRSYVRQLNVIDNQRTLSQMSHRLEPRRP

SEQ ID NO: 13 - protein, 1255 aa, Artificial Sequence
  Synthetic
MVAAHAAHSSSSAEWIACLDKRPLERSSEDVDIIFTRLKEVKAFEKFHPNLLHQICLCGYYENLEKGITLFRQGDIGTNWYAVLAGSLDVKVSETSSHQDAVTICTLGIGTAFGESILDNTPRHATIVTRESSELLRIEQKDFKALWEKYRQYMAGLLAPPYGVMETGSNNDRIPDKENTPLIEPHVPLRPANTITKVPSEKILRAGKILRNAILSRAPHMIRDRKYHLKTYRQCCVGTELVDWMMQQTPCVHSRTQAVGMWQVLLEDGVLNHVDQEHHFQDKYLFYRFLDDEHEDAPLPTEEEKKECDEELQDTMLLLSQMGPDAHMRMILRKPPGQRTVDDLEIIYEELLHIKALSHLSTTVKRELAGVLIFESHAKGGTVLFNQGEEGTSWYIILKGSVNVVIYGKGVVCTLHEGDDFGKLALVNDAPRAASIVLREDNCHFLRVDKEDFNRILRDVLENVYIKADKQKNGIKANFKIRHNIEDGGVQLAYHYQQNTPIGDGPVLLPDNHYLSVQSILSKDPNEKRDHMVLLEFVTAAGITLGMDELYKGGTGGSMVSKGEELFTRGVVPIQVELDGDVNGHKFSVSGEGEGDATYGKLTLKFICTTGKLPVPWPTLVTTLTYGVQCFSRYPDHMKQHDFFKSAMPEGYIQERTIFFKDDGNYKTRAEVKFEGDTLVNRIELKGIDFKEDGNILGHKLEYNTRNTVRLKEHDQDVLVLEKVPAGNRASNQGNSQPQQKYTVMSGTPEKILEHFLETIRLEATLNEATDSVLNDFIMMHCVFMPNTQLCPALVAHYHAQPSQGTEQEKMDYALNNKRRVIRLVLQWAAMYGDLLQEDDVSMAFLEEFYVSVSDDARMIAALKEQLPELEKIVKQISEDAKAPQKKHKVLLQQFNTGDERAQKRQPIRGSDEVLFKVYCMDPTYTTIRVPVATSVKEVISAVADKLGSGEGLIIVKMSSGGEKVVLKPNDVSVFMTLTINGRLFACPREQFDSLTPLPEQEGPTVGTVGTFELMSSKDLAYQMTIYDWELFNCVHELELIYHTFGRHNFKKTTANLDLFLRRFNEIQFWVVTEICLCSQLSKRVQLLKKFIKIAAHCKEYKNLNSFFAIVMGLSNVAVSRLALTWEKLPSKFKKFYAEFESLMDPSRNHRAYRLTVAKLEPPLIPFMPLLIKDMTFTHEGNKTFIDNLVNFEKMRMIANTARTVRYYRSQPFNPDAAQANKNHQDVRSYVRQLNVIDNQRTLSQMSHRLEPRRP

SEQ ID NO: 14 - protein, 1255 aa, Artificial Sequence
  Synthetic
MVAAHAAHSSSSAEWIACLDKRPLERSSEDVDIIFTRLKEVKAFEKFHPNLLHQICLCGYYENLEKGITLFRQGDIGTNWYAVLAGSLDVKVSETSSHQDAVTICTLGIGTAFGESILDNTPRHATIVTRESSELLRIEQKDFKALWEKYRQYMAGLLAPPYGVMETGSNNDRIPDKENTPLIEPHVPLRPANTITKVPSEKILRAGKILRNAILSRAPHMIRDRKYHLKTYRQCCVGTELVDWMMQQTPCVHSRTQAVGMWQVLLEDGVLNHVDQEHHFQDKYLFYRFLDDEHEDAPLPTEEEKKECDEELQDTMLLLSQMGPDAHMRMILRKPPGQRTVDDLEIIYEELLHIKALSHLSTTVKRELAGVLIFESHAKGGTVLFNQGEEGTSWYIILKGSVNVVIYGKGVVCTLHEGDDFGKLALVNDAPRAASIVLREDNCHFLRVDKEDFNRILRLENVYIKADKQKNGIKANFKIRHNIEDGGVQLAYHYQQNTPIGDGPVLLPDNHYLSVQSILSKDPNEKRDHMVLLEFVTAAGITLGMDELFKGGTGGSMVSKGEELFTGVVPIQVELDGDVNGHKFSVSGEGEGDATYGKLTLKFICTTGKLPVPWPTLVTTLTYGVQCFSRYPDHMKQHDFFKSAMPEGYIQERTIFFKDDGNYKTRAEVKFEGDTLVNRIELKGIDFKEDGNILGHKLEYNTRVEANTVRLKEHDQDVLVLEKVPAGNRASNQGNSQPQQKYTVMSGTPEKILEHFLETIRLEATLNEATDSVLNDFIMMHCVFMPNTQLCPALVAHYHAQPSQGTEQEKMDYALNNKRRVIRLVLQWAAMYGDLLQEDDVSMAFLEEFYVSVSDDARMIAALKEQLPELEKIVKQISEDAKAPQKKHKVLLQQFNTGDERAQKRQPIRGSDEVLFKVYCMDPTYTTIRVPVATSVKEVISAVADKLGSGEGLIIVKMSSGGEKVVLKPNDVSVFMTLTINGRLFACPREQFDSLTPLPEQEGPTVGTVGTFELMSSKDLAYQMTIYDWELFNCVHELELIYHTFGRHNFKKTTANLDLFLRRFNEIQFWVVTEICLCSQLSKRVQLLKKFIKIAAHCKEYKNLNSFFAIVMGLSNVAVSRLALTWEKLPSKFKKFYAEFESLMDPSRNHRAYRLTVAKLEPPLIPFMPLLIKDMTFTHEGNKTFIDNLVNFEKMRMIANTARTVRYYRSQPFNPDAAQANKNHQDVRSYVRQLNVIDNQRTLSQMSHRLEPRRP

SEQ ID NO: 15 - protein, 1261 aa, Artificial Sequence
  Synthetic
MVAAHAAHSSSSAEWIACLDKRPLERSSEDVDIIFTRLKEVKAFEKFHPNLLHQICLCGYYENLEKGITLFRQGDIGTNWYAVLAGSLDVKVSETSSHQDAVTICTLGIGTAFGESILDNTPRHATIVTRESSELLRIEQKDFKALWEKYRQYMAGLLAPPYGVMETGSNNDRIPDKENTPLIEPHVPLRPANTITKVPSEKILRAGKILRNAILSRAPHMIRDRKYHLKTYRQCCVGTELVDWMMQQTPCVHSRTQAVGMWQVLLEDGVLNHVDQEHHFQDKYLFYRFLDDEHEDAPLPTEEEKKECDEELQDTMLLLSQMGPDAHMRMILRKPPGQRTVDDLEIIYEELLHIKALSHLSTTVKRELAGVLIFESHAKGGTVLFNQGEEGTSWYIILKGSVNVVIYGKGVVCTLHEGDDFGKLALVNDAPRAASIVLREDNCHFLRVDKEDFNRILRDVLENVYIKADKQKNGIKANFKIRHNIEDGGVQLAYHYQQNTPIGDGPVLLPDNHYLSVQSILSKDPNEKRDHMVLLEFVTAPGITLGMDELYKGGTGGSMVSKGEELFTGVVPIQVELDGDVNGHKFSVSGEGEGDATYGKLTLKFICTTGKLPVPWPTLVTTLTYGVQCFSRYPDHMKQHDFFKSAMPEGYIQERTIFFKDDGNYKTRAEVKFEGDTLVNRIELKGIDFKEDGNILGHKLEYNTRILRDVEANTVRLKEHDQDVLVLEKVPAGNRASNQGNSQPQQKYTVMSGTPEKILEHFLETIRLEATLNEATDSVLNDFIMMHCVFMPNTQLCPALVAHYHAQPSQGTEQEKMDYALNNKRRVIRLVLQWAAMYGDLLQEDDVSMAFLEEFYVSVSDDARMIAALKEQLPELEKIVKQISEDAKAPQKKHKVLLQQFNTGDERAQKRQPIRGSDEVLFKVYCMDPTYTTIRVPVATSVKEVISAVADKLGSGEGLIIVKMSSGGEKVVLKPNDVSVFMTLTINGRLFACPREQFDSLTPLPEQEGPTVGTVGTFELMSSKDLAYQMTIYDWELFNCVHELELIYHTFGRHNFKKTTANLDLFLRRFNEIQFWVVTEICLCSQLSKRVQLLKKFIKIAAHCKEYKNLNSFFAIVMGLSNVAVSRLALTWEKLPSKFKKFYAEFESLMDPSRNHRAYRLTVAKLEPPLIPFMPLLIKDMTFTHEGNKTFIDNLVNFEKMRMIANTARTVRYYRSQPFNPDAAQANKNHQDVRSYVRQLNVIDNQRTLSQMSHRLEPRRP

SEQ ID NO: 16 - protein, 700 aa, Artificial Sequence
  Synthetic
MVAAHAAHSSSSAEWIACLDKRPLERSSEDVDIIFTRLKEVKAFEKFHPNLLHQICLCGYYENLEKGITLFRQGDIGTNWYAVLAGSLDVKVSETSSHQDAVTICTLGIGTAFGESILDNTPRHATIVTRESSELLRIEQKDFKALWEKYRQYMAGLLAPPYGVMETGSNNDRIPDKENTPLIEPHVPLRPANTITKVPSEKILRAGKILRNAILSRAPHMIRDRKYHLKTYRQCCVGTELVDWMMQQTPCVHSRTQAVGMWQVLLEDGVLNHVDQEHHFQDKYLFYRFLDDEHEDAPLPTEEEKKECDEELQDTMLLLSQMGPDAHMRMILRKPPGQRTVDDLEIIYEELLHIKALSHLSTTVKRELAGVLIFESHAKGGTVLFNQGEEGTSWYIILKGSVNVVIYGKGVVCTLHEGDDFGKLALVNDAPRAASIVLREDNCHFLRVDKEDFNRILRRANVYIKADKQKNGIKANFKIRHNIEDGGVQLAYHYQQNTPIGDGPVLLPDNHYLSVQSILSKDPNEKRDHMVLLEFVTAAGITLGMDELYKGGTGGSMVSKGEELFTGVVPIQVELDGDVNGHKFSVSGEGEGDATYGKLTLKFICTTGKLPVPWPTLVTTLTYGVQCFSRYPDHMKQHDFFKSAMPEGYIQERTIFFKDDGNYKTRAEVKFEGDTLVNRIELKGIDFKEDGNILGHKLEY

SEQ ID NO: 17 - protein, 1256 aa, Artificial Sequence
  Synthetic
MVAAHAAHSSSSAEWIACLDKRPLERSSEDVDIIFTRLKEVKAFEKFHPNLLHQICLCGYYENLEKGITLFRQGDIGTNWYAVLAGSLDVKVSETSSHQDAVTICTLGIGTAFGESILDNTPRHATIVTRESSELLRIEQKDFKALWEKYRQYMAGLLAPPYGVMETGSNNDRIPDKENTPLIEPHVPLRPANTITKVPSEKILRAGKILRNAILSRAPHMIRDRKYHLKTYRQCCVGTELVDWMMQQTPCVHSRTQAVGMWQVLLEDGVLNHVDQEHHFQDKYLFYRFLDDEHEDAPLPTEEEKKECDEELQDTMLLLSQMGPDAHMRMILRKPPGQRTVDDLEIIYEELLHIKALSHLSTTVKRELAGVLIFESHAKGGTVLFNQGEEGTSWYIILKGSVNVVIYGKGVVCTLHEGDDFGKLALVNDAPRAASIVLREDNCHFLRVDKEDFNRILRDVEANLENVYIKADKQKNGIKANFKIRHNIEDGGVQLAYHYQQNTPIGDGPVLLPDNHYLSVQSILSKDPNEKRDHMVLLEFVTAAGITLGMDELYKGGTGGSMVSKGEELFTGVVPIQVELDGDVNGHKFSVSGEGEGDATYGKLTLKFICTTGKLPVPWPTLVTTLTYGVQCFSRYPDHMKQHDFFKSAMPEGYIQERTIFFKDDGNYKTRAEVKFEGDTLVNRIELKGIDFKEDGNILGHKLEYNTRTVRLKEHDQDVLVLEKVPAGNRASNQGNSQPQQKYTVMSGTPEKILEHFLETIRLEATLNEATDSVLNDFIMMHCVFMPNTQLCPALVAHYHAQPSQGTEQEKMDYALNNKRRVIRLVLQWAAMYGDLLQEDDVSMAFLEEFYVSVSDDARMIAALKEQLPELEKIVKQISEDAKAPQKKHKVLLQQFNTGDERAQKRQPIRGSDEVLFKVYCMDPTYTTIRVPVATSVKEVISAVADKLGSGEGLIIVKMSSGGEKVVLKPNDVSVFMTLTINGRLFACPREQFDSLTPLPEQEGPTVGTVGTFELMSSKDLAYQMTIYDWELFNCVHELELIYHTFGRHNFKKTTANLDLFLRRFNEIQFWVVTEICLCSQLSKRVQLLKKFIKIAAHCKEYKNLNSFFAIVMGLSNVAVSRLALTWEKLPSKFKKFYAEFESLMDPSRNHRAYRLTVAKLEPPLIPFMPLLIKDMTFTHEGNKTFIDNLVNFEKMRMIANTARTVRYYRSQPFNPDAAQANKNHQDVRSYVRQLNVIDNQRTLSQMSHRLEPRRP

SEQ ID NO: 18 - protein, 1255 aa, Artificial Sequence
  Synthetic
MVAAHAAHSSSSAEWIACLDKRPLERSSEDVDIIFTRLKEVKAFEKFHPNLLHQICLCGYYENLEKGITLFRQGDIGTNWYAVLAGSLDVKVSETSSHQDAVTICTLGIGTAFGESILDNTPRHATIVTRESSELLRIEQKDFKALWEKYRQYMAGLLAPPYGVMETGSNNDRIPDKENTPLIEPHVPLRPANTITKVPSEKILRAGKILRNAILSRAPHMIRDRKYHLKTYRQCCVGTELVDWMMQQTPCVHSRTQAVGMWQVLLEDGVLNHVDQEHHFQDKYLFYRFLDDEHEDAPLPTEEEKKECDEELQDTMLLLSQMGPDAHMRMILRKPPGQRTVDDLEIIYEELLHIKALSHLSTTVKRELAGVLIFESHAKGGTVLFNQGEEGTSWYIILKGSVNVVIYGKGVVCTLHEGDDFGKLALVNDAPRAASIVLREDNCHFLRVDKEDFNRILRLENVYIKADKQKNGIKANFKIRHNIEDGGVQLAYHYQQNTPIGDGPVLLPDNHYLSVQSILSKDPNEKRDHMVLLEFVTAAGITLGMDELYKGGTGGSMVSKGEELFTGVVPIQVELDGDVNGHKFSVSGEGEGDATYGKLTLKFICTTGKLPVPWPTLVTTLTYGVQCFSRYPDHMKQHDFFKSAMPEGYIQERTIFFKDDGNYKTRAEVKFEGDTLVNRIELKGIDFKEDGNILGHKLEYNTRVEANTVRLKEHDQDVLVLEKVPAGNRASNQGNSQPQQKYTVMSGTPEKILEHFLETIRLEATLNEATDSVLNDFIMMHCVFMPNTQLCPALVAHYHAQPSQGTEQEKMDYALNNKRRVIRLVLQWAAMYGDLLQEDDVSMAFLEEFYVSVSDDARMIAALKEQLPELEKIVKQISEDAKAPQKKHKVLLQQFNTGDERAQKRQPIRGSDEVLFKVYCMDPTYTTIRVPVATSVKEVISAVADKLGSGEGLIIVKMSSGGEKVVLKPNDVSVFMTLTINGRLFACPREQFDSLTPLPEQEGPTVGTVGTFELMSSKDLAYQMTIYDWELFNCVHELELIYHTFGRHNFKKTTANLDLFLRRFNEIQFWVVTEICLCSQLSKRVQLLKKFIKIAAHCKEYKNLNSFFAIVMGLSNVAVSRLALTWEKLPSKFKKFYAEFESLMDPSRNHRAYRLTVAKLEPPLIPFMPLLIKDMTFTHEGNKTFIDNLVNFEKMRMIANTARTVRYYRSQPFNPDAAQANKNHQDVRSYVRQLNVIDNQRTLSQMSHRLEPRRP

SEQ ID NO: 19 - protein, 1258 aa, Artificial Sequence
  Synthetic
MVAAHAAHSSSSAEWIACLDKRPLERSSEDVDIIFTRLKEVKAFEKFHPNLLHQICLCGYYENLEKGITLFRQGDIGTNWYAVLAGSLDVKVSETSSHQDAVTICTLGIGTAFGESILDNTPRHATIVTRESSELLRIEQKDFKALWEKYRQYMAGLLAPPYGVMETGSNNDRIPDKENTPLIEPHVPLRPANTITKVPSEKILRAGKILRNAILSRAPHMIRDRKYHLKTYRQCCVGTELVDWMMQQTPCVHSRTQAVGMWQVLLEDGVLNHVDQEHHFQDKYLFYRFLDDEHEDAPLPTEEEKKECDEELQDTMLLLSQMGPDAHMRMILRKPPGQRTVDDLEIIYEELLHIKALSHLSTTVKRELAGVLIFESHAKGGTVLFNQGEEGTSWYIILKGSVNVVIYGKGVVCTLHEGDDFGKLALVNDAPRAASIVLREDNCHFLRVDKEDFNRILRLENVYIKADKQKNGIKANFKIRHNIEDGGVQLAYHYQQNTPIGDGPVLLPDNHYLSVQSILSKDPNEKRDHMVLLEFVTAAGITLGMDELYKGGTGGSMVSKGEELFTGVVPIQVELDGDVNGHKFSVSGEGEGDATYGKLTLKFICTTGKLPVPWPTLVTTLTYGVQCFSRYPDHMKQHDFFKSAMPEGYIQERTIFFKDDGNYKTRAEVKFEGDTLVNRIELKGIDFKEDGNILGHKLEYNTRILRDVEANTVRLKEHDQDVLVLEKVPAGNRASNQGNSQPQQKYTVMSGTPEKILEHFLETIRLEATLNEATDSVLNDFIMMHCVFMPNTQLCPALVAHYHAQPSQGTEQEKMDYALNNKRRVIRLVLQWAAMYGDLLQEDDVSMAFLEEFYVSVSDDARMIAALKEQLPELEKIVKQISEDAKAPQKKHKVLLQQFNTGDERAQKRQPIRGSDEVLFKVYCMDPTYTTIRVPVATSVKEVISAVADKLGSGEGLIIVKMSSGGEKVVLKPNDVSVFMTLTINGRLFACPREQFDSLTPLPEQEGPTVGTVGTFELMSSKDLAYQMTIYDWELFNCVHELELIYHTFGRHNFKKTTANLDLFLRRFNEIQFWVVTEICLCSQLSKRVQLLKKFIKIAAHCKEYKNLNSFFAIVMGLSNVAVSRLALTWEKLPSKFKKFYAEFESLMDPSRNHRAYRLTVAKLEPPLIPFMPLLIKDMTFTHEGNKTFIDNLVNFEKMRMIANTARTVRYYRSQPFNPDAAQANKNHQDVRSYVRQLNVIDNQRTLSQMSHRLEPRR

SEQ ID NO: 20 - protein, 1252 aa, Artificial Sequence
  Synthetic
MVAAHAAHSSSSAEWIACLDKRPLERSSEDVDIIFTRLKEVKAFEKFHPNLLHQICLCGYYENLEKGITLFRQGDIGTNWYAVLAGSLDVKVSETSSHQDAVTICTLGIGTAFGESILDNTPRHATIVTRESSELLRIEQKDFKALWEKYRQYMAGLLAPPYGVMETGSNNDRIPDKENTPLIEPHVPLRPANTITKVPSEKILRAGKILRNAILSRAPHMIRDRKYHLKTYRQCCVGTELVDWMMQQTPCVHSRTQAVGMWQVLLEDGVLNHVDQEHHFQDKYLFYRFLDDEHEDAPLPTEEEKKECDEELQDTMLLLSQMGPDAHMRMILRKPPGQRTVDDLEIIYEELLHIKALSHLSTTVKRELAGVLIFESHAKGGTVLFNQGEEGTSWYIILKGSVNVVIYGKGVVCTLHEGDDFGKLALVNDAPRAASIVLREDNCHFLRVDKEDFNRILRLENVYIKADKQKNGIKANFKIRHNIEDGGVQLAYHYQQNTPIGDGPVLLPDNHYLSVQSILSKDPNEKRDHMVLLEFVTAAGITLGMDELYKGGTGGSMVSKGEELFTGVVPIQVELDGDVNGHKFSVSGEGEGDATYGKLTLKFICTTGKLPVPWPTLVTTLTYGVQCFSRYPDHMKQHDFFKSAMPEGYIQERTIFFKDDGNYKTRAEVKFEGDTLVNRIELKGIDFKEDGNILGHKLEYNTRNTVRLKEHDQDVLVLEKVPAGNRASNQGNSQPQQKYTVMSGTPEKILEHFLETIRLEATLNEATDSVLNDFIMMHCVFMPNTQLCPALVAHYHAQPSQGTEQEKMDYALNNKRRVIRLVLQWAAMYGDLLQEDDVSMAFLEEFYVSVSDDARMIAALKEQLPELEKIVKQISEDAKAPQKKHKVLLQQFNTGDERAQKRQPIRGSDEVLFKVYCMDPTYTTIRVPVATSVKEVISAVADKLGSGEGLIIVKMSSGGEKVVLKPNDVSVFMTLTINGRLFACPREQFDSLTPLPEQEGPTVGTVGTFELMSSKDLAYQMTIYDWELFNCVHELELIYHTFGRHNFKKTTANLDLFLRRFNEIQFWVVTEICLCSQLSKRVQLLKKFIKIAAHCKEYKNLNSFFAIVMGLSNVAVSRLALTWEKLPSKFKKFYAEFESLMDPSRNHRAYRLTVAKLEPPLIPFMPLLIKDMTFTHEGNKTFIDNLVNFEKMRMIANTARTVRYYRSQPFNPDAAQANKNHQDVRSYVRQLNVIDNQRTLSQMSHRLEPRRP

SEQ ID NO: 21 - protein, 1260 aa, Artificial Sequence
  Synthetic
MVAAHAAHSSSSAEWIACLDKRPLERSSEDVDIIFTRLKEVKAFEKFHPNLLHQICLCGYYENLEKGITLFRQGDIGTNWYAVLAGSLDVKVSETSSHQDAVTICTLGIGTAFGESILDNTPRHATIVTRESSELLRIEQKDFKALWEKYRQYMAGLLAPPYGVMETGSNNDRIPDKENTPLIEPHVPLRPANTITKVPSEKILRAGKILRNAILSRAPHMIRDRKYHLKTYRQCCVGTELVDWMMQQTPCVHSRTQAVGMWQVLLEDGVLNHVDQEHHFQDKYLFYRFLDDEHEDAPLPTEEEKKECDEELQDTMLLLSQMGPDAHMRMILRKPPGQRTVDDLEIIYEELLHIKALSHLSTTVKRELAGVLIFESHAKGGTVLFNQGEEGTSWYIILKGSVNVVIYGKGVVCTLHEGDDFGKLALVNDAPRAASIVLREDNCHFLRVDKEDFNRILRLENVYIKADKQKNGIKANFKIRHNIEDGGVQLAYHYQQNTPIGDGPVLLPDNHYLSVQSILSKDPNEKRDHMVLLEFVTAAGITLGMDELYKGGTGGSMVSKGEELFTGVVPIQVELDGDVNGHKFSVSGEGEGDATYGKLTLKFICTTGKLPVPWPTLVTTLTYGVQCFSRYPDHMKQHDFFKSAMPEGYIQERTIFFKDDGNYKTRAEVKFEGDTLVNRIELKGIDFKEDGNILGHKLEYNTRNRILRDVEANTVRLKEHDQDVLVLEKVPAGNRASNQGNSQPQQKYTVMSGTPEKILEHFLETIRLEATLNEATDSVLNDFIMMHCVFMPNTQLCPALVAHYHAQPSQGTEQEKMDYALNNKRRVIRLVLQWAAMYGDLLQEDDVSMAFLEEFYVSVSDDARMIAALKEQLPELEKIVKQISEDAKAPQKKHKVLLQQFNTGDERAQKRQPIRGSDEVLFKVYCMDPTYTTIRVPVATSVKEVISAVADKLGSGEGLIIVKMSSGGEKVVLKPNDVSVFMTLTINGRLFACPREQFDSLTPLPEQEGPTVGTVGTFELMSSKDLAYQMTIYDWELFNCVHELELIYHTFGRHNFKKTTANLDLFLRRFNEIQFWVVTEICLCSQLSKRVQLLKKFIKIAAHCKEYKNLNSFFAIVMGLSNVAVSRLALTWEKLPSKFKKFYAEFESLMDPSRNHRAYRLTVAKLEPPLIPFMPLLIKDMTFTHEGNKTFIDNLVNFEKMRMIANTARTVRYYRSQPFNPDAAQANKNHQDVRSYVRQLNVIDNQRTLSQMSHRLEPRR

SEQ ID NO: 22 - protein, 1270 aa, Artificial Sequence
  Synthetic
MVAAHAAHSSSSAEWIACLDKRPLERSSEDVDIIFTRLKEVKAFEKFHPNLLHQICLCGYYENLEKGITLFRQGDIGTNWYAVLAGSLDVKVSETSSHQDAVTICTLGIGTAFGESILDNTPRHATIVTRESSELLRIEQKDFKALWEKYRQYMAGLLAPPYGVMETGSNNDRIPDKENTPLIEPHVPLRPANTITKVPSEKILRAGKILRNAILSRAPHMIRDRKYHLKTYRQCCVGTELVDWMMQQTPCVHSRTQAVGMWQVLLEDGVLNHVDQEHHFQDKYLFYRFLDDEHEDAPLPTEEEKKECDEELQDTMLLLSQMGPDAHMRMILRKPPGQRTVDDLEIIYEELLHIKALSHLSTTVKRELAGVLIFESHAKGGTVLFNQGEEGTSWYIILKGSVNVVIYGKGVVCTLHEGDDFGKLALVNDAPRAASIVLREDNCHFLRVDKEDFNRILRDVEANLENVYIKADKQKNGIKANFKIRHNIEDGGVQLAYHYQQNTPIGDGPVLLPDNHYLSVQSILSKDPNEKRDHMVLLEFVTAAGITLGMDELYKGGTGGSMVSKGEELFTGVVPIQVELDGDVNGHKFSVSGEGEGDATYGKLTLKFICTTGKLPVPWPTLVTTLTYGVQCFSRYPDHMKQHDFFKSAMPEGYIQERTIFFKDDGNYKTRAEVKFEGDTLVNRIELKGIDFKEDGNILGHKLEYNTRKEDFNRILRDVEANTVRLKEHDQDVLVLEKVPAGNRASNQGNSQPQQKYTVMSGTPEKILEHFLETIRLEATLNEATDSVLNDFIMMHCVFMPNTQLCPALVAHYHAQPSQGTEQEKMDYALNNKRRVIRLVLQWAAMYGDLLQEDDVSMAFLEEFYVSVSDDARMIAALKEQLPELEKIVKQISEDAKAPQKKHKVLLQQFNTGDERAQKRQPIRGSDEVLFKVYCMDPTYTTIRVPVATSVKEVISAVADKLGSGEGLIIVKMSSGGEKVVLKPNDVSVFMTLTINGRLFACPREQFDSLTPLPEQEGPTVGTVGTFELMSSKDLAYQMTIYDWELFNCVHELELIYHTFGRHNFKKTTANLDLFLRRFNEIQFWVVTEICLCSQLSKRVQLLKKFIKIAAHCKEYKNLNSFFAIVMGLSNVAVSRLALTWEKLPSKFKKFYAEFESLMDPSRNHRAYRLTVAKLEPPLIPFMPLLIKDMTFTHEGNKTFIDNLVNFEKMRMIANTARTVRYYRSQPFNPDAAQANKNHQDVRSYVRQLNVIDNQRTLSQMSHRLEPRRP

SEQ ID NO: 23 - protein, 1253 aa, Artificial Sequence
  Synthetic
MVAAHAAHSSSSAEWIACLDKRPLERSSEDVDIIFTRLKEVKAFEKFHPNLLHQICLCGYYENLEKGITLFRQGDIGTNWYAVLAGSLDVKVSETSSHQDAVTICTLGIGTAFGESILDNTPRHATIVTRESSELLRIEQKDFKALWEKYRQYMAGLLAPPYGVMETGSNNDRIPDKENTPLIEPHVPLRPANTITKVPSEKILRAGKILRNAILSRAPHMIRDRKYHLKTYRQCCVGTELVDWMMQQTPCVHSRTQAVGMWQVLLEDGVLNHVDQEHHFQDKYLFYRFLDDEHEDAPLPTEEEKKECDEELQDTMLLLSQMGPDAHMRMILRKPPGQRTVDDLEIIYEELLHIKALSHLSTTVKRELAGVLIFESHAKGGTVLFNQGEEGTSWYIILKGSVNVVIYGKGVVCTLHEGDDFGKLALVNDAPRAASIVLREDNCHFLRVDKEDFNRILRDVLENVYIKADKQKNGIKANFKIRHNIEDGGVQLAYHYQQNTPIGDGPVLLPDNHYLSVQSILSKDPNEKRDHMVLLEFVTAAGITLGMDELYKGGTGGSMVSKGEELFTGVVPIQVELDGDVNGHKFSVSGEGEGDATYGKLTLKFICTTGKLPVPWPTLVTTLTYGVQCFSRYPDHMKQHDFFKSAMPEGYIQERTIFFKDDGNYKTRAEVKFEGDTLVNRIELKGIDFKEDGNILGHKLEYNTRTVRLKEHDQDVLVLEKVPAGNRASNQGNSQPQQKYTVMSGTPEKILEHFLETIRLEATLNEATDSVLNDFIMMHCVFMPNTQLCPALVAHYHAQPSQGTEQEKMDYALNNKRRVIRLVLQWAAMYGDLLQEDDVSMAFLEEFYVSVSDDARMIAALKEQLPELEKIVKQISEDAKAPQKKHKVLLQQFNTGDERAQKRQPIRGSDEVLFKVYCMDPTYTTIRVPVATSVKEVISAVADKLGSGEGLIIVKMSSGGEKVVLKPNDVSVFMTLTINGRLFACPREQFDSLTPLPEQEGPTVGTVGTFELMSSKDLAYQMTIYDWELFNCVHELELIYHTFGRHNFKKTTANLDLFLRRFNEIQFWVVTEICLCSQLSKRVQLLKKFIKIAAHCKEYKNLNSFFAIVMGLSNVAVSRLALTWEKLPSKFKKFYAEFESLMDPSRNHRAYRLTVAKLEPPLIPFMPLLIKDMTFTHEGNKTFIDNLVNFEKMRMIANTARTVRYYRSQPFNPDAAQANKNHQDVRSYVRQLNVIDNQRTLSQMSHRLEPRRP

SEQ ID NO: 24 - protein, 1256 aa, Artificial Sequence
  Synthetic
MVAAHAAHSSSSAEWIACLDKRPLERSSEDVDIIFTRLKEVKAFEKFHPNLLHQICLCGYYENLEKGITLFRQGDIGTNWYAVLAGSLDVKVSETSSHQDAVTICTLGIGTAFGESILDNTPRHATIVTRESSELLRIEQKDFKALWEKYRQYMAGLLAPPYGVMETGSNNDRIPDKENTPLIEPHVPLRPANTITKVPSEKILRAGKILRNAILSRAPHMIRDRKYHLKTYRQCCVGTELVDWMMQQTPCVHSRTQAVGMWQVLLEDGVLNHVDQEHHFQDKYLFYRFLDDEHEDAPLPTEEEKKECDEELQDTMLLLSQMGPDAHMRMILRKPPGQRTVDDLEIIYEELLHIKALSHLSTTVKRELAGVLIFESHAKGGTVLFNQGEEGTSWYIILKGSVNVVIYGKGVVCTLHEGDDFGKLALVNDAPRAASIVLREDNCHFLRVDKEDFNRILRMSNVYIKADKQKNGIKANFKIRHNIEDGGVQLAYHYQQNTPIGDGPVLLPDNHYLSVQSILSKDPNEKRDHMVLLEFVTAAGITLGMDELYKGGTGGSMVSKGEELFTGVVPIQVELDGDVNGHKFSVSGEGEGDATYGKLTLKFICTTGKLPVPWPTLVTTLTYGVQCFSRYPDHMKQHDFFKSAMPEGYIQERTIFFKDDGNYKTRAEVKFEGDTLVNRIELKGIDFKEDGNILGHKLEYNVSDVEANTVRLKEHDQDVLVLEKVPAGNRASNQGNSQPQQKYTVMSGTPEKILEHFLETIRLEATLNEATDSVLNDFIMMHCVFMPNTQLCPALVAHYHAQPSQGTEQEKMDYALNNKRRVIRLVLQWAAMYGDLLQEDDVSMAFLEEFYVSVSDDARMIAALKEQLPELEKIVKQISEDAKAPQKKHKVLLQQFNTGDERAQKRQPIRGSDEVLFKVYCMDPTYTTIRVPVATSVKEVISAVADKLGSGEGLIIVKMSSGGEKVVLKPNDVSVFMTLTINGRLFACPREQFDSLTPLPEQEGPTVGTVGTFELMSSKDLAYQMTIYDWELFNCVHELELIYHTFGRHNFKKTTANLDLFLRRFNEIQFWVVTEICLCSQLSKRVQLLKKFIKIAAHCKEYKNLNSFFAIVMGLSNVAVSRLALTWEKLPSKFKKFYAEFESLMDPSRNHRAYRLTVAKLEPPLIPFMPLLIKDMTFTHEGNKTFIDNLVNFEKMRMIANTARTVRYYRSQPFNPDAAQANKNHQDVRSYVRQLNVIDNQRTLSQMSHRLEPRRP

SEQ ID NO: 25 - protein, 1256 aa, Artificial Sequence
  Synthetic
MVAAHAAHSSSSAEWIACLDKRPLERSSEDVDIIFTRLKEVKAFEKFHPNLLHQICLCGYYENLEKGITLFRQGDIGTNWYAVLAGSLDVKVSETSSHQDAVTICTLGIGTAFGESILDNTPRHATIVTRESSELLRIEQKDFKALWEKYRQYMAGLLAPPYGVMETGSNNDRIPDKENTPLIEPHVPLRPANTITKVPSEKILRAGKILRNAILSRAPHMIRDRKYHLKTYRQCCVGTELVDWMMQQTPCVHSRTQAVGMWQVLLEDGVLNHVDQEHHFQDKYLFYRFLDDEHEDAPLPTEEEKKECDEELQDTMLLLSQMGPDAHMRMILRKPPGQRTVDDLEIIYEELLHIKALSHLSTTVKRELAGVLIFESHAKGGTVLFNQGEEGTSWYIILKGSVNVVIYGKGVVCTLHEGDDFGKLALVNDAPRAASIVLREDNCHFLRVDKEDFNRILRLENVYIKADKQKNGIKANFKIRHNIEDGGVQLAYHYQQNTPIGDGPVLLPDNHYLSVQSILSKDPNEKRDHMVLLEFVTAAGITLGMDELYKGGTGGSMVSKGEELFTGVVPIQVELDGDVNGHKFSVSGEGEGDATYGKLTLKFICTTGKLPVPWPTLVTTLTYGVQCFSRYPDHMKQHDFFKSAMPEGYIQERTIFFKDDGNYKTRAEVKFEGDTLVNRIELKGIDFKEDGNILGHKLEYNTRDVEANTVRLKEHDQDVLVLEKVPAGNRASNQGNSQPQQKYTVMSGTPEKILEHFLETIRLEATLNEATDSVLNDFIMMHCVFMPNTQLCPALVAHYHAQPSQGTEQEKMDYALNNKRRVIRLVLQWAAMYGDLLQEDDVSMAFLEEFYVSVSDDARMIAALKEQLPELEKIVKQISEDAKAPQKKHKVLLQQFNTGDERAQKRQPIRGSDEVLFKVYCMDPTYTTIRVPVATSVKEVISAVADKLGSGEGLIIVKMSSGGEKVVLKPNDVSVFMTLTINGRLFACPREQFDSLTPLPEQEGPTVGTVGTFELMSSKDLAYQMTIYDWELFNCVHELELIYHTFGRHNFKKTTANLDLFLRRFNEIQFWVVTEICLCSQLSKRVQLLKKFIKIAAHCKEYKNLNSFFAIVMGLSNVAVSRLALTWEKLPSKFKKFYAEFESLMDPSRNHRAYRLTVAKLEPPLIPFMPLLIKDMTFTHEGNKTFIDNLVNFEKMRMIANTARTVRYYRSQPFNPDAAQANKNHQDVRSYVRQLNVIDNQRTLSQMSHRLEPRRP

SEQ ID NO: 26 - protein, 1258 aa, Artificial Sequence
  Synthetic
MVAAHAAHSSSSAEWIACLDKRPLERSSEDVDIIFTRLKEVKAFEKFHPNLLHQICLCGYYENLEKGITLFRQGDIGTNWYAVLAGSLDVKVSETSSHQDAVTICTLGIGTAFGESILDNTPRHATIVTRESSELLRIEQKDFKALWEKYRQYMAGLLAPPYGVMETGSNNDRIPDKENTPLIEPHVPLRPANTITKVPSEKILRAGKILRNAILSRAPHMIRDRKYHLKTYRQCCVGTELVDWMMQQTPCVHSRTQAVGMWQVLLEDGVLNHVDQEHHFQDKYLFYRFLDDEHEDAPLPTEEEKKECDEELQDTMLLLSQMGPDAHMRMILRKPPGQRTVDDLEIIYEELLHIKALSHLSTTVKRELAGVLIFESHAKGGTVLFNQGEEGTSWYIILKGSVNVVIYGKGVVCTLHEGDDFGKLALVNDAPRAASIVLREDNCHFLRVDKEDFNRILRLVSHNVYIKADKQKNGIKANFKIRHNIEDGGVQLAYHYQQNTPIGDGPVLLPDNHYLSVQSILSKDPNEKRDHMVLLEFVTAAGITLGMDELYKGGTGGSMVSKGEELFTGVVPIQVELDGDVNGHKFSVSGEGEGDATYGKLTLKFICTTGKLPVPWPTLVTTLTYGVQCFSRYPDHMKQHDFFKSAMPEGYIQERTIFFKDDGNYKTRAEVKFEGDTLVNRIELKGIDFKEDGNILGHKLEYNFNDVEANTVRLKEHDQDVLVLEKVPAGNRASNQGNSQPQQKYTVMSGTPEKILEHFLETIRLEATLNEATDSVLNDFIMMHCVFMPNTQLCPALVAHYHAQPSQGTEQEKMDYALNNKRRVIRLVLQWAAMYGDLLQEDDVSMAFLEEFYVSVSDDARMIAALKEQLPELEKIVKQISEDAKAPQKKHKVLLQQFNTGDERAQKRQPIRGSDEVLFKVYCMDPTYTTIRVPVATSVKEVISAVADKLGSGEGLIIVKMSSGGEKVVLKPNDVSVFMTLTINGRLFACPREQFDSLTPLPEQEGPTVGTVGTFELMSSKDLAYQMTIYDWELFNCVHELELIYHTFGRHNFKKTTANLDLFLRRFNEIQFWVVTEICLCSQLSKRVQLLKKFIKIAAHCKEYKNLNSFFAIVMGLSNVAVSRLALTWEKLPSKFKKFYAEFESLMDPSRNHRAYRLTVAKLEPPLIPFMPLLIKDMTFTHEGNKTFIDNLVNFEKMRMIANTARTVRYYRSQPFNPDAAQANKNHQDVRSYVRQLNVIDNQRTLSQMSHRLEPRRP

SEQ ID NO: 27 - protein, 1439 aa, Artificial Sequence
  Synthetic
MVAAHAAHSSSSAEWIACLDKRPLERSSEDVDIIFTRLKEVKAFEKFHPNLLHQICLCGYYENLEKGITLFRQGDIGTNWYAVLAGSLDVKVSETSSHQDAVTICTLGIGTAFGESILDNTPRHATIVTRESSELLRIEQKDFKALWEKYRQYMAGLLAPPYGVMETGSNNDRIPDKENTPLIEPHVPLRPANTITKVPSEKILRAGKILRNAILSRAPHMIRDRKYHLKTYRQCCVGTELVDWMMQQTPCVHSRTQAVGMWQVLLEDGVLNHVDQEHHFQDKYLFYRFLDDEHEDAPLPTEEEKKECDEELQDTMLLLSQMGPDAHMRMILRKPPGQRTVDDLEIIYEELLHIKALSHLSTTVKRELAGVLIFESHAKGGTVLFNQGEEGTSWYIILKGSVNVVIYGKGVVCTLHEGDDFGKLALVNDAPRAASIVLREDNCHFLRVDKEDFNRILRDVEANTVRLKEHDQDVLVLEKVPAGNRASNQGNSQPQQKYTVMSGTPEKILEHFLETIRLEATLNEATDSVLNDFIMMHCVFMPNTQLCPALVAHYHAQPSQGTEQEKMDYALNNKRRVIRLVLQWAAMYGDLLQEDDVSMAFLEEFYVSVSDDARMIAALKEQLPELEKIVKQISEDAKAPQKKHKVLLQQFNTGDERAQKRQPIRGSDEVLFKVYCMDPTYTTIRVPVATSVKEVISAVADKLGSGEGLIIVKMSSGGEKVVLKPNDVSVFMTLTINGRLFACPREQFDSLTPLPEQEGPTVGTVGTFELMSSKDLAYQMTIYDWELFNCVHELELIYHTFGRHNFKKTTANLDLFLRRFNEIQFWVVTEICLCSQLSKRVQLLKKFIKIAAHCKEYKNLNSFFAIVMGLSNVAVSRLALTWEKLPSKFKKFYAEFESLMDPSRNHRAYRLTVAKLEPPLIPFMPLLIKDMTFTHEGNKTFIDNLVNFEKMRMIANTARTVRYYRSQPFNPDAAQANKNHQDVRSYVRQLNVIDNQRTLSQMSHRLEPRRPLENVYIKADKQKNGIKANFKIRHNIEDGGVQLAYHYQQNTPIGDGPVLLPDNHYLSVQSILSKDPNEKRDHMVLLEFVTAAGITLGMDELYKGGTGGSMVSKGEELFTGVVPIQVELDGDVNGHKFSVSGEGEGDATYGKLTLKFICTTGKLPVPWPTLVTTLTYGVQCFSRYPDHMKQHDFFKSAMPEGYIQERTIFFKDDGNYKTRAEVKFEGDTLVNRIELKGIDFKEDGNILGHKLEYNTRREYKLVVLGSGGVGKSALTVQFVQGIFVEKYDPTIEDSYRKQVEVDAQQCMLEILDTAGTEQFTAMRDLYMKNGQGFALVYSITAQSTFNDLQDLREQILRVKDTDDVPMILVGNKCDLEDERVVGKEQGQNLARQWNNCAFLESSAKSKINVNEIFYDLVRQINRKTPVPGKARKKSSCQLL

SEQ ID NO: 28 - protein, 1256 aa, Artificial Sequence
  Synthetic
MVAAHAAHSSSSAEWIACLDKRPLERSSEDVDIIFTRLKEVKAFEKFHPNLLHQICLCGYYENLEKGITLFRQGDIGTNWYAVLAGSLDVKVSETSSHQDAVTICTLGIGTAFGESILDNTPRHATIVTRESSELLRIEQKDFKALWEKYRQYMAGLLAPPYGVMETGSNNDRIPDKENTPLIEPHVPLRPANTITKVPSEKILRAGKILRNAILSRAPHMIRDRKYHLKTYRQCCVGTELVDWMMQQTPCVHSRTQAVGMWQVLLEDGVLNHVDQEHHFQDKYLFYRFLDDEHEDAPLPTEEEKKECDEELQDTMLLLSQMGPDAHMRMILRKPPGQRTVDDLEIIYEELLHIKALSHLSTTVKRELAGVLIFESHAKGGTVLFNQGEEGTSWYIILKGSVNVVIYGKGVVCTLHEGDDFGKLALVNDAPRAASIVLREDNCHFLRVDKEDFNRILRDVELENVYIKADKQKNGIKANFKIRHNIEDGGVQLAYHYQQNTPIGDGPVLLPDNHYLSVQSILSKDPNEKRDHMVLLEFVTAAGITLGMDELYKGGTGGSMVSKGEELFTGVVPIQVELDGDVNGHKFSVSGEGEGDATYGKLTLKFICTTGKLPVPWPTLVTTLTYGVQCFSRYPDHMKQHDFFKSAMPEGYIQERTIFFKDDGNYKTRAEVKFEGDTLVNRIELKGIDFKEDGNILGHKLEYNTRANTVRLKEHDQDVLVLEKVPAGNRASNQGNSQPQQKYTVMSGTPEKILEHFLETIRLEATLNEATDSVLNDFIMMHCVFMPNTQLCPALVAHYHAQPSQGTEQEKMDYALNNKRRVIRLVLQWAAMYGDLLQEDDVSMAFLEEFYVSVSDDARMIAALKEQLPELEKIVKQISEDAKAPQKKHKVLLQQFNTGDERAQKRQPIRGSDEVLFKVYCMDPTYTTIRVPVATSVKEVISAVADKLGSGEGLIIVKMSSGGEKVVLKPNDVSVFMTLTINGRLFACPREQFDSLTPLPEQEGPTVGTVGTFELMSSKDLAYQMTIYDWELFNCVHELELIYHTFGRHNFKKTTANLDLFLRRFNEIQFWVVTEICLCSQLSKRVQLLKKFIKIAAHCKEYKNLNSFFAIVMGLSNVAVSRLALTWEKLPSKFKKFYAEFESLMDPSRNHRAYRLTVAKLEPPLIPFMPLLIKDMTFTHEGNKTFIDNLVNFEKMRMIANTARTVRYYRSQPFNPDAAQANKNHQDVRSYVRQLNVIDNQRTLSQMSHRLEPRRP

SEQ ID NO: 29 - protein, 1256 aa, Artificial Sequence
  Synthetic
MVAAHAAHSSSSAEWIACLDKRPLERSSEDVDIIFTRLKEVKAFEKFHPNLLHQICLCGYYENLEKGITLFRQGDIGTNWYAVLAGSLDVKVSETSSHQDAVTICTLGIGTAFGESILDNTPRHATIVTRESSELLRIEQKDFKALWEKYRQYMAGLLAPPYGVMETGSNNDRIPDKENTPLIEPHVPLRPANTITKVPSEKILRAGKILRNAILSRAPHMIRDRKYHLKTYRQCCVGTELVDWMMQQTPCVHSRTQAVGMWQVLLEDGVLNHVDQEHHFQDKYLFYRFLDDEHEDAPLPTEEEKKECDEELQDTMLLLSQMGPDAHMRMILRKPPGQRTVDDLEIIYEELLHIKALSHLSTTVKRELAGVLIFESHAKGGTVLFNQGEEGTSWYIILKGSVNVVIYGKGVVCTLHEGDDFGKLALVNDAPRAASIVLREDNCHFLRVDKEDFNRILRDVEANTVRLKEHDQDVLVLEKVPAGNRASNQGNSQPQQKYTVMSGTPEKILEHFLETIRLLENVYIKADKQKNGIKANFKIRHNIEDGGVQLAYHYQQNTPIGDGPVLLPDNHYLSVQSILSKDPNEKRDHMVLLEFVTAAGITLGMDELYKGGTGGSMVSKGEELFTGVVPIQVELDGDVNGHKFSVSGEGEGDATYGKLTLKFICTTGKLPVPWPTLVTTLTYGVQCFSRYPDHMKQHDFFKSAMPEGYIQERTIFFKDDGNYKTRAEVKFEGDTLVNRIELKGIDFKEDGNILGHKLEYNTREATLNEATDSVLNDFIMMHCVFMPNTQLCPALVAHYHAQPSQGTEQEKMDYALNNKRRVIRLVLQWAAMYGDLLQEDDVSMAFLEEFYVSVSDDARMIAALKEQLPELEKIVKQISEDAKAPQKKHKVLLQQFNTGDERAQKRQPIRGSDEVLFKVYCMDPTYTTIRVPVATSVKEVISAVADKLGSGEGLIIVKMSSGGEKVVLKPNDVSVFMTLTINGRLFACPREQFDSLTPLPEQEGPTVGTVGTFELMSSKDLAYQMTIYDWELFNCVHELELIYHTFGRHNFKKTTANLDLFLRRFNEIQFWVVTEICLCSQLSKRVQLLKKFIKIAAHCKEYKNLNSFFAIVMGLSNVAVSRLALTWEKLPSKFKKFYAEFESLMDPSRNHRAYRLTVAKLEPPLIPFMPLLIKDMTFTHEGNKTFIDNLVNFEKMRMIANTARTVRYYRSQPFNPDAAQANKNHQDVRSYVRQLNVIDNQRTLSQMSHRLEPRRP

SEQ ID NO: 30 - protein, 1256 aa, Artificial Sequence
  Synthetic
MVAAHAAHSSSSAEWIACLDKRPLERSSEDVDIIFTRLKEVKAFEKFHPNLLHQICLCGYYENLEKGITLFRQGDIGTNWYAVLAGSLDVKVSETSSHQDAVTICTLGIGTAFGESILDNTPRHATIVTRESSELLRIEQKDFKALWEKYRQYMAGLLAPPYGVMETGSNNDRIPDKENTPLIEPHVPLRPANTITKVPSEKILRAGKILRNAILSRAPHMIRDRKYHLKTYRQCCVGTELVDWMMQQTPCVHSRTQAVGMWQVLLEDGVLNHVDQEHHFQDKYLFYRFLDDEHEDAPLPTEEEKKECDEELQDTMLLLSQMGPDAHMRMILRKPPGQRTVDDLEIIYEELLHIKALSHLSTTVKRELAGVLIFESHAKGGTVLFNQGEEGTSWYIILKGSVNVVIYGKGVVCTLHEGDDFGKLALVNDAPRAASIVLREDNCHFLRVDKEDFNRILLENVYIKADKQKNGIKANFKIRHNIEDGGVQLAYHYQQNTPIGDGPVLLPDNHYLSVQSILSKDPNEKRDHMVLLEFVTAAGITLGMDELYKGGTGGSMVSKGEELFTGVVPIQVELDGDVNGHKFSVSGEGEGDATYGKLTLKFICTTGKLPVPWPTLVTTLTYGVQCFSRYPDHMKQHDFFKSAMPEGYIQERTIFFKDDGNYKTRAEVKFEGDTLVNRIELKGIDFKEDGNILGHKLEYNTRRDVEANTVRLKEHDQDVLVLEKVPAGNRASNQGNSQPQQKYTVMSGTPEKILEHFLETIRLEATLNEATDSVLNDFIMMHCVFMPNTQLCPALVAHYHAQPSQGTEQEKMDYALNNKRRVIRLVLQWAAMYGDLLQEDDVSMAFLEEFYVSVSDDARMIAALKEQLPELEKIVKQISEDAKAPQKKHKVLLQQFNTGDERAQKRQPIRGSDEVLFKVYCMDPTYTTIRVPVATSVKEVISAVADKLGSGEGLIIVKMSSGGEKVVLKPNDVSVFMTLTINGRLFACPREQFDSLTPLPEQEGPTVGTVGTFELMSSKDLAYQMTIYDWELFNCVHELELIYHTFGRHNFKKTTANLDLFLRRFNEIQFWVVTEICLCSQLSKRVQLLKKFIKIAAHCKEYKNLNSFFAIVMGLSNVAVSRLALTWEKLPSKFKKFYAEFESLMDPSRNHRAYRLTVAKLEPPLIPFMPLLIKDMTFTHEGNKTFIDNLVNFEKMRMIANTARTVRYYRSQPFNPDAAQANKNHQDVRSYVRQLNVIDNQRTLSQMSHRLEPRRP

SEQ ID NO: 31 - protein, 1256 aa, Artificial Sequence
  Synthetic
MVAAHAAHSSSSAEWIACLDKRPLERSSEDVDIIFTRLKEVKAFEKFHPNLLHQICLCGYYENLEKGITLFRQGDIGTNWYAVLAGSLDVKVSETSSHQDAVTICTLGIGTAFGESILDNTPRHATIVTRESSELLRIEQKDFKALWEKYRQYMAGLLAPPYGVMETGSNNDRIPDKENTPLIEPHVPLRPANTITKVPSEKILRAGKILRNAILSRAPHMIRDRKYHLKTYRQCCVGTELVDWMMQQTPCVHSRTQAVGMWQVLLEDGVLNHVDQEHHFQDKYLFYRFLDDEHEDAPLPTEEEKKECDEELQDTMLLLSQMGPDAHMRMILRKPPGQRTVLENVYIKADKQKNGIKANFKIRHNIEDGGVQLAYHYQQNTPIGDGPVLLPDNHYLSVQSILSKDPNEKRDHMVLLEFVTAAGITLGMDELYKGGTGGSMVSKGEELFTGVVPIQVELDGDVNGHKFSVSGEGEGDATYGKLTLKFICTTGKLPVPWPTLVTTLTYGVQCFSRYPDHMKQHDFFKSAMPEGYIQERTIFFKDDGNYKTRAEVKFEGDTLVNRIELKGIDFKEDGNILGHKLEYNTRDDLEIIYEELLHIKALSHLSTTVKRELAGVLIFESHAKGGTVLFNQGEEGTSWYIILKGSVNVVIYGKGVVCTLHEGDDFGKLALVNDAPRAASIVLREDNCHFLRVDKEDFNRILRDVEANTVRLKEHDQDVLVLEKVPAGNRASNQGNSQPQQKYTVMSGTPEKILEHFLETIRLEATLNEATDSVLNDFIMMHCVFMPNTQLCPALVAHYHAQPSQGTEQEKMDYALNNKRRVIRLVLQWAAMYGDLLQEDDVSMAFLEEFYVSVSDDARMIAALKEQLPELEKIVKQISEDAKAPQKKHKVLLQQFNTGDERAQKRQPIRGSDEVLFKVYCMDPTYTTIRVPVATSVKEVISAVADKLGSGEGLIIVKMSSGGEKVVLKPNDVSVFMTLTINGRLFACPREQFDSLTPLPEQEGPTVGTVGTFELMSSKDLAYQMTIYDWELFNCVHELELIYHTFGRHNFKKTTANLDLFLRRFNEIQFWVVTEICLCSQLSKRVQLLKKFIKIAAHCKEYKNLNSFFAIVMGLSNVAVSRLALTWEKLPSKFKKFYAEFESLMDPSRNHRAYRLTVAKLEPPLIPFMPLLIKDMTFTHEGNKTFIDNLVNFEKMRMIANTARTVRYYRSQPFNPDAAQANKNHQDVRSYVRQLNVIDNQRTLSQMSHRLEPRRP

SEQ ID NO: 32 - protein, 1256 aa, Artificial Sequence
  Synthetic
MVAAHAAHSSSSAEWIACLDKRPLERSSEDVDIIFTRLKEVKAFEKFHPNLLHQICLCGYYENLEKGITLFRQGDIGTNWYAVLAGSLDVKVSETSSHQDAVTICTLGIGTAFGESILDNTPRHATIVTRESSELLRIEQKDFKALWEKYRQYMAGLLAPPYGVMETGSNNDRIPDKENTPLIEPHVPLRPANTITKVPSEKILRAGKILRNAILSRAPHMIRDRKYHLKTYRQCCVGTELVDWMMQQTPCVHSRTQAVGMWQVLLEDGVLNHVDQEHHFQDKYLFYRFLDDEHEDAPLPTEEEKKECDEELQDTMLLLSQMGPDAHMRMILRKPPGQRTVDDLEIIYEELLHIKALSHLSTTVKRELAGVLIFESHAKGGTVLFNQGEEGTSWYIILKGSVNVVIYGKGVVCTLHEGDDFGKLALVNDAPRAASIVLREDNCHFLRVDKEDFNRILRDVEANTVRLKEHDQDVLVLEKVPAGNRALENVYIKADKQKNGIKANFKIRHNIEDGGVQLAYHYQQNTPIGDGPVLLPDNHYLSVQSILSKDPNEKRDHMVLLEFVTAAGITLGMDELYKGGTGGSMVSKGEELFTGVVPIQVELDGDVNGHKFSVSGEGEGDATYGKLTLKFICTTGKLPVPWPTLVTTLTYGVQCFSRYPDHMKQHDFFKSAMPEGYIQERTIFFKDDGNYKTRAEVKFEGDTLVNRIELKGIDFKEDGNILGHKLEYNTRSNQGNSQPQQKYTVMSGTPEKILEHFLETIRLEATLNEATDSVLNDFIMMHCVFMPNTQLCPALVAHYHAQPSQGTEQEKMDYALNNKRRVIRLVLQWAAMYGDLLQEDDVSMAFLEEFYVSVSDDARMIAALKEQLPELEKIVKQISEDAKAPQKKHKVLLQQFNTGDERAQKRQPIRGSDEVLFKVYCMDPTYTTIRVPVATSVKEVISAVADKLGSGEGLIIVKMSSGGEKVVLKPNDVSVFMTLTINGRLFACPREQFDSLTPLPEQEGPTVGTVGTFELMSSKDLAYQMTIYDWELFNCVHELELIYHTFGRHNFKKTTANLDLFLRRFNEIQFWVVTEICLCSQLSKRVQLLKKFIKIAAHCKEYKNLNSFFAIVMGLSNVAVSRLALTWEKLPSKFKKFYAEFESLMDPSRNHRAYRLTVAKLEPPLIPFMPLLIKDMTFTHEGNKTFIDNLVNFEKMRMIANTARTVRYYRSQPFNPDAAQANKNHQDVRSYVRQLNVIDNQRTLSQMSHRLEPRRP

SEQ ID NO: 33 - protein, 1256 aa, Artificial Sequence
  Synthetic
MVAAHAAHSSSSAEWIACLDKRPLERSSEDVDIIFTRLKEVKAFEKFHPNLLHQICLCGYYENLEKGITLFRQGDIGTNWYAVLAGSLDVKVSETSSHQDAVTICTLGIGTAFGESILDNTPRHATIVTRESSELLRIEQKDFKALWEKYRQYMAGLLAPPYGVMETGSNNDRIPDKENTPLIEPHVPLRPANTITKVPSEKILRAGKILRNAILSRAPHMIRDRKYHLKTYRQCCVGTELVDWMMQQTPCVHSRTQAVGMWQVLLEDGVLNHVDQEHHFQDKYLFYRFLDDEHEDAPLPTEEEKKECDEELQDTMLLLSQMGPDAHMRMILRKPPGQRTVDDLEIIYEELLHIKALSHLSTTVKRELAGVLIFESHAKGGTVLFNQGEEGTSWYIILKGSVNVVIYGKGVVCTLHEGDDFGKLALVNDAPRAASIVLREDNCHFLRVDKEDFNRILRDVEANTVRLKEHDQDVLVLEKVPAGNRASNQGNSQPQQKYTVMSGTPEKILEHFLETIRLEALENVYIKADKQKNGIKANFKIRHNIEDGGVQLAYHYQQNTPIGDGPVLLPDNHYLSVQSILSKDPNEKRDHMVLLEFVTAAGITLGMDELYKGGTGGSMVSKGEELFTGVVPIQVELDGDVNGHKFSVSGEGEGDATYGKLTLKFICTTGKLPVPWPTLVTTLTYGVQCFSRYPDHMKQHDFFKSAMPEGYIQERTIFFKDDGNYKTRAEVKFEGDTLVNRIELKGIDFKEDGNILGHKLEYNTRTLNEATDSVLNDFIMMHCVFMPNTQLCPALVAHYHAQPSQGTEQEKMDYALNNKRRVIRLVLQWAAMYGDLLQEDDVSMAFLEEFYVSVSDDARMIAALKEQLPELEKIVKQISEDAKAPQKKHKVLLQQFNTGDERAQKRQPIRGSDEVLFKVYCMDPTYTTIRVPVATSVKEVISAVADKLGSGEGLIIVKMSSGGEKVVLKPNDVSVFMTLTINGRLFACPREQFDSLTPLPEQEGPTVGTVGTFELMSSKDLAYQMTIYDWELFNCVHELELIYHTFGRHNFKKTTANLDLFLRRFNEIQFWVVTEICLCSQLSKRVQLLKKFIKIAAHCKEYKNLNSFFAIVMGLSNVAVSRLALTWEKLPSKFKKFYAEFESLMDPSRNHRAYRLTVAKLEPPLIPFMPLLIKDMTFTHEGNKTFIDNLVNFEKMRMIANTARTVRYYRSQPFNPDAAQANKNHQDVRSYVRQLNVIDNQRTLSQMSHRLEPRRP

SEQ ID NO: 34 - protein, 14 aa, Homo sapiens
KEDFNRILRDVEAN

SEQ ID NO: 35 - protein, 1011 aa, Homo sapiens
MVAAHAAHSSSSAEWIACLDKRPLERSSEDVDIIFTRLKEVKAFEKFHPNLLHQICLCGYYENLEKGITLFRQGDIGTNWYAVLAGSLDVKVSETSSHQDAVTICTLGIGTAFGESILDNTPRHATIVTRESSELLRIEQKDFKALWEKYRQYMAGLLAPPYGVMETGSNNDRIPDKENTPLIEPHVPLRPANTITKVPSEKILRAGKILRNAILSRAPHMIRDRKYHLKTYRQCCVGTELVDWMMQQTPCVHSRTQAVGMWQVLLEDGVLNHVDQEHHFQDKYLFYRFLDDEHEDAPLPTEEEKKECDEELQDTMLLLSQMGPDAHMRMILRKPPGQRTVDDLEIIYEELLHIKALSHLSTTVKRELAGVLIFESHAKGGTVLFNQGEEGTSWYIILKGSVNVVIYGKGVVCTLHEGDDFGKLALVNDAPRAASIVLREDNCHFLRVDKEDFNRILRDVEANTVRLKEHDQDVLVLEKVPAGNRASNQGNSQPQQKYTVMSGTPEKILEHFLETIRLEATLNEATDSVLNDFIMMHCVFMPNTQLCPALVAHYHAQPSQGTEQEKMDYALNNKRRVIRLVLQWAAMYGDLLQEDDVSMAFLEEFYVSVSDDARMIAALKEQLPELEKIVKQISEDAKAPQKKHKVLLQQFNTGDERAQKRQPIRGSDEVLFKVYCMDPTYTTIRVPVATSVKEVISAVADKLGSGEGLIIVKMSSGGEKVVLKPNDVSVFMTLTINGRLFACPREQFDSLTPLPEQEGPTVGTVGTFELMSSKDLAYQMTIYDWELFNCVHELELIYHTFGRHNFKKTTANLDLFLRRFNEIQFWVVTEICLCSQLSKRVQLLKKFIKIAAHCKEYKNLNSFFAIVMGLSNVAVSRLALTWEKLPSKFKKFYAEFESLMDPSRNHRAYRLTVAKLEPPLIPFMPLLIKDMTFTHEGNKTFIDNLVNFEKMRMIANTARTVRYYRSQPFNPDAAQANKNHQDVRSYVRQLNVIDNQRTLSQMSHRLEPRRP

SEQ ID NO: 36 - protein, 124 aa, Artificial Sequence
  Synthetic
AFEKFHPNLLHQICLCGYYENLEKGITLFRQGDIGTNWYAVLAGSLDVKVSETSSHQDAVTICTLGIGTAFGESILDNTPRHATIVTRESSELLRIEQKDFKALWEKYRQYMAGLLAPPYGVME

SEQ ID NO: 37 - protein, 121 aa, Artificial Sequence
  Synthetic
ALSHLSTTVKRELAGVLIFESHAKGGTVLFNQGEEGTSWYIILKGSVNVVIYGKGVVCTLHEGDDFGKLALVNDAPRAASIVLREDNCHFLRVDKEDFNRILRDVEANTVRLKEHDQDVLV

SEQ ID NO: 38 - protein, 241 aa, Artificial Sequence
  Synthetic
NVYIKADKQKNGIKANFKIRHNIEDGGVQLAYHYQQNTPIGDGPVLLPDNHYLSVQSALSKDPNEKRDHMVLLEFVTAAGITHGMDELYKGGTGGSMVSKGEELFTGVVPIQVELDGDVNGHKFSVSGEGEGDATYGKLTLKFICTTGKLPVPWPTLVTTLTYGVQCFSRYPDHMKQHDFFKSAMPEGYIQERTIFFKDDGNYKTRAEVKFEGDTLVNRIELKGIDFKEDGNILGHKLEYN

SEQ ID NO: 39 - DNA, 3033 bp, Homo sapiens
atggtcgctgcgcacgctgcccattcttcctcctctgccgagtggatcgcctgcctggataaaagaccactggagcgatccagcgaagatgtggatataatcttcactcgactgaaagaagttaaagcttttgagaaatttcacccaaatctccttcatcagatttgcttatgtggttattatgagaatctggaaaagggaataacattatttcgccagggtgatattggaacaaactggtatgctgtcctggcagggtctttggatgttaaagtatctgagaccagcagtcaccaggatgctgtgaccatctgtaccctgggaattgggacggcctttggagagtccattctggacaacacaccccgccatgcaaccatcgttaccagggagagcagtgaactgctccgcatcgagcagaaggacttcaaggcactatgggagaaatatcgacagtatatggcaggacttctggctcctccttatggtgttatggaaacgggctctaacaatgacaggattcctgacaaggagaacacacctctcattgaacctcacgttcctcttcgtcctgctaacaccattaccaaggtcccttcagagaagatcctcagagctggaaaaattttacgaaatgccattctctctcgagcacctcacatgataagagatagaaaataccacctaaagacatacagacaatgctgtgtgggaactgaactggtggactggatgatgcagcagacaccatgtgttcactcccggactcaagctgttggcatgtggcaagtcctgttagaagatggtgttctcaaccacgtggaccaggagcaccatttccaagacaaatatttattctatcgatttctggatgatgagcacgaggatgcccctttgcctactgaggaggagaagaaggagtgtgatgaggagctccaggacaccatgctgctgctgtcacagatgggccccgacgcccacatgaggatgatccttcgcaaaccacctggccagaggactgtggatgacctagagattatctatgaggagcttcttcatattaaagccttatcccatctttctaccacagtgaaacgagagttagcaggtgttctcatttttgagtctcacgccaaaggagggactgtgttgtttaaccagggggaagaaggtacctcctggtacattattctaaaaggatcagtgaatgtagtcatttacggcaagggtgtggtctgcaccctgcatgaaggagatgacttcggcaagttagcactagtgaatgatgccccacgagctgcctctatcgtcttacgagaagataactgccatttcttaagagtagacaaggaggatttcaaccggatcctaagggacgtggaggcgaatacagtcagacttaaagaacatgaccaagatgtcttggtgctggagaaggtcccagcagggaacagagcttctaatcaaggaaactcacagcctcagcaaaagtatactgtgatgtcaggaacacctgaaaaaattttagagcattttctagaaacaatacgccttgaggcaactttaaatgaagcaacagattctgttttaaatgactttattatgatgcactgtgtttttatgccaaatacccagctttgcccggcactggtggcccactaccacgcacagccttcacaaggtacagaacaggagaaaatggattatgccctcaacaataagaggcgagtcatccgcctggttctacagtgggctgccatgtatggagacctcctgcaagaggatgacgtgtctatggccttcctggaggagttttatgtatctgtatcagatgatgcccggatgattgctgccctcaaggagcaactgccagagttggagaagattgtcaagcaaatctcagaagatgcaaaggcaccacaaaagaagcacaaggttcttttgcaacagttcaatacgggcgatgagagagcccagaagcgccagcctatccgcggctctgatgaagttctgtttaaggtctattgcatggaccccacctacacaaccattcgggtgccagtggccacttcggtgaaggaagtcatcagtgcagttgccgacaagctgggctccggggagggcctgatcatagtcaagatgagttccggaggagaaaaggtggtgctcaaacctaatgatgtttcagtatttatgacgctcaccattaatggacgcctgtttgcttgcccgcgagagcaattcgattcactgactcccttaccagaacaggaaggcccaactgttggaacagtgggaacttttgaactgatgagctccaaagatttagcataccagatgacaatttatgattgggaactcttcaactgcgtgcatgagctggagctaatctatcacacatttggaaggcataattttaaaaagaccacagcaaacttggatttgttcctgaggagatttaatgaaattcagttttgggtcgtcactgagatctgcctttgttctcagctcagcaagcgtgttcagctattaaaaaaatttattaagatagcagcccactgtaaggagtataaaaatctgaattccttttttgccatcgtcatgggactaagtaacgttgctgtgagccgcttggcactaacgtgggagaaactgccaagcaagttcaagaagttctatgcggagtttgaaagtttaatggacccttcaaggaaccacagggcctacaggctgacagtagctaagctggaacctcctctcatccccttcatgcctttgctcattaaagatatgacatttactcatgaggggaacaagacgttcattgacaatctagtaaactttgaaaaaatgcgcatgattgcaaatacggccagaacagtgagatactacaggagccaacccttcaatcctgatgcagctcaagctaataagaaccatcaggatgtccggagttatgtacggcaattaaatgtgattgacaaccagagaactttatcacagatgtcacacagattagagcctcgtcgacca

SEQ ID NO: 40 - DNA, 42 bp, Homo sapiens
aaggaggatttcaaccggatcctaagggacgtggaggcgaat

SEQ ID NO: 41 - DNA, 2217 bp, Artificial Sequence
  Synthetic
atgggctctaacaatgacaggattcctgacaaggagaacacacctctcattgaacctcacgttcctcttcgtcctgctaacaccattaccaaggtcccttcagagaagatcctcagagctggaaaaattttacgaaatgccattctctctcgagcacctcacatgataagagatagaaaataccacctaaagacatacagacaatgctgtgtgggaactgaactggtggactggatgatgcagcagacaccatgtgttcactcccggactcaagctgttggcatgtggcaagtcctgttagaagatggtgttctcaaccacgtggaccaggagcaccatttccaagacaaatatttattctatcgatttctggatgatgagcacgaggatgcccctttgcctactgaggaggagaagaaggagtgtgatgaggagctccaggacaccatgctgctgctgtcacagatgggccccgacgcccacatgaggatgatccttcgcaaaccacctggccagaggactgtggatgacctagagattatctatgaggagcttcttcatattaaagccttatcccatctttctaccacagtgaaacgagagttagcaggtgttctcatttttgagtctcacgccaaaggagggactgtgttgtttaaccagggggaagaaggtacctcctggtacattattctaaaaggatcagtgaatgtagtcatttacggcaagggtgtggtctgcaccctgcatgaaggagatgacttcggcaagttagcactagtgaatgatgccccacgagctgcctctatcgtcttacgagaagataactgccatttcttaagagtagacaaggaggatttcaaccggatcctaaggctggtgtcgcacaacgtctatatcaaggccgacaagcagaagaacggcatcaaggcgaacttcaagatccgccacaacatcgaggacggcggcgtgcagctcgcctaccactaccagcagaacacccccatcggcgacggccccgtgctgctgcccgacaaccactacctgagcgtgcagtccatactttcgaaagaccccaacgagaagcgcgatcacatggtcctgctggagttcgtgaccgccgccgggatcactctcggcatggacgagctgtacaagggcggtaccggagggagcatggtgagcaagggcgaggagctgttcaccggggtggtgcccatccaggtcgagctggacggcgacgtaaacggccacaagttcagcgtgtccggcgagggtgagggcgatgccacctacggcaagctgaccctgaagttcatctgcaccaccggcaagctgcccgtgccctggcccaccctcgtgaccaccctgacctacggcgtgcagtgcttcagccgctaccccgaccacatgaagcagcacgacttcttcaagtccgccatgcccgaaggctacatccaggagcgcaccatcttcttcaaggacgacggcaactacaagacccgcgccgaggtgaagttcgagggcgacaccctggtgaaccgcatcgagctgaagggcatcgacttcaaggaggacggcaacatcctggggcacaagctggagtacaacttcaacaaccctgacgtggaggcgaatacagtcagacttaaagaacatgaccaagatgtcttggtgctggagaaggtcccagcagggaacagagcttctaatcaaggaaactcacagcctcagcaaaagtatactgtgatgtcaggaacacctgaaaaaattttagagcattttctagaaacaatacgccttgaggcaactttaaatgaagcaacagattctgttttaaatgactttattatgatgcactgtgtttttatgccaaatacccagctttgcccggcactggtggcccactaccacgcacagccttcacaaggtacagaacaggagaaaatggattatgccctcaacaataagaggcgagtcatccgcctggttctacagtgggctgccatgtatggagacctcctgcaagaggatgacgtgtctatggccttcctggaggagttttatgtatctgtatcagatgatgcccggatgattgctgccctcaaggagcaactgccagagttggagaagattgtcaagcaaatctcagaagatgcaaaggcaccacaaaagaagcacaaggttcttttgcaacagttcaatacgggcgatgag

SEQ ID NO: 42 - DNA, 3807 bp, Artificial Sequence
  Synthetic
atggtcgctgcgcacgctgcccattcttcctcctctgccgagtggatcgcctgcctggataaaagaccactggagcgatccagcgaagatgtggatataatcttcactcgactgaaagaagttaaagcttttgagaaatttcacccaaatctccttcatcagatttgcttatgtggttattatgagaatctggaaaagggaataacattatttcgccagggtgatattggaacaaactggtatgctgtcctggcagggtctttggatgttaaagtatctgagaccagcagtcaccaggatgctgtgaccatctgtaccctgggaattgggacggcctttggagagtccattctggacaacacaccccgccatgcaaccatcgttaccagggagagcagtgaactgctccgcatcgagcagaaggacttcaaggcactatgggagaaatatcgacagtatatggcaggacttctggctcctccttatggtgttatggaaacgggctctaacaatgacaggattcctgacaaggagaacacacctctcattgaacctcacgttcctcttcgtcctgctaacaccattaccaaggtcccttcagagaagatcctcagagctggaaaaattttacgaaatgccattctctctcgagcacctcacatgataagagatagaaaataccacctaaagacatacagacaatgctgtgtgggaactgaactggtggactggatgatgcagcagacaccatgtgttcactcccggactcaagctgttggcatgtggcaagtcctgttagaagatggtgttctcaaccacgtggaccaggagcaccatttccaagacaaatatttattctatcgatttctggatgatgagcacgaggatgcccctttgcctactgaggaggagaagaaggagtgtgatgaggagctccaggacaccatgctgctgctgtcacagatgggccccgacgcccacatgaggatgatccttcgcaaaccacctggccagaggactgtggatgacctagagattatctatgaggagcttcttcatattaaagccttatcccatctttctaccacagtgaaacgagagttagcaggtgttctcatttttgagtctcacgccaaaggagggactgtgttgtttaaccagggggaagaaggtacctcctggtacattattctaaaaggatcagtgaatgtagtcatttacggcaagggtgtggtctgcaccctgcatgaaggagatgacttcggcaagttagcactagtgaatgatgccccacgagctgcctctatcgtcttacgagaagataactgccatttcttaagagtagacaaggaggatttcaaccggatcctaagggacgtggaggcgctcgagaacgtctatatcaaggccgacaagcagaagaacggcatcaaggcgaacttcaagatccgccacaacatcgaggacggcggcgtgcagctcgcctaccactaccagcagaacacccccatcggcgacggccccgtgctgctgcccgacaaccactacctgagcgtgcagtccatactttcgaaagaccccaacgagaagcgcgatcacatggtcctgctggagttcgtgaccgccgccgggatcactctcggcatggacgagctgtacaagggcggtaccggagggagcatggtgagcaagggcgaggagctgttcaccggggtggtgcccatccaggtcgagctggacggcgacgtaaacggccacaagttcagcgtgtccggcgagggtgagggcgatgccacctacggcaagctgaccctgaagttcatctgcaccaccggcaagctgcccgtgccctggcccaccctcgtgaccaccctgacctacggcgtgcagtgcttcagccgctaccccgaccacatgaagcagcacgacttcttcaagtccgccatgcccgaaggctacatccaggagcgcaccatcttcttcaaggacgacggcaactacaagacccgcgccgaggtgaagttcgagggcgacaccctggtgaaccgcatcgagctgaagggcatcgacttcaaggaggacggcaacatcctggggcacaagctggagtacaacacgcgtaaggaggatttcaaccggatcctaagggacgtggaggcgaatacagtcagacttaaagaacatgaccaagatgtcttggtgctggagaaggtcccagcagggaacagagcttctaatcaaggaaactcacagcctcagcaaaagtatactgtgatgtcaggaacacctgaaaaaattttagagcattttctagaaacaatacgccttgaggcaactttaaatgaagcaacagattctgttttaaatgactttattatgatgcactgtgtttttatgccaaatacccagctttgcccggcactggtggcccactaccacgcacagccttcacaaggtacagaacaggagaaaatggattatgccctcaacaataagaggcgagtcatccgcctggttctacagtgggctgccatgtatggagacctcctgcaagaggatgacgtgtctatggccttcctggaggagttttatgtatctgtatcagatgatgcccggatgattgctgccctcaaggagcaactgccagagttggagaagattgtcaagcaaatctcagaagatgcaaaggcaccacaaaagaagcacaaggttcttttgcaacagttcaatacgggcgatgagagagcccagaagcgccagcctatccgcggctctgatgaagttctgtttaaggtctattgcatggaccccacctacacaaccattcgggtgccagtggccacttcggtgaaggaagtcatcagtgcagttgccgacaagctgggctccggggagggcctgatcatagtcaagatgagttccggaggagaaaaggtggtgctcaaacctaatgatgtttcagtatttatgacgctcaccattaatggacgcctgtttgcttgcccgcgagagcaattcgattcactgactcccttaccagaacaggaaggcccaactgttggaacagtgggaacttttgaactgatgagctccaaagatttagcataccagatgacaatttatgattgggaactcttcaactgcgtgcatgagctggagctaatctatcacacatttggaaggcataattttaaaaagaccacagcaaacttggatttgttcctgaggagatttaatgaaattcagttttgggtcgtcactgagatctgcctttgttctcagctcagcaagcgtgttcagctattaaaaaaatttattaagatagcagcccactgtaaggagtataaaaatctgaattccttttttgccatcgtcatgggactaagtaacgttgctgtgagccgcttggcactaacgtgggagaaactgccaagcaagttcaagaagttctatgcggagtttgaaagtttaatggacccttcaaggaaccacagggcctacaggctgacagtagctaagctggaacctcctctcatccccttcatgcctttgctcattaaagatatgacatttactcatgaggggaacaagacgttcattgacaatctagtaaactttgaaaaaatgcgcatgattgcaaatacggccagaacagtgagatactacaggagccaacccttcaatcctgatgcagctcaagctaataagaaccatcaggatgtccggagttatgtacggcaattaaatgtgattgacaaccagagaactttatcacagatgtcacacagattagagcctcgtcgacca

SEQ ID NO: 43 - DNA, 2244 bp, Artificial Sequence
  Synthetic
atgggctctaacaatgacaggattcctgacaaggagaacacacctctcattgaacctcacgttcctcttcgtcctgctaacaccattaccaaggtcccttcagagaagatcctcagagctggaaaaattttacgaaatgccattctctctcgagcacctcacatgataagagatagaaaataccacctaaagacatacagacaatgctgtgtgggaactgaactggtggactggatgatgcagcagacaccatgtgttcactcccggactcaagctgttggcatgtggcaagtcctgttagaagatggtgttctcaaccacgtggaccaggagcaccatttccaagacaaatatttattctatcgatttctggatgatgagcacgaggatgcccctttgcctactgaggaggagaagaaggagtgtgatgaggagctccaggacaccatgctgctgctgtcacagatgggccccgacgcccacatgaggatgatccttcgcaaaccacctggccagaggactgtggatgacctagagattatctatgaggagcttcttcatattaaagccttatcccatctttctaccacagtgaaacgagagttagcaggtgttctcatttttgagtctcacgccaaaggagggactgtgttgtttaaccagggggaagaaggtacctcctggtacattattctaaaaggatcagtgaatgtagtcatttacggcaagggtgtggtctgcaccctgcatgaaggagatgacttcggcaagttagcactagtgaatgatgccccacgagctgcctctatcgtcttacgagaagataactgccatttcttaagagtagacaaggaggatttcaaccggatcctaagggacgtggaggcgctcgagaacgtctatatcaaggccgacaagcagaagaacggcatcaaggcgaacttcaagatccgccacaacatcgaggacggcggcgtgcagctcgcctaccactaccagcagaacacccccatcggcgacggccccgtgctgctgcccgacaaccactacctgagcgtgcagtccatactttcgaaagaccccaacgagaagcgcgatcacatggtcctgctggagttcgtgaccgccgccgggatcactctcggcatggacgagctgtacaagggcggtaccggagggagcatggtgagcaagggcgaggagctgttcaccggggtggtgcccatccaggtcgagctggacggcgacgtaaacggccacaagttcagcgtgtccggcgagggtgagggcgatgccacctacggcaagctgaccctgaagttcatctgcaccaccggcaagctgcccgtgccctggcccaccctcgtgaccaccctgacctacggcgtgcagtgcttcagccgctaccccgaccacatgaagcagcacgacttcttcaagtccgccatgcccgaaggctacatccaggagcgcaccatcttcttcaaggacgacggcaactacaagacccgcgccgaggtgaagttcgagggcgacaccctggtgaaccgcatcgagctgaagggcatcgacttcaaggaggacggcaacatcctggggcacaagctggagtacaacacgcgtaaggaggatttcaaccggatcctaagggacgtggaggcgaatacagtcagacttaaagaacatgaccaagatgtcttggtgctggagaaggtcccagcagggaacagagcttctaatcaaggaaactcacagcctcagcaaaagtatactgtgatgtcaggaacacctgaaaaaattttagagcattttctagaaacaatacgccttgaggcaactttaaatgaagcaacagattctgttttaaatgactttattatgatgcactgtgtttttatgccaaatacccagctttgcccggcactggtggcccactaccacgcacagccttcacaaggtacagaacaggagaaaatggattatgccctcaacaataagaggcgagtcatccgcctggttctacagtgggctgccatgtatggagacctcctgcaagaggatgacgtgtctatggccttcctggaggagttttatgtatctgtatcagatgatgcccggatgattgctgccctcaaggagcaactgccagagttggagaagattgtcaagcaaatctcagaagatgcaaaggcaccacaaaagaagcacaaggttcttttgcaacagttcaatacgggcgatgag

SEQ ID NO: 44 - DNA, 3780 bp, Artificial Sequence
  Synthetic
atggtcgctgcgcacgctgcccattcttcctcctctgccgagtggatcgcctgcctggataaaagaccactggagcgatccagcgaagatgtggatataatcttcactcgactgaaagaagttaaagcttttgagaaatttcacccaaatctccttcatcagatttgcttatgtggttattatgagaatctggaaaagggaataacattatttcgccagggtgatattggaacaaactggtatgctgtcctggcagggtctttggatgttaaagtatctgagaccagcagtcaccaggatgctgtgaccatctgtaccctgggaattgggacggcctttggagagtccattctggacaacacaccccgccatgcaaccatcgttaccagggagagcagtgaactgctccgcatcgagcagaaggacttcaaggcactatgggagaaatatcgacagtatatggcaggacttctggctcctccttatggtgttatggaaacgggctctaacaatgacaggattcctgacaaggagaacacacctctcattgaacctcacgttcctcttcgtcctgctaacaccattaccaaggtcccttcagagaagatcctcagagctggaaaaattttacgaaatgccattctctctcgagcacctcacatgataagagatagaaaataccacctaaagacatacagacaatgctgtgtgggaactgaactggtggactggatgatgcagcagacaccatgtgttcactcccggactcaagctgttggcatgtggcaagtcctgttagaagatggtgttctcaaccacgtggaccaggagcaccatttccaagacaaatatttattctatcgatttctggatgatgagcacgaggatgcccctttgcctactgaggaggagaagaaggagtgtgatgaggagctccaggacaccatgctgctgctgtcacagatgggccccgacgcccacatgaggatgatccttcgcaaaccacctggccagaggactgtggatgacctagagattatctatgaggagcttcttcatattaaagccttatcccatctttctaccacagtgaaacgagagttagcaggtgttctcatttttgagtctcacgccaaaggagggactgtgttgtttaaccagggggaagaaggtacctcctggtacattattctaaaaggatcagtgaatgtagtcatttacggcaagggtgtggtctgcaccctgcatgaaggagatgacttcggcaagttagcactagtgaatgatgccccacgagctgcctctatcgtcttacgagaagataactgccatttcttaagagtagacaaggaggatttcaaccggatcctaaggctggtgtcgcacaacgtctatatcaaggccgacaagcagaagaacggcatcaaggcgaacttcaagatccgccacaacatcgaggacggcggcgtgcagctcgcctaccactaccagcagaacacccccatcggcgacggccccgtgctgctgcccgacaaccactacctgagcgtgcagtccatactttcgaaagaccccaacgagaagcgcgatcacatggtcctgctggagttcgtgaccgccgccgggatcactctcggcatggacgagctgtacaagggcggtaccggagggagcatggtgagcaagggcgaggagctgttcaccggggtggtgcccatccaggtcgagctggacggcgacgtaaacggccacaagttcagcgtgtccggcgagggtgagggcgatgccacctacggcaagctgaccctgaagttcatctgcaccaccggcaagctgcccgtgccctggcccaccctcgtgaccaccctgacctacggcgtgcagtgcttcagccgctaccccgaccacatgaagcagcacgacttcttcaagtccgccatgcccgaaggctacatccaggagcgcaccatcttcttcaaggacgacggcaactacaagacccgcgccgaggtgaagttcgagggcgacaccctggtgaaccgcatcgagctgaagggcatcgacttcaaggaggacggcaacatcctggggcacaagctggagtacaacttcaacaaccctgacgtggaggcgaatacagtcagacttaaagaacatgaccaagatgtcttggtgctggagaaggtcccagcagggaacagagcttctaatcaaggaaactcacagcctcagcaaaagtatactgtgatgtcaggaacacctgaaaaaattttagagcattttctagaaacaatacgccttgaggcaactttaaatgaagcaacagattctgttttaaatgactttattatgatgcactgtgtttttatgccaaatacccagctttgcccggcactggtggcccactaccacgcacagccttcacaaggtacagaacaggagaaaatggattatgccctcaacaataagaggcgagtcatccgcctggttctacagtgggctgccatgtatggagacctcctgcaagaggatgacgtgtctatggccttcctggaggagttttatgtatctgtatcagatgatgcccggatgattgctgccctcaaggagcaactgccagagttggagaagattgtcaagcaaatctcagaagatgcaaaggcaccacaaaagaagcacaaggttcttttgcaacagttcaatacgggcgatgagagagcccagaagcgccagcctatccgcggctctgatgaagttctgtttaaggtctattgcatggaccccacctacacaaccattcgggtgccagtggccacttcggtgaaggaagtcatcagtgcagttgccgacaagctgggctccggggagggcctgatcatagtcaagatgagttccggaggagaaaaggtggtgctcaaacctaatgatgtttcagtatttatgacgctcaccattaatggacgcctgtttgcttgcccgcgagagcaattcgattcactgactcccttaccagaacaggaaggcccaactgttggaacagtgggaacttttgaactgatgagctccaaagatttagcataccagatgacaatttatgattgggaactcttcaactgcgtgcatgagctggagctaatctatcacacatttggaaggcataattttaaaaagaccacagcaaacttggatttgttcctgaggagatttaatgaaattcagttttgggtcgtcactgagatctgcctttgttctcagctcagcaagcgtgttcagctattaaaaaaatttattaagatagcagcccactgtaaggagtataaaaatctgaattccttttttgccatcgtcatgggactaagtaacgttgctgtgagccgcttggcactaacgtgggagaaactgccaagcaagttcaagaagttctatgcggagtttgaaagtttaatggacccttcaaggaaccacagggcctacaggctgacagtagctaagctggaacctcctctcatccccttcatgcctttgctcattaaagatatgacatttactcatgaggggaacaagacgttcattgacaatctagtaaactttgaaaaaatgcgcatgattgcaaatacggccagaacagtgagatactacaggagccaacccttcaatcctgatgcagctcaagctaataagaaccatcaggatgtccggagttatgtacggcaattaaatgtgattgacaaccagagaactttatcacagatgtcacacagattagagcctcgtcgacca

SEQ ID NO: 45 - DNA, 3768 bp, Artificial Sequence
  Synthetic
atggtcgctgcgcacgctgcccattcttcctcctctgccgagtggatcgcctgcctggataaaagaccactggagcgatccagcgaagatgtggatataatcttcactcgactgaaagaagttaaagcttttgagaaatttcacccaaatctccttcatcagatttgcttatgtggttattatgagaatctggaaaagggaataacattatttcgccagggtgatattggaacaaactggtatgctgtcctggcagggtctttggatgttaaagtatctgagaccagcagtcaccaggatgctgtgaccatctgtaccctgggaattgggacggcctttggagagtccattctggacaacacaccccgccatgcaaccatcgttaccagggagagcagtgaactgctccgcatcgagcagaaggacttcaaggcactatgggagaaatatcgacagtatatggcaggacttctggctcctccttatggtgttatggaaacgggctctaacaatgacaggattcctgacaaggagaacacacctctcattgaacctcacgttcctcttcgtcctgctaacaccattaccaaggtcccttcagagaagatcctcagagctggaaaaattttacgaaatgccattctctctcgagcacctcacatgataagagatagaaaataccacctaaagacatacagacaatgctgtgtgggaactgaactggtggactggatgatgcagcagacaccatgtgttcactcccggactcaagctgttggcatgtggcaagtcctgttagaagatggtgttctcaaccacgtggaccaggagcaccatttccaagacaaatatttattctatcgatttctggatgatgagcacgaggatgcccctttgcctactgaggaggagaagaaggagtgtgatgaggagctccaggacaccatgctgctgctgtcacagatgggccccgacgcccacatgaggatgatccttcgcaaaccacctggccagaggactgtggatgacctagagattatctatgaggagcttcttcatattaaagccttatcccatctttctaccacagtgaaacgagagttagcaggtgttctcatttttgagtctcacgccaaaggagggactgtgttgtttaaccagggggaagaaggtacctcctggtacattattctaaaaggatcagtgaatgtagtcatttacggcaagggtgtggtctgcaccctgcatgaaggagatgacttcggcaagttagcactagtgaatgatgccccacgagctgcctctatcgtcttacgagaagataactgccatttcttaagagtagacaaggaggatttcaaccggatcctaagggacgtgctcgagaacgtctatatcaaggccgacaagcagaagaacggcatcaaggcgaacttcaagatccgccacaacatcgaggacggcggcgtgcagctcgcctaccactaccagcagaacacccccatcggcgacggccccgtgctgctgcccgacaaccactacctgagcgtgcagtccatactttcgaaagaccccaacgagaagcgcgatcacatggtcctgctggagttcgtgaccgccgccgggatcactctcggcatggacgagctgtacaagggcggtaccggagggagcatggtgagcaagggcgaggagctgttcaccggggtggtgcccatccaggtcgagctggacggcgacgtaaacggccacaagttcagcgtgtccggcgagggtgagggcgatgccacctacggcaagctgaccctgaagttcatctgcaccaccggcaagctgcccgtgccctggcccaccctcgtgaccaccctgacctacggcgtgcagtgcttcagccgctaccccgaccacatgaagcagcacgacttcttcaagtccgccatgcccgaaggctacatccaggagcgcaccatcttcttcaaggacgacggcaactacaagacccgcgccgaggtgaagttcgagggcgacaccctggtgaaccgcatcgagctgaagggcatcgacttcaaggaggacggcaacatcctggggcacaagctggagtacaacacgcgtgaggcgaatacagtcagacttaaagaacatgaccaagatgtcttggtgctggagaaggtcccagcagggaacagagcttctaatcaaggaaactcacagcctcagcaaaagtatactgtgatgtcaggaacacctgaaaaaattttagagcattttctagaaacaatacgccttgaggcaactttaaatgaagcaacagattctgttttaaatgactttattatgatgcactgtgtttttatgccaaatacccagctttgcccggcactggtggcccactaccacgcacagccttcacaaggtacagaacaggagaaaatggattatgccctcaacaataagaggcgagtcatccgcctggttctacagtgggctgccatgtatggagacctcctgcaagaggatgacgtgtctatggccttcctggaggagttttatgtatctgtatcagatgatgcccggatgattgctgccctcaaggagcaactgccagagttggagaagattgtcaagcaaatctcagaagatgcaaaggcaccacaaaagaagcacaaggttcttttgcaacagttcaatacgggcgatgagagagcccagaagcgccagcctatccgcggctctgatgaagttctgtttaaggtctattgcatggaccccacctacacaaccattcgggtgccagtggccacttcggtgaaggaagtcatcagtgcagttgccgacaagctgggctccggggagggcctgatcatagtcaagatgagttccggaggagaaaaggtggtgctcaaacctaatgatgtttcagtatttatgacgctcaccattaatggacgcctgtttgcttgcccgcgagagcaattcgattcactgactcccttaccagaacaggaaggcccaactgttggaacagtgggaacttttgaactgatgagctccaaagatttagcataccagatgacaatttatgattgggaactcttcaactgcgtgcatgagctggagctaatctatcacacatttggaaggcataattttaaaaagaccacagcaaacttggatttgttcctgaggagatttaatgaaattcagttttgggtcgtcactgagatctgcctttgttctcagctcagcaagcgtgttcagctattaaaaaaatttattaagatagcagcccactgtaaggagtataaaaatctgaattccttttttgccatcgtcatgggactaagtaacgttgctgtgagccgcttggcactaacgtgggagaaactgccaagcaagttcaagaagttctatgcggagtttgaaagtttaatggacccttcaaggaaccacagggcctacaggctgacagtagctaagctggaacctcctctcatccccttcatgcctttgctcattaaagatatgacatttactcatgaggggaacaagacgttcattgacaatctagtaaactttgaaaaaatgcgcatgattgcaaatacggccagaacagtgagatactacaggagccaacccttcaatcctgatgcagctcaagctaataagaaccatcaggatgtccggagttatgtacggcaattaaatgtgattgacaaccagagaactttatcacagatgtcacacagattagagcctcgtcgacca

SEQ ID NO: 46 - DNA, 1605 bp, Artificial Sequence
  Synthetic
atgggctctaacaatgacaggattcctgacaaggagaacacacctctcattgaacctcacgttcctcttcgtcctgctaacaccattaccaaggtcccttcagagaagatcctcagagctggaaaaattttacgaaatgccattctctctcgagcacctcacatgataagagatagaaaataccacctaaagacatacagacaatgctgtgtgggaactgaactggtggactggatgatgcagcagacaccatgtgttcactcccggactcaagctgttggcatgtggcaagtcctgttagaagatggtgttctcaaccacgtggaccaggagcaccatttccaagacaaatatttattctatcgatttctggatgatgagcacgaggatgcccctttgcctactgaggaggagaagaaggagtgtgatgaggagctccaggacaccatgctgctgctgtcacagatgggccccgacgcccacatgaggatgatccttcgcaaaccacctggccagaggactgtggatgacctagagattatctatgaggagcttcttcatattaaagccttatcccatctttctaccacagtgaaacgagagttagcaggtgttctcatttttgagtctcacgccaaaggagggactgtgttgtttaaccagggggaagaaggtacctcctggtacattattctaaaaggatcagtgaatgtagtcatttacggcaagggtgtggtctgcaccctgcatgaaggagatgacttcggcaagttagcactagtgaatgatgccccacgagctgcctctatcgtcttacgagaagataactgccatttcttaagagtagacaaggaggatttcaaccggatcctaaggcgtgcgaacgtctatatcaaggccgacaagcagaagaacggcatcaaggcgaacttcaagatccgccacaacatcgaggacggcggcgtgcagctcgcctaccactaccagcagaacacccccatcggcgacggccccgtgctgctgcccgacaaccactacctgagcgtgcagtccatactttcgaaagaccccaacgagaagcgcgatcacatggtcctgctggagttcgtgaccgccgccgggatcactctcggcatggacgagctgtacaagggcggtaccggagggagcatggtgagcaagggcgaggagctgttcaccggggtggtgcccatccaggtcgagctggacggcgacgtaaacggccacaagttcagcgtgtccggcgagggtgagggcgatgccacctacggcaagctgaccctgaagttcatctgcaccaccggcaagctgcccgtgccctggcccaccctcgtgaccaccctgacctacggcgtgcagtgcttcagccgctaccccgaccacatgaagcagcacgacttcttcaagtccgccatgcccgaaggctacatccaggagcgcaccatcttcttcaaggacgacggcaactacaagacccgcgccgaggtgaagttcgagggcgacaccctggtgaaccgcatcgagctgaagggcatcgacttcaaggaggacggcaacatcctggggcacaagctggagtacaac

SEQ ID NO: 47 - DNA, 3795 bp, Artificial Sequence
  Synthetic
atggtcgctgcgcacgctgcccattcttcctcctctgccgagtggatcgcctgcctggataaaagaccactggagcgatccagcgaagatgtggatataatcttcactcgactgaaagaagttaaagcttttgagaaatttcacccaaatctccttcatcagatttgcttatgtggttattatgagaatctggaaaagggaataacattatttcgccagggtgatattggaacaaactggtatgctgtcctggcagggtctttggatgttaaagtatctgagaccagcagtcaccaggatgctgtgaccatctgtaccctgggaattgggacggcctttggagagtccattctggacaacacaccccgccatgcaaccatcgttaccagggagagcagtgaactgctccgcatcgagcagaaggacttcaaggcactatgggagaaatatcgacagtatatggcaggacttctggctcctccttatggtgttatggaaacgggctctaacaatgacaggattcctgacaaggagaacacacctctcattgaacctcacgttcctcttcgtcctgctaacaccattaccaaggtcccttcagagaagatcctcagagctggaaaaattttacgaaatgccattctctctcgagcacctcacatgataagagatagaaaataccacctaaagacatacagacaatgctgtgtgggaactgaactggtggactggatgatgcagcagacaccatgtgttcactcccggactcaagctgttggcatgtggcaagtcctgttagaagatggtgttctcaaccacgtggaccaggagcaccatttccaagacaaatatttattctatcgatttctggatgatgagcacgaggatgcccctttgcctactgaggaggagaagaaggagtgtgatgaggagctccaggacaccatgctgctgctgtcacagatgggccccgacgcccacatgaggatgatccttcgcaaaccacctggccagaggactgtggatgacctagagattatctatgaggagcttcttcatattaaagccttatcccatctttctaccacagtgaaacgagagttagcaggtgttctcatttttgagtctcacgccaaaggagggactgtgttgtttaaccagggggaagaaggtacctcctggtacattattctaaaaggatcagtgaatgtagtcatttacggcaagggtgtggtctgcaccctgcatgaaggagatgacttcggcaagttagcactagtgaatgatgccccacgagctgcctctatcgtcttacgagaagataactgccatttcttaagagtagacaaggaggatttcaaccggatcctaaggctcgagaacgtctatatcaaggccgacaagcagaagaacggcatcaaggcgaacttcaagatccgccacaacatcgaggacggcggcgtgcagctcgcctaccactaccagcagaacacccccatcggcgacggccccgtgctgctgcccgacaaccactacctgagcgtgcagtccatactttcgaaagaccccaacgagaagcgcgatcacatggtcctgctggagttcgtgaccgccgccgggatcactctcggcatggacgagctgtacaagggcggtaccggagggagcatggtgagcaagggcgaggagctgttcaccggggtggtgcccatccaggtcgagctggacggcgacgtaaacggccacaagttcagcgtgtccggcgagggtgagggcgatgccacctacggcaagctgaccctgaagttcatctgcaccaccggcaagctgcccgtgccctggcccaccctcgtgaccaccctgacctacggcgtgcagtgcttcagccgctaccccgaccacatgaagcagcacgacttcttcaagtccgccatgcccgaaggctacatccaggagcgcaccatcttcttcaaggacgacggcaactacaagacccgcgccgaggtgaagttcgagggcgacaccctggtgaaccgcatcgagctgaagggcatcgacttcaaggaggacggcaacatcctggggcacaagctggagtacaacacgcgtaaggaggatttcaaccggatcctaagggacgtggaggcgaatacagtcagacttaaagaacatgaccaagatgtcttggtgctggagaaggtcccagcagggaacagagcttctaatcaaggaaactcacagcctcagcaaaagtatactgtgatgtcaggaacacctgaaaaaattttagagcattttctagaaacaatacgccttgaggcaactttaaatgaagcaacagattctgttttaaatgactttattatgatgcactgtgtttttatgccaaatacccagctttgcccggcactggtggcccactaccacgcacagccttcacaaggtacagaacaggagaaaatggattatgccctcaacaataagaggcgagtcatccgcctggttctacagtgggctgccatgtatggagacctcctgcaagaggatgacgtgtctatggccttcctggaggagttttatgtatctgtatcagatgatgcccggatgattgctgccctcaaggagcaactgccagagttggagaagattgtcaagcaaatctcagaagatgcaaaggcaccacaaaagaagcacaaggttcttttgcaacagttcaatacgggcgatgagagagcccagaagcgccagcctatccgcggctctgatgaagttctgtttaaggtctattgcatggaccccacctacacaaccattcgggtgccagtggccacttcggtgaaggaagtcatcagtgcagttgccgacaagctgggctccggggagggcctgatcatagtcaagatgagttccggaggagaaaaggtggtgctcaaacctaatgatgtttcagtatttatgacgctcaccattaatggacgcctgtttgcttgcccgcgagagcaattcgattcactgactcccttaccagaacaggaaggcccaactgttggaacagtgggaacttttgaactgatgagctccaaagatttagcataccagatgacaatttatgattgggaactcttcaactgcgtgcatgagctggagctaatctatcacacatttggaaggcataattttaaaaagaccacagcaaacttggatttgttcctgaggagatttaatgaaattcagttttgggtcgtcactgagatctgcctttgttctcagctcagcaagcgtgttcagctattaaaaaaatttattaagatagcagcccactgtaaggagtataaaaatctgaattccttttttgccatcgtcatgggactaagtaacgttgctgtgagccgcttggcactaacgtgggagaaactgccaagcaagttcaagaagttctatgcggagtttgaaagtttaatggacccttcaaggaaccacagggcctacaggctgacagtagctaagctggaacctcctctcatccccttcatgcctttgctcattaaagatatgacatttactcatgaggggaacaagacgttcattgacaatctagtaaactttgaaaaaatgcgcatgattgcaaatacggccagaacagtgagatactacaggagccaacccttcaatcctgatgcagctcaagctaataagaaccatcaggatgtccggagttatgtacggcaattaaatgtgattgacaaccagagaactttatcacagatgtcacacagattagagcctcgtcgacca

SEQ ID NO: 48 - DNA, 3771 bp, Artificial Sequence
  Synthetic
atggtcgctgcgcacgctgcccattcttcctcctctgccgagtggatcgcctgcctggataaaagaccactggagcgatccagcgaagatgtggatataatcttcactcgactgaaagaagttaaagcttttgagaaatttcacccaaatctccttcatcagatttgcttatgtggttattatgagaatctggaaaagggaataacattatttcgccagggtgatattggaacaaactggtatgctgtcctggcagggtctttggatgttaaagtatctgagaccagcagtcaccaggatgctgtgaccatctgtaccctgggaattgggacggcctttggagagtccattctggacaacacaccccgccatgcaaccatcgttaccagggagagcagtgaactgctccgcatcgagcagaaggacttcaaggcactatgggagaaatatcgacagtatatggcaggacttctggctcctccttatggtgttatggaaacgggctctaacaatgacaggattcctgacaaggagaacacacctctcattgaacctcacgttcctcttcgtcctgctaacaccattaccaaggtcccttcagagaagatcctcagagctggaaaaattttacgaaatgccattctctctcgagcacctcacatgataagagatagaaaataccacctaaagacatacagacaatgctgtgtgggaactgaactggtggactggatgatgcagcagacaccatgtgttcactcccggactcaagctgttggcatgtggcaagtcctgttagaagatggtgttctcaaccacgtggaccaggagcaccatttccaagacaaatatttattctatcgatttctggatgatgagcacgaggatgcccctttgcctactgaggaggagaagaaggagtgtgatgaggagctccaggacaccatgctgctgctgtcacagatgggccccgacgcccacatgaggatgatccttcgcaaaccacctggccagaggactgtggatgacctagagattatctatgaggagcttcttcatattaaagccttatcccatctttctaccacagtgaaacgagagttagcaggtgttctcatttttgagtctcacgccaaaggagggactgtgttgtttaaccagggggaagaaggtacctcctggtacattattctaaaaggatcagtgaatgtagtcatttacggcaagggtgtggtctgcaccctgcatgaaggagatgacttcggcaagttagcactagtgaatgatgccccacgagctgcctctatcgtcttacgagaagataactgccatttcttaagagtagacaaggaggatttcaaccggatcctaagggacgtgctcgagaacgtctatatcaaggccgacaagcagaagaacggcatcaaggcgaacttcaagatccgccacaacatcgaggacggcggcgtgcagctcgcctaccactaccagcagaacacccccatcggcgacggccccgtgctgctgcccgacaaccactacctgagcgtgcagtccatactttcgaaagaccccaacgagaagcgcgatcacatggtcctgctggagttcgtgaccgccgccgggatcactctcggcatggacgagctgtacaagggcggtaccggagggagcatggtgagcaagggcgaggaggtttcctccgggggggtgcccatccaggtcgagctggacggcgacgtaaacggccacaagttcagcgtgtccggcgagggtgagggcgatgccacctacggcaagctgaccctgaagttcatctgcaccaccggcaagctgcccgtgccctggcccaccctcgtgaccaccctgacctacggcgtgcagtgcttcagccgctaccccgaccacatgaagcagcacgacttcttcaagtccgccatgcccgaaggctacatccaggagcgcaccatcttcttcaaggacgacggcaactacaagacccgcgccgaggtgaagttcgagggcgacaccctggtgaaccgcatcgagctgaagggcatcgacttcaaggaggacggcaacatcctggggcacaagctggagtacaacacgcgtgtggaggcgaatacagtcagacttaaagaacatgaccaagatgtcttggtgctggagaaggtcccagcagggaacagagcttctaatcaaggaaactcacagcctcagcaaaagtatactgtgatgtcaggaacacctgaaaaaattttagagcattttctagaaacaatacgccttgaggcaactttaaatgaagcaacagattctgttttaaatgactttattatgatgcactgtgtttttatgccaaatacccagctttgcccggcactggtggcccactaccacgcacagccttcacaaggtacagaacaggagaaaatggattatgccctcaacaataagaggcgagtcatccgcctggttctacagtgggctgccatgtatggagacctcctgcaagaggatgacgtgtctatggccttcctggaggagttttatgtatctgtatcagatgatgcccggatgattgctgccctcaaggagcaactgccagagttggagaagattgtcaagcaaatctcagaagatgcaaaggcaccacaaaagaagcacaaggttcttttgcaacagttcaatacgggcgatgagagagcccagaagcgccagcctatccgcggctctgatgaagttctgtttaaggtctattgcatggaccccacctacacaaccattcgggtgccagtggccacttcggtgaaggaagtcatcagtgcagttgccgacaagctgggctccggggagggcctgatcatagtcaagatgagttccggaggagaaaaggtggtgctcaaacctaatgatgtttcagtatttatgacgctcaccattaatggacgcctgtttgcttgcccgcgagagcaattcgattcactgactcccttaccagaacaggaaggcccaactgttggaacagtgggaacttttgaactgatgagctccaaagatttagcataccagatgacaatttatgattgggaactcttcaactgcgtgcatgagctggagctaatctatcacacatttggaaggcataattttaaaaagaccacagcaaacttggatttgttcctgaggagatttaatgaaattcagttttgggtcgtcactgagatctgcctttgttctcagctcagcaagcgtgttcagctattaaaaaaatttattaagatagcagcccactgtaaggagtataaaaatctgaattccttttttgccatcgtcatgggactaagtaacgttgctgtgagccgcttggcactaacgtgggagaaactgccaagcaagttcaagaagttctatgcggagtttgaaagtttaatggacccttcaaggaaccacagggcctacaggctgacagtagctaagctggaacctcctctcatccccttcatgcctttgctcattaaagatatgacatttactcatgaggggaacaagacgttcattgacaatctagtaaactttgaaaaaatgcgcatgattgcaaatacggccagaacagtgagatactacaggagccaacccttcaatcctgatgcagctcaagctaataagaaccatcaggatgtccggagttatgtacggcaattaaatgtgattgacaaccagagaactttatcacagatgtcacacagattagagcctcgtcgacca

SEQ ID NO: 49 - DNA, 3765 bp, Artificial Sequence
  Synthetic
atggtcgctgcgcacgctgcccattcttcctcctctgccgagtggatcgcctgcctggataaaagaccactggagcgatccagcgaagatgtggatataatcttcactcgactgaaagaagttaaagcttttgagaaatttcacccaaatctccttcatcagatttgcttatgtggttattatgagaatctggaaaagggaataacattatttcgccagggtgatattggaacaaactggtatgctgtcctggcagggtctttggatgttaaagtatctgagaccagcagtcaccaggatgctgtgaccatctgtaccctgggaattgggacggcctttggagagtccattctggacaacacaccccgccatgcaaccatcgttaccagggagagcagtgaactgctccgcatcgagcagaaggacttcaaggcactatgggagaaatatcgacagtatatggcaggacttctggctcctccttatggtgttatggaaacgggctctaacaatgacaggattcctgacaaggagaacacacctctcattgaacctcacgttcctcttcgtcctgctaacaccattaccaaggtcccttcagagaagatcctcagagctggaaaaattttacgaaatgccattctctctcgagcacctcacatgataagagatagaaaataccacctaaagacatacagacaatgctgtgtgggaactgaactggtggactggatgatgcagcagacaccatgtgttcactcccggactcaagctgttggcatgtggcaagtcctgttagaagatggtgttctcaaccacgtggaccaggagcaccatttccaagacaaatatttattctatcgatttctggatgatgagcacgaggatgcccctttgcctactgaggaggagaagaaggagtgtgatgaggagctccaggacaccatgctgctgctgtcacagatgggccccgacgcccacatgaggatgatccttcgcaaaccacctggccagaggactgtggatgacctagagattatctatgaggagcttcttcatattaaagccttatcccatctttctaccacagtgaaacgagagttagcaggtgttctcatttttgagtctcacgccaaaggagggactgtgttgtttaaccagggggaagaaggtacctcctggtacattattctaaaaggatcagtgaatgtagtcatttacggcaagggtgtggtctgcaccctgcatgaaggagatgacttcggcaagttagcactagtgaatgatgccccacgagctgcctctatcgtcttacgagaagataactgccatttcttaagagtagacaaggaggatttcaaccggatcctaagggacgtgctcgagaacgtctatatcaaggccgacaagcagaagaacggcatcaaggcgaacttcaagatccgccacaacatcgaggacggcggcgtgcagctcgcctaccactaccagcagaacacccccatcggcgacggccccgtgctgctgcccgacaaccactacctgagcgtgcagtccatactttcgaaagaccccaacgagaagcgcgatcacatggtcctgctggagttcgtgaccgccgccgggatcactctcggcatggacgagctgtacaagggcggtaccggagggagcatggtgagcaagggcgaggagctgttcaccggggtggtgcccatccaggtcgagctggacggcgacgtaaacggccacaagttcagcgtgtccggcgagggtgagggcgatgccacctacggcaagctgaccctgaagttcatctgcaccaccggcaagctgcccgtgccctggcccaccctcgtgaccaccctgacctacggcgtgcagtgcttcagccgctaccccgaccacatgaagcagcacgacttcttcaagtccgccatgcccgaaggctacatccaggagcgcaccatcttcttcaaggacgacggcaactacaagacccgcgccgaggtgaagttcgagggcgacaccctggtgaaccgcatcgagctgaagggcatcgacttcaaggaggacggcaacatcctggggcacaagctggagtacaacacgcgtgcgaatacagtcagacttaaagaacatgaccaagatgtcttggtgctggagaaggtcccagcagggaacagagcttctaatcaaggaaactcacagcctcagcaaaagtatactgtgatgtcaggaacacctgaaaaaattttagagcattttctagaaacaatacgccttgaggcaactttaaatgaagcaacagattctgttttaaatgactttattatgatgcactgtgtttttatgccaaatacccagctttgcccggcactggtggcccactaccacgcacagccttcacaaggtacagaacaggagaaaatggattatgccctcaacaataagaggcgagtcatccgcctggttctacagtgggctgccatgtatggagacctcctgcaagaggatgacgtgtctatggccttcctggaggagttttatgtatctgtatcagatgatgcccggatgattgctgccctcaaggagcaactgccagagttggagaagattgtcaagcaaatctcagaagatgcaaaggcaccacaaaagaagcacaaggttcttttgcaacagttcaatacgggcgatgagagagcccagaagcgccagcctatccgcggctctgatgaagttctgtttaaggtctattgcatggaccccacctacacaaccattcgggtgccagtggccacttcggtgaaggaagtcatcagtgcagttgccgacaagctgggctccggggagggcctgatcatagtcaagatgagttccggaggagaaaaggtggtgctcaaacctaatgatgtttcagtatttatgacgctcaccattaatggacgcctgtttgcttgcccgcgagagcaattcgattcactgactcccttaccagaacaggaaggcccaactgttggaacagtgggaacttttgaactgatgagctccaaagatttagcataccagatgacaatttatgattgggaactcttcaactgcgtgcatgagctggagctaatctatcacacatttggaaggcataattttaaaaagaccacagcaaacttggatttgttcctgaggagatttaatgaaattcagttttgggtcgtcactgagatctgcctttgttctcagctcagcaagcgtgttcagctattaaaaaaatttattaagatagcagcccactgtaaggagtataaaaatctgaattccttttttgccatcgtcatgggactaagtaacgttgctgtgagccgcttggcactaacgtgggagaaactgccaagcaagttcaagaagttctatgcggagtttgaaagtttaatggacccttcaaggaaccacagggcctacaggctgacagtagctaagctggaacctcctctcatccccttcatgcctttgctcattaaagatatgacatttactcatgaggggaacaagacgttcattgacaatctagtaaactttgaaaaaatgcgcatgattgcaaatacggccagaacagtgagatactacaggagccaacccttcaatcctgatgcagctcaagctaataagaaccatcaggatgtccggagttatgtacggcaattaaatgtgattgacaaccagagaactttatcacagatgtcacacagattagagcctcgtcgacca

SEQ ID NO: 50 - DNA, 3780 bp, Artificial Sequence
  Synthetic
atggtcgctgcgcacgctgcccattcttcctcctctgccgagtggatcgcctgcctggataaaagaccactggagcgatccagcgaagatgtggatataatcttcactcgactgaaagaagttaaagcttttgagaaatttcacccaaatctccttcatcagatttgcttatgtggttattatgagaatctggaaaagggaataacattatttcgccagggtgatattggaacaaactggtatgctgtcctggcagggtctttggatgttaaagtatctgagaccagcagtcaccaggatgctgtgaccatctgtaccctgggaattgggacggcctttggagagtccattctggacaacacaccccgccatgcaaccatcgttaccagggagagcagtgaactgctccgcatcgagcagaaggacttcaaggcactatgggagaaatatcgacagtatatggcaggacttctggctcctccttatggtgttatggaaacgggctctaacaatgacaggattcctgacaaggagaacacacctctcattgaacctcacgttcctcttcgtcctgctaacaccattaccaaggtcccttcagagaagatcctcagagctggaaaaattttacgaaatgccattctctctcgagcacctcacatgataagagatagaaaataccacctaaagacatacagacaatgctgtgtgggaactgaactggtggactggatgatgcagcagacaccatgtgttcactcccggactcaagctgttggcatgtggcaagtcctgttagaagatggtgttctcaaccacgtggaccaggagcaccatttccaagacaaatatttattctatcgatttctggatgatgagcacgaggatgcccctttgcctactgaggaggagaagaaggagtgtgatgaggagctccaggacaccatgctgctgctgtcacagatgggccccgacgcccacatgaggatgatccttcgcaaaccacctggccagaggactgtggatgacctagagattatctatgaggagcttcttcatattaaagccttatcccatctttctaccacagtgaaacgagagttagcaggtgttctcatttttgagtctcacgccaaaggagggactgtgttgtttaaccagggggaagaaggtacctcctggtacattattctaaaaggatcagtgaatgtagtcatttacggcaagggtgtggtctgcaccctgcatgaaggagatgacttcggcaagttagcactagtgaatgatgccccacgagctgcctctatcgtcttacgagaagataactgccatttcttaagagtagacaaggaggatttcaaccggatcctaaggctcgagaacgtctatatcaaggccgacaagcagaagaacggcatcaaggcgaacttcaagatccgccacaacatcgaggacggcggcgtgcagctcgcctaccactaccagcagaacacccccatcggcgacggccccgtgctgctgcccgacaaccactacctgagcgtgcagtccatactttcgaaagaccccaacgagaagcgcgatcacatggtcctgctggagttcgtgaccgccgccgggatcactctcggcatggacgagctgtacaagggcggtaccggagggagcatggtgagcaagggcgaggagctgttcaccggggtggtgcccatccaggtcgagctggacggcgacgtaaacggccacaagttcagcgtgtccggcgagggtgagggcgatgccacctacggcaagctgaccctgaagttcatctgcaccaccggcaagctgcccgtgccctggcccaccctcgtgaccaccctgacctacggcgtgcagtgcttcagccgctaccccgaccacatgaagcagcacgacttcttcaagtccgccatgcccgaaggctacatccaggagcgcaccatcttcttcaaggacgacggcaactacaagacccgcgccgaggtgaagttcgagggcgacaccctggtgaaccgcatcgagctgaagggcatcgacttcaaggaggacggcaacatcctggggcacaagctggagtacaacacgcgtcggatcctaagggacgtggaggcgaatacagtcagacttaaagaacatgaccaagatgtcttggtgctggagaaggtcccagcagggaacagagcttctaatcaaggaaactcacagcctcagcaaaagtatactgtgatgtcaggaacacctgaaaaaattttagagcattttctagaaacaatacgccttgaggcaactttaaatgaagcaacagattctgttttaaatgactttattatgatgcactgtgtttttatgccaaatacccagctttgcccggcactggtggcccactaccacgcacagccttcacaaggtacagaacaggagaaaatggattatgccctcaacaataagaggcgagtcatccgcctggttctacagtgggctgccatgtatggagacctcctgcaagaggatgacgtgtctatggccttcctggaggagttttatgtatctgtatcagatgatgcccggatgattgctgccctcaaggagcaactgccagagttggagaagattgtcaagcaaatctcagaagatgcaaaggcaccacaaaagaagcacaaggttcttttgcaacagttcaatacgggcgatgagagagcccagaagcgccagcctatccgcggctctgatgaagttctgtttaaggtctattgcatggaccccacctacacaaccattcgggtgccagtggccacttcggtgaaggaagtcatcagtgcagttgccgacaagctgggctccggggagggcctgatcatagtcaagatgagttccggaggagaaaaggtggtgctcaaacctaatgatgtttcagtatttatgacgctcaccattaatggacgcctgtttgcttgcccgcgagagcaattcgattcactgactcccttaccagaacaggaaggcccaactgttggaacagtgggaacttttgaactgatgagctccaaagatttagcataccagatgacaatttatgattgggaactcttcaactgcgtgcatgagctggagctaatctatcacacatttggaaggcataattttaaaaagaccacagcaaacttggatttgttcctgaggagatttaatgaaattcagttttgggtcgtcactgagatctgcctttgttctcagctcagcaagcgtgttcagctattaaaaaaatttattaagatagcagcccactgtaaggagtataaaaatctgaattccttttttgccatcgtcatgggactaagtaacgttgctgtgagccgcttggcactaacgtgggagaaactgccaagcaagttcaagaagttctatgcggagtttgaaagtttaatggacccttcaaggaaccacagggcctacaggctgacagtagctaagctggaacctcctctcatccccttcatgcctttgctcattaaagatatgacatttactcatgaggggaacaagacgttcattgacaatctagtaaactttgaaaaaatgcgcatgattgcaaatacggccagaacagtgagatactacaggagccaacccttcaatcctgatgcagctcaagctaataagaaccatcaggatgtccggagttatgtacggcaattaaatgtgattgacaaccagagaactttatcacagatgtcacacagattagagcctcgtcgacca

SEQ ID NO: 51 - DNA, 3768 bp, Artificial Sequence; identical to SEQ ID NO: 45
  Synthetic

SEQ ID NO: 52 - DNA, 3789 bp, Artificial Sequence
  Synthetic
atggtcgctgcgcacgctgcccattcttcctcctctgccgagtggatcgcctgcctggataaaagaccactggagcgatccagcgaagatgtggatataatcttcactcgactgaaagaagttaaagcttttgagaaatttcacccaaatctccttcatcagatttgcttatgtggttattatgagaatctggaaaagggaataacattatttcgccagggtgatattggaacaaactggtatgctgtcctggcagggtctttggatgttaaagtatctgagaccagcagtcaccaggatgctgtgaccatctgtaccctgggaattgggacggcctttggagagtccattctggacaacacaccccgccatgcaaccatcgttaccagggagagcagtgaactgctccgcatcgagcagaaggacttcaaggcactatgggagaaatatcgacagtatatggcaggacttctggctcctccttatggtgttatggaaacgggctctaacaatgacaggattcctgacaaggagaacacacctctcattgaacctcacgttcctcttcgtcctgctaacaccattaccaaggtcccttcagagaagatcctcagagctggaaaaattttacgaaatgccattctctctcgagcacctcacatgataagagatagaaaataccacctaaagacatacagacaatgctgtgtgggaactgaactggtggactggatgatgcagcagacaccatgtgttcactcccggactcaagctgttggcatgtggcaagtcctgttagaagatggtgttctcaaccacgtggaccaggagcaccatttccaagacaaatatttattctatcgatttctggatgatgagcacgaggatgcccctttgcctactgaggaggagaagaaggagtgtgatgaggagctccaggacaccatgctgctgctgtcacagatgggccccgacgcccacatgaggatgatccttcgcaaaccacctggccagaggactgtggatgacctagagattatctatgaggagcttcttcatattaaagccttatcccatctttctaccacagtgaaacgagagttagcaggtgttctcatttttgagtctcacgccaaaggagggactgtgttgtttaaccagggggaagaaggtacctcctggtacattattctaaaaggatcagtgaatgtagtcatttacggcaagggtgtggtctgcaccctgcatgaaggagatgacttcggcaagttagcactagtgaatgatgccccacgagctgcctctatcgtcttacgagaagataactgccatttcttaagagtagacaaggaggatttcaaccggatcctaagggacctcgagaacgtctatatcaaggccgacaagcagaagaacggcatcaaggcgaacttcaagatccgccacaacatcgaggacggcggcgtgcagctcgcctaccactaccagcagaacacccccatcggcgacggccccgtgctgctgcccgacaaccactacctgagcgtgcagtccatactttcgaaagaccccaacgagaagcgcgatcacatggtcctgctggagttcgtgaccgccgccgggatcactctcggcatggacgagctgtacaagggcggtaccggagggagcatggtgagcaagggcgaggagctgttcaccggggtggtgcccatccaggtcgagctggacggcgacgtaaacggccacaagttcagcgtgtccggcgagggtgagggcgatgccacctacggcaagctgaccctgaagttcatctgcaccaccggcaagctgcccgtgccctggcccaccctcgtgaccaccctgacctacggcgtgcagtgcttcagccgctaccccgaccacatgaagcagcacgacttcttcaagtccgccatgcccgaaggctacatccaggagcgcaccatcttcttcaaggacgacggcaactacaagacccgcgccgaggtgaagttcgagggcgacaccctggtgaaccgcatcgagctgaagggcatcgacttcaaggaggacggcaacatcctggggcacaagctggagtacaacacgcgtttcaaccggatcctaagggacgtggaggcgaatacagtcagacttaaagaacatgaccaagatgtcttggtgctggagaaggtcccagcagggaacagagcttctaatcaaggaaactcacagcctcagcaaaagtatactgtgatgtcaggaacacctgaaaaaattttagagcattttctagaaacaatacgccttgaggcaactttaaatgaagcaacagattctgttttaaatgactttattatgatgcactgtgtttttatgccaaatacccagctttgcccggcactggtggcccactaccacgcacagccttcacaaggtacagaacaggagaaaatggattatgccctcaacaataagaggcgagtcatccgcctggttctacagtgggctgccatgtatggagacctcctgcaagaggatgacgtgtctatggccttcctggaggagttttatgtatctgtatcagatgatgcccggatgattgctgccctcaaggagcaactgccagagttggagaagattgtcaagcaaatctcagaagatgcaaaggcaccacaaaagaagcacaaggttcttttgcaacagttcaatacgggcgatgagagagcccagaagcgccagcctatccgcggctctgatgaagttctgtttaaggtctattgcatggaccccacctacacaaccattcgggtgccagtggccacttcggtgaaggaagtcatcagtgcagttgccgacaagctgggctccggggagggcctgatcatagtcaagatgagttccggaggagaaaaggtggtgctcaaacctaatgatgtttcagtatttatgacgctcaccattaatggacgcctgtttgcttgcccgcgagagcaattcgattcactgactcccttaccagaacaggaaggcccaactgttggaacagtgggaacttttgaactgatgagctccaaagatttagcataccagatgacaatttatgattgggaactcttcaactgcgtgcatgagctggagctaatctatcacacatttggaaggcataattttaaaaagaccacagcaaacttggatttgttcctgaggagatttaatgaaattcagttttgggtcgtcactgagatctgcctttgttctcagctcagcaagcgtgttcagctattaaaaaaatttattaagatagcagcccactgtaaggagtataaaaatctgaattccttttttgccatcgtcatgggactaagtaacgttgctgtgagccgcttggcactaacgtgggagaaactgccaagcaagttcaagaagttctatgcggagtttgaaagtttaatggacccttcaaggaaccacagggcctacaggctgacagtagctaagctggaacctcctctcatccccttcatgcctttgctcattaaagatatgacatttactcatgaggggaacaagacgttcattgacaatctagtaaactttgaaaaaatgcgcatgattgcaaatacggccagaacagtgagatactacaggagccaacccttcaatcctgatgcagctcaagctaataagaaccatcaggatgtccggagttatgtacggcaattaaatgtgattgacaaccagagaactttatcacagatgtcacacagattagagcctcgtcgacca

SEQ ID NO: 53 - DNA, 3764 bp, Artificial Sequence
  Synthetic
atggtcgctgcgcacgctgcccattcttcctcctctgccgagtggatcgcctgcctggataaaagaccactggagcgatccagcgaagatgtggatataatcttcactcgactgaaagaagttaaagcttttgagaaatttcacccaaatctccttcatcagatttgcttatgtggttattatgagaatctggaaaagggaataacattatttcgccagggtgatattggaacaaactggtatgctgtcctggcagggtctttggatgttaaagtatctgagaccagcagtcaccaggatgctgtgaccatctgtaccctgggaattgggacggcctttggagagtccattctggacaacacaccccgccatgcaaccatcgttaccagggagagcagtgaactgctccgcatcgagcagaaggacttcaaggcactatgggagaaatatcgacagtatatggcaggacttctggctcctccttatggtgttatggaaacgggctctaacaatgacaggattcctgacaaggagaacacacctctcattgaacctcacgttcctcttcgtcctgctaacaccattaccaaggtcccttcagagaagatcctcagagctggaaaaattttacgaaatgccattctctctcgagcacctcacatgataagagatagaaaataccacctaaagacatacagacaatgctgtgtgggaactgaactggtggactggatgatgcagcagacaccatgtgttcactcccggactcaagctgttggcatgtggcaagtcctgttagaagatggtgttctcaaccacgtggaccaggagcaccatttccaagacaaatatttattctatcgatttctggatgatgagcacgaggatgcccctttgcctactgaggaggagaagaaggagtgtgatgaggagctccaggacaccatgctgctgctgtcacagatgggccccgacgcccacatgaggatgatccttcgcaaaccacctggccagaggactgtggatgacctagagattatctatgaggagcttcttcatattaaagccttatcccatctttctaccacagtgaaacgagagttagcaggtgttctcatttttgagtctcacgccaaaggagggactgtgttgtttaaccagggggaagaaggtacctcctggtacattattctaaaaggatcagtgaatgtagtcatttacggcaagggtgtggtctgcaccctgcatgaaggagatgacttcggcaagttagcactagtgaatgatgccccacgagctgcctctatcgtcttacgagaagataactgccatttcttaagagtagacaaggaggatttcaaccggatcctaagggacgtgctcgagaacgtctatatcaaggccgacaagcagaagaacggcatcaaggcgaacttcaagatccgccacaacatcgaggacggcggcgtgcagctcgcctaccactaccagcagaacacccccatcggcgacggccccgtgctgctgcccgacaaccactacctgagcgtgcagtccatactttcgaaagaccccaacgagaagcgcgatcacatggtcctgctggagttcgtgaccgccgccgggatcactctcggcatggacgagctgtacaagggcggtaccggagggagcatggtgagcaagggcgaggagctgttcacccggggggtggtgcccatccaggtcgagctggacggcgacgtaaacggccacaagttcagcgtgtccggcgagggtgagggcgatgccacctacggcaagctgaccctgaagttcatctgcaccaccggcaagctgcccgtgccctggcccaccctcgtgaccaccctgacctacggcgtgcagtgcttcagccgctaccccgaccacatgaagcagcacgacttcttcaagtccgccatgcccgaaggctacatccaggagcgcaccatcttcttcaaggacgacggcaactacaagacccgcgccgaggtgaagttcgagggcgacaccctggtgaaccgcatcgagctgaagggcatcgacttcaaggaggacggcaacatcctggggcacaagctggagtacaacacgcgtaatacagtcagacttaaagaacatgaccaagatgtcttggtgctggagaaggtcccagcagggaacagagcttctaatcaaggaaactcacagcctcagcaaaagtatactgtgatgtcaggaacacctgaaaaaattttagagcattttctagaaacaatacgccttgaggcaactttaaatgaagcaacagattctgttttaaatgactttattatgatgcactgtgtttttatgccaaatacccagctttgcccggcactggtggcccactaccacgcacagccttcacaaggtacagaacaggagaaaatggattatgccctcaacaataagaggcgagtcatccgcctggttctacagtgggctgccatgtatggagacctcctgcaagaggatgacgtgtctatggccttcctggaggagttttatgtatctgtatcagatgatgcccggatgattgctgccctcaaggagcaactgccagagttggagaagattgtcaagcaaatctcagaagatgcaaaggcaccacaaaagaagcacaaggttcttttgcaacagttcaatacgggcgatgagagagcccagaagcgccagcctatccgcggctctgatgaagttctgtttaaggtctattgcatggaccccacctacacaaccattcgggtgccagtggccacttcggtgaaggaagtcatcagtgcagttgccgacaagctgggctccggggagggcctgatcatagtcaagatgagttccggaggagaaaaggtggtgctcaaacctaatgatgtttcagtatttatgacgctcaccattaatggacgcctgtttgcttgcccgcgagagcaattcgattcactgactcccttaccagaacaggaaggcccaactgttggaacagtgggaacttttgaactgatgagctccaaagatttagcataccagatgacaatttatgattgggaactcttcaactgcgtgcatgagctggagctaatctatcacacatttggaaggcataattttaaaaagaccacagcaaacttggatttgttcctgaggagatttaatgaaattcagttttgggtcgtcactgagatctgcctttgttctcagctcagcaagcgtgttcagctattaaaaaaatttattaagatagcagcccactgtaaggagtataaaaatctgaattccttttttgccatcgtcatgggactaagtaacgttgctgtgagccgcttggcactaacgtgggagaaactgccaagcaagttcaagaagttctatgcggagtttgaaagtttaatggacccttcaaggaaccacagggcctacaggctgacagtagctaagctggaacctcctctcatccccttcatgcctttgctcattaaagatatgacatttactcatgaggggaacaagacgttcattgacaatctagtaaactttgaaaaaatgcgcatgattgcaaatacggccagaacagtgagatactacaggagccaacccttcaatcctgatgcagctcaagctaataagaaccatcaggatgtccggagttatgtacggcaattaaatgtgattgacaaccagagaactttatcacagatgtcacacagattagagcctcgtcgacc

SEQ ID NO: 54 - DNA, 3765 bp, Artificial Sequence
  Synthetic
atggtcgctgcgcacgctgcccattcttcctcctctgccgagtggatcgcctgcctggataaaagaccactggagcgatccagcgaagatgtggatataatcttcactcgactgaaagaagttaaagcttttgagaaatttcacccaaatctccttcatcagatttgcttatgtggttattatgagaatctggaaaagggaataacattatttcgccagggtgatattggaacaaactggtatgctgtcctggcagggtctttggatgttaaagtatctgagaccagcagtcaccaggatgctgtgaccatctgtaccctgggaattgggacggcctttggagagtccattctggacaacacaccccgccatgcaaccatcgttaccagggagagcagtgaactgctccgcatcgagcagaaggacttcaaggcactatgggagaaatatcgacagtatatggcaggacttctggctcctccttatggtgttatggaaacgggctctaacaatgacaggattcctgacaaggagaacacacctctcattgaacctcacgttcctcttcgtcctgctaacaccattaccaaggtcccttcagagaagatcctcagagctggaaaaattttacgaaatgccattctctctcgagcacctcacatgataagagatagaaaataccacctaaagacatacagacaatgctgtgtgggaactgaactggtggactggatgatgcagcagacaccatgtgttcactcccggactcaagctgttggcatgtggcaagtcctgttagaagatggtgttctcaaccacgtggaccaggagcaccatttccaagacaaatatttattctatcgatttctggatgatgagcacgaggatgcccctttgcctactgaggaggagaagaaggagtgtgatgaggagctccaggacaccatgctgctgctgtcacagatgggccccgacgcccacatgaggatgatccttcgcaaaccacctggccagaggactgtggatgacctagagattatctatgaggagcttcttcatattaaagccttatcccatctttctaccacagtgaaacgagagttagcaggtgttctcatttttgagtctcacgccaaaggagggactgtgttgtttaaccagggggaagaaggtacctcctggtacattattctaaaaggatcagtgaatgtagtcatttacggcaagggtgtggtctgcaccctgcatgaaggagatgacttcggcaagttagcactagtgaatgatgccccacgagctgcctctatcgtcttacgagaagataactgccatttcttaagagtagacaaggaggatttcaaccggatcctaaggctcgagaacgtctatatcaaggccgacaagcagaagaacggcatcaaggcgaacttcaagatccgccacaacatcgaggacggcggcgtgcagctcgcctaccactaccagcagaacacccccatcggcgacggccccgtgctgctgcccgacaaccactacctgagcgtgcagtccatactttcgaaagaccccaacgagaagcgcgatcacatggtcctgctggagttcgtgaccgccgccgggatcactctcggcatggacgagctgttcaagggcggtaccggagggagcatggtgagcaagggcgaggagctgttcaccggggtggtgcccatccaggtcgagctggacggcgacgtaaacggccacaagttcagcgtgtccggcgagggtgagggcgatgccacctacggcaagctgaccctgaagttcatctgcaccaccggcaagctgcccgtgccctggcccaccctcgtgaccaccctgacctacggcgtgcagtgcttcagccgctaccccgaccacatgaagcagcacgacttcttcaagtccgccatgcccgaaggctacatccaggagcgcaccatcttcttcaaggacgacggcaactacaagacccgcgccgaggtgaagttcgagggcgacaccctggtgaaccgcatcgagctgaagggcatcgacttcaaggaggacggcaacatcctggggcacaagctggagtacaacacgcgtgtggaggcgaatacagtcagacttaaagaacatgaccaagatgtcttggtgctggagaaggtcccagcagggaacagagcttctaatcaaggaaactcacagcctcagcaaaagtatactgtgatgtcaggaacacctgaaaaaattttagagcattttctagaaacaatacgccttgaggcaactttaaatgaagcaacagattctgttttaaatgactttattatgatgcactgtgtttttatgccaaatacccagctttgcccggcactggtggcccactaccacgcacagccttcacaaggtacagaacaggagaaaatggattatgccctcaacaataagaggcgagtcatccgcctggttctacagtgggctgccatgtatggagacctcctgcaagaggatgacgtgtctatggccttcctggaggagttttatgtatctgtatcagatgatgcccggatgattgctgccctcaaggagcaactgccagagttggagaagattgtcaagcaaatctcagaagatgcaaaggcaccacaaaagaagcacaaggttcttttgcaacagttcaatacgggcgatgagagagcccagaagcgccagcctatccgcggctctgatgaagttctgtttaaggtctattgcatggaccccacctacacaaccattcgggtgccagtggccacttcggtgaaggaagtcatcagtgcagttgccgacaagctgggctccggggagggcctgatcatagtcaagatgagttccggaggagaaaaggtggtgctcaaacctaatgatgtttcagtatttatgacgctcaccattaatggacgcctgtttgcttgcccgcgagagcaattcgattcactgactcccttaccagaacaggaaggcccaactgttggaacagtgggaacttttgaactgatgagctccaaagatttagcataccagatgacaatttatgattgggaactcttcaactgcgtgcatgagctggagctaatctatcacacatttggaaggcataattttaaaaagaccacagcaaacttggatttgttcctgaggagatttaatgaaattcagttttgggtcgtcactgagatctgcctttgttctcagctcagcaagcgtgttcagctattaaaaaaatttattaagatagcagcccactgtaaggagtataaaaatctgaattccttttttgccatcgtcatgggactaagtaacgttgctgtgagccgcttggcactaacgtgggagaaactgccaagcaagttcaagaagttctatgcggagtttgaaagtttaatggacccttcaaggaaccacagggcctacaggctgacagtagctaagctggaacctcctctcatccccttcatgcctttgctcattaaagatatgacatttactcatgaggggaacaagacgttcattgacaatctagtaaactttgaaaaaatgcgcatgattgcaaatacggccagaacagtgagatactacaggagccaacccttcaatcctgatgcagctcaagctaataagaaccatcaggatgtccggagttatgtacggcaattaaatgtgattgacaaccagagaactttatcacagatgtcacacagattagagcctcgtcgacca

SEQ ID NO: 55 - DNA, 3783 bp, Artificial Sequence
  Synthetic
atggtcgctgcgcacgctgcccattcttcctcctctgccgagtggatcgcctgcctggataaaagaccactggagcgatccagcgaagatgtggatataatcttcactcgactgaaagaagttaaagcttttgagaaatttcacccaaatctccttcatcagatttgcttatgtggttattatgagaatctggaaaagggaataacattatttcgccagggtgatattggaacaaactggtatgctgtcctggcagggtctttggatgttaaagtatctgagaccagcagtcaccaggatgctgtgaccatctgtaccctgggaattgggacggcctttggagagtccattctggacaacacaccccgccatgcaaccatcgttaccagggagagcagtgaactgctccgcatcgagcagaaggacttcaaggcactatgggagaaatatcgacagtatatggcaggacttctggctcctccttatggtgttatggaaacgggctctaacaatgacaggattcctgacaaggagaacacacctctcattgaacctcacgttcctcttcgtcctgctaacaccattaccaaggtcccttcagagaagatcctcagagctggaaaaattttacgaaatgccattctctctcgagcacctcacatgataagagatagaaaataccacctaaagacatacagacaatgctgtgtgggaactgaactggtggactggatgatgcagcagacaccatgtgttcactcccggactcaagctgttggcatgtggcaagtcctgttagaagatggtgttctcaaccacgtggaccaggagcaccatttccaagacaaatatttattctatcgatttctggatgatgagcacgaggatgcccctttgcctactgaggaggagaagaaggagtgtgatgaggagctccaggacaccatgctgctgctgtcacagatgggccccgacgcccacatgaggatgatccttcgcaaaccacctggccagaggactgtggatgacctagagattatctatgaggagcttcttcatattaaagccttatcccatctttctaccacagtgaaacgagagttagcaggtgttctcatttttgagtctcacgccaaaggagggactgtgttgtttaaccagggggaagaaggtacctcctggtacattattctaaaaggatcagtgaatgtagtcatttacggcaagggtgtggtctgcaccctgcatgaaggagatgacttcggcaagttagcactagtgaatgatgccccacgagctgcctctatcgtcttacgagaagataactgccatttcttaagagtagacaaggaggatttcaaccggatcctaagggacgtgctcgagaacgtctatatcaaggccgacaagcagaagaacggcatcaaggcgaacttcaagatccgccacaacatcgaggacggcggcgtgcagctcgcctaccactaccagcagaacacccccatcggcgacggccccgtgctgctgcccgacaaccactacctgagcgtgcagtccatactttcgaaagaccccaacgagaagcgcgatcacatggtcctgctggagttcgtaaccgcccccgggatcactctcggcatggacgagctgtacaagggcggtaccggagggagcatggtgagcaagggcgaggagctgttcaccggggtggtgcccatccaggtcgagctggacggcgacgtaaacggccacaagttcagcgtgtccggcgagggtgagggcgatgccacctacggcaagctgaccctgaagttcatctgcaccaccggcaagctgcccgtgccctggcccaccctcgtgaccaccctgacctacggcgtgcagtgcttcagccgctaccccgaccacatgaagcagcacgacttcttcaagtccgccatgcccgaaggctacatccaggagcgcaccatcttcttcaaggacgacggcaactacaagacccgcgccgaggtgaagttcgagggcgacaccctggtgaaccgcatcgagctgaagggcatcgacttcaaggaggacggcaacatcctggggcacaagctggagtacaacacgcgtatcctaagggacgtggaggcgaatacagtcagacttaaagaacatgaccaagatgtcttggtgctggagaaggtcccagcagggaacagagcttctaatcaaggaaactcacagcctcagcaaaagtatactgtgatgtcaggaacacctgaaaaaattttagagcattttctagaaacaatacgccttgaggcaactttaaatgaagcaacagattctgttttaaatgactttattatgatgcactgtgtttttatgccaaatacccagctttgcccggcactggtggcccactaccacgcacagccttcacaaggtacagaacaggagaaaatggattatgccctcaacaataagaggcgagtcatccgcctggttctacagtgggctgccatgtatggagacctcctgcaagaggatgacgtgtctatggccttcctggaggagttttatgtatctgtatcagatgatgcccggatgattgctgccctcaaggagcaactgccagagttggagaagattgtcaagcaaatctcagaagatgcaaaggcaccacaaaagaagcacaaggttcttttgcaacagttcaatacgggcgatgagagagcccagaagcgccagcctatccgcggctctgatgaagttctgtttaaggtctattgcatggaccccacctacacaaccattcgggtgccagtggccacttcggtgaaggaagtcatcagtgcagttgccgacaagctgggctccggggagggcctgatcatagtcaagatgagttccggaggagaaaaggtggtgctcaaacctaatgatgtttcagtatttatgacgctcaccattaatggacgcctgtttgcttgcccgcgagagcaattcgattcactgactcccttaccagaacaggaaggcccaactgttggaacagtgggaacttttgaactgatgagctccaaagatttagcataccagatgacaatttatgattgggaactcttcaactgcgtgcatgagctggagctaatctatcacacatttggaaggcataattttaaaaagaccacagcaaacttggatttgttcctgaggagatttaatgaaattcagttttgggtcgtcactgagatctgcctttgttctcagctcagcaagcgtgttcagctattaaaaaaatttattaagatagcagcccactgtaaggagtataaaaatctgaattccttttttgccatcgtcatgggactaagtaacgttgctgtgagccgcttggcactaacgtgggagaaactgccaagcaagttcaagaagttctatgcggagtttgaaagtttaatggacccttcaaggaaccacagggcctacaggctgacagtagctaagctggaacctcctctcatccccttcatgcctttgctcattaaagatatgacatttactcatgaggggaacaagacgttcattgacaatctagtaaactttgaaaaaatgcgcatgattgcaaatacggccagaacagtgagatactacaggagccaacccttcaatcctgatgcagctcaagctaataagaaccatcaggatgtccggagttatgtacggcaattaaatgtgattgacaaccagagaactttatcacagatgtcacacagattagagcctcgtcgacca

SEQ ID NO: 56 - DNA, 2103 bp, Artificial Sequence
  Synthetic
atggtcgctgcgcacgctgcccattcttcctcctctgccgagtggatcgcctgcctggataaaagaccactggagcgatccagcgaagatgtggatataatcttcactcgactgaaagaagttaaagcttttgagaaatttcacccaaatctccttcatcagatttgcttatgtggttattatgagaatctggaaaagggaataacattatttcgccagggtgatattggaacaaactggtatgctgtcctggcagggtctttggatgttaaagtatctgagaccagcagtcaccaggatgctgtgaccatctgtaccctgggaattgggacggcctttggagagtccattctggacaacacaccccgccatgcaaccatcgttaccagggagagcagtgaactgctccgcatcgagcagaaggacttcaaggcactatgggagaaatatcgacagtatatggcaggacttctggctcctccttatggtgttatggaaacgggctctaacaatgacaggattcctgacaaggagaacacacctctcattgaacctcacgttcctcttcgtcctgctaacaccattaccaaggtcccttcagagaagatcctcagagctggaaaaattttacgaaatgccattctctctcgagcacctcacatgataagagatagaaaataccacctaaagacatacagacaatgctgtgtgggaactgaactggtggactggatgatgcagcagacaccatgtgttcactcccggactcaagctgttggcatgtggcaagtcctgttagaagatggtgttctcaaccacgtggaccaggagcaccatttccaagacaaatatttattctatcgatttctggatgatgagcacgaggatgcccctttgcctactgaggaggagaagaaggagtgtgatgaggagctccaggacaccatgctgctgctgtcacagatgggccccgacgcccacatgaggatgatccttcgcaaaccacctggccagaggactgtggatgacctagagattatctatgaggagcttcttcatattaaagccttatcccatctttctaccacagtgaaacgagagttagcaggtgttctcatttttgagtctcacgccaaaggagggactgtgttgtttaaccagggggaagaaggtacctcctggtacattattctaaaaggatcagtgaatgtagtcatttacggcaagggtgtggtctgcaccctgcatgaaggagatgacttcggcaagttagcactagtgaatgatgccccacgagctgcctctatcgtcttacgagaagataactgccatttcttaagagtagacaaggaggatttcaaccggatcctaaggcgtgcgaacgtctatatcaaggccgacaagcagaagaacggcatcaaggcgaacttcaagatccgccacaacatcgaggacggcggcgtgcagctcgcctaccactaccagcagaacacccccatcggcgacggccccgtgctgctgcccgacaaccactacctgagcgtgcagtccatactttcgaaagaccccaacgagaagcgcgatcacatggtcctgctggagttcgtgaccgccgccgggatcactctcggcatggacgagctgtacaagggcggtaccggagggagcatggtgagcaagggcgaggagctgttcaccggggtggtgcccatccaggtcgagctggacggcgacgtaaacggccacaagttcagcgtgtccggcgagggtgagggcgatgccacctacggcaagctgaccctgaagttcatctgcaccaccggcaagctgcccgtgccctggcccaccctcgtgaccaccctgacctacggcgtgcagtgcttcagccgctaccccgaccacatgaagcagcacgacttcttcaagtccgccatgcccgaaggctacatccaggagcgcaccatcttcttcaaggacgacggcaactacaagacccgcgccgaggtgaagttcgagggcgacaccctggtgaaccgcatcgagctgaagggcatcgacttcaaggaggacggcaacatcctggggcacaagctggagtacaac

SEQ ID NO: 57 - DNA, 3768 bp, Artificial Sequence
  Synthetic
atggtcgctgcgcacgctgcccattcttcctcctctgccgagtggatcgcctgcctggataaaagaccactggagcgatccagcgaagatgtggatataatcttcactcgactgaaagaagttaaagcttttgagaaatttcacccaaatctccttcatcagatttgcttatgtggttattatgagaatctggaaaagggaataacattatttcgccagggtgatattggaacaaactggtatgctgtcctggcagggtctttggatgttaaagtatctgagaccagcagtcaccaggatgctgtgaccatctgtaccctgggaattgggacggcctttggagagtccattctggacaacacaccccgccatgcaaccatcgttaccagggagagcagtgaactgctccgcatcgagcagaaggacttcaaggcactatgggagaaatatcgacagtatatggcaggacttctggctcctccttatggtgttatggaaacgggctctaacaatgacaggattcctgacaaggagaacacacctctcattgaacctcacgttcctcttcgtcctgctaacaccattaccaaggtcccttcagagaagatcctcagagctggaaaaattttacgaaatgccattctctctcgagcacctcacatgataagagatagaaaataccacctaaagacatacagacaatgctgtgtgggaactgaactggtggactggatgatgcagcagacaccatgtgttcactcccggactcaagctgttggcatgtggcaagtcctgttagaagatggtgttctcaaccacgtggaccaggagcaccatttccaagacaaatatttattctatcgatttctggatgatgagcacgaggatgcccctttgcctactgaggaggagaagaaggagtgtgatgaggagctccaggacaccatgctgctgctgtcacagatgggccccgacgcccacatgaggatgatccttcgcaaaccacctggccagaggactgtggatgacctagagattatctatgaggagcttcttcatattaaagccttatcccatctttctaccacagtgaaacgagagttagcaggtgttctcatttttgagtctcacgccaaaggagggactgtgttgtttaaccagggggaagaaggtacctcctggtacattattctaaaaggatcagtgaatgtagtcatttacggcaagggtgtggtctgcaccctgcatgaaggagatgacttcggcaagttagcactagtgaatgatgccccacgagctgcctctatcgtcttacgagaagataactgccatttcttaagagtagacaaggaggatttcaaccggatcctaagggacgtggaggcgaatctcgagaacgtctatatcaaggccgacaagcagaagaacggcatcaaggcgaacttcaagatccgccacaacatcgaggacggcggcgtgcagctcgcctaccactaccagcagaacacccccatcggcgacggccccgtgctgctgcccgacaaccactacctgagcgtgcagtccatactttcgaaagaccccaacgagaagcgcgatcacatggtcctgctggagttcgtgaccgccgccgggatcactctcggcatggacgagctgtacaagggcggtaccggagggagcatggtgagcaagggcgaggagctgttcaccggggtggtgcccatccaggtcgagctggacggcgacgtaaacggccacaagttcagcgtgtccggcgagggtgagggcgatgccacctacggcaagctgaccctgaagttcatctgcaccaccggcaagctgcccgtgccctggcccaccctcgtgaccaccctgacctacggcgtgcagtgcttcagccgctaccccgaccacatgaagcagcacgacttcttcaagtccgccatgcccgaaggctacatccaggagcgcaccatcttcttcaaggacgacggcaactacaagacccgcgccgaggtgaagttcgagggcgacaccctggtgaaccgcatcgagctgaagggcatcgacttcaaggaggacggcaacatcctggggcacaagctggagtacaacacgcgtacagtcagacttaaagaacatgaccaagatgtcttggtgctggagaaggtcccagcagggaacagagcttctaatcaaggaaactcacagcctcagcaaaagtatactgtgatgtcaggaacacctgaaaaaattttagagcattttctagaaacaatacgccttgaggcaactttaaatgaagcaacagattctgttttaaatgactttattatgatgcactgtgtttttatgccaaatacccagctttgcccggcactggtggcccactaccacgcacagccttcacaaggtacagaacaggagaaaatggattatgccctcaacaataagaggcgagtcatccgcctggttctacagtgggctgccatgtatggagacctcctgcaagaggatgacgtgtctatggccttcctggaggagttttatgtatctgtatcagatgatgcccggatgattgctgccctcaaggagcaactgccagagttggagaagattgtcaagcaaatctcagaagatgcaaaggcaccacaaaagaagcacaaggttcttttgcaacagttcaatacgggcgatgagagagcccagaagcgccagcctatccgcggctctgatgaagttctgtttaaggtctattgcatggaccccacctacacaaccattcgggtgccagtggccacttcggtgaaggaagtcatcagtgcagttgccgacaagctgggctccggggagggcctgatcatagtcaagatgagttccggaggagaaaaggtggtgctcaaacctaatgatgtttcagtatttatgacgctcaccattaatggacgcctgtttgcttgcccgcgagagcaattcgattcactgactcccttaccagaacaggaaggcccaactgttggaacagtgggaacttttgaactgatgagctccaaagatttagcataccagatgacaatttatgattgggaactcttcaactgcgtgcatgagctggagctaatctatcacacatttggaaggcataattttaaaaagaccacagcaaacttggatttgttcctgaggagatttaatgaaattcagttttgggtcgtcactgagatctgcctttgttctcagctcagcaagcgtgttcagctattaaaaaaatttattaagatagcagcccactgtaaggagtataaaaatctgaattccttttttgccatcgtcatgggactaagtaacgttgctgtgagccgcttggcactaacgtgggagaaactgccaagcaagttcaagaagttctatgcggagtttgaaagtttaatggacccttcaaggaaccacagggcctacaggctgacagtagctaagctggaacctcctctcatccccttcatgcctttgctcattaaagatatgacatttactcatgaggggaacaagacgttcattgacaatctagtaaactttgaaaaaatgcgcatgattgcaaatacggccagaacagtgagatactacaggagccaacccttcaatcctgatgcagctcaagctaataagaaccatcaggatgtccggagttatgtacggcaattaaatgtgattgacaaccagagaactttatcacagatgtcacacagattagagcctcgtcgacca

SEQ ID NO: 58 - DNA, 3765 bp, Artificial Sequence
  Synthetic
atggtcgctgcgcacgctgcccattcttcctcctctgccgagtggatcgcctgcctggataaaagaccactggagcgatccagcgaagatgtggatataatcttcactcgactgaaagaagttaaagcttttgagaaatttcacccaaatctccttcatcagatttgcttatgtggttattatgagaatctggaaaagggaataacattatttcgccagggtgatattggaacaaactggtatgctgtcctggcagggtctttggatgttaaagtatctgagaccagcagtcaccaggatgctgtgaccatctgtaccctgggaattgggacggcctttggagagtccattctggacaacacaccccgccatgcaaccatcgttaccagggagagcagtgaactgctccgcatcgagcagaaggacttcaaggcactatgggagaaatatcgacagtatatggcaggacttctggctcctccttatggtgttatggaaacgggctctaacaatgacaggattcctgacaaggagaacacacctctcattgaacctcacgttcctcttcgtcctgctaacaccattaccaaggtcccttcagagaagatcctcagagctggaaaaattttacgaaatgccattctctctcgagcacctcacatgataagagatagaaaataccacctaaagacatacagacaatgctgtgtgggaactgaactggtggactggatgatgcagcagacaccatgtgttcactcccggactcaagctgttggcatgtggcaagtcctgttagaagatggtgttctcaaccacgtggaccaggagcaccatttccaagacaaatatttattctatcgatttctggatgatgagcacgaggatgcccctttgcctactgaggaggagaagaaggagtgtgatgaggagctccaggacaccatgctgctgctgtcacagatgggccccgacgcccacatgaggatgatccttcgcaaaccacctggccagaggactgtggatgacctagagattatctatgaggagcttcttcatattaaagccttatcccatctttctaccacagtgaaacgagagttagcaggtgttctcatttttgagtctcacgccaaaggagggactgtgttgtttaaccagggggaagaaggtacctcctggtacattattctaaaaggatcagtgaatgtagtcatttacggcaagggtgtggtctgcaccctgcatgaaggagatgacttcggcaagttagcactagtgaatgatgccccacgagctgcctctatcgtcttacgagaagataactgccatttcttaagagtagacaaggaggatttcaaccggatcctaaggctcgagaacgtctatatcaaggccgacaagcagaagaacggcatcaaggcgaacttcaagatccgccacaacatcgaggacggcggcgtgcagctcgcctaccactaccagcagaacacccccatcggcgacggccccgtgctgctgcccgacaaccactacctgagcgtgcagtccatactttcgaaagaccccaacgagaagcgcgatcacatggtcctgctggagttcgtgaccgccgccgggatcactctcggcatggacgagctgtacaagggcggtaccggagggagcatggtgagcaagggcgaggagctgttcaccggggtggtgcccatccaggtcgagctggacggcgacgtaaacggccacaagttcagcgtgtccggcgagggtgagggcgatgccacctacggcaagctgaccctgaagttcatctgcaccaccggcaagctgcccgtgccctggcccaccctcgtgaccaccctgacctacggcgtgcagtgcttcagccgctaccccgaccacatgaagcagcacgacttcttcaagtccgccatgcccgaaggctacatccaggagcgcaccatcttcttcaaggacgacggcaactacaagacccgcgccgaggtgaagttcgagggcgacaccctggtgaaccgcatcgagctgaagggcatcgacttcaaggaggacggcaacatcctggggcacaagctggagtacaacacgcgtgtggaggcgaatacagtcagacttaaagaacatgaccaagatgtcttggtgctggagaaggtcccagcagggaacagagcttctaatcaaggaaactcacagcctcagcaaaagtatactgtgatgtcaggaacacctgaaaaaattttagagcattttctagaaacaatacgccttgaggcaactttaaatgaagcaacagattctgttttaaatgactttattatgatgcactgtgtttttatgccaaatacccagctttgcccggcactggtggcccactaccacgcacagccttcacaaggtacagaacaggagaaaatggattatgccctcaacaataagaggcgagtcatccgcctggttctacagtgggctgccatgtatggagacctcctgcaagaggatgacgtgtctatggccttcctggaggagttttatgtatctgtatcagatgatgcccggatgattgctgccctcaaggagcaactgccagagttggagaagattgtcaagcaaatctcagaagatgcaaaggcaccacaaaagaagcacaaggttcttttgcaacagttcaatacgggcgatgagagagcccagaagcgccagcctatccgcggctctgatgaagttctgtttaaggtctattgcatggaccccacctacacaaccattcgggtgccagtggccacttcggtgaaggaagtcatcagtgcagttgccgacaagctgggctccggggagggcctgatcatagtcaagatgagttccggaggagaaaaggtggtgctcaaacctaatgatgtttcagtatttatgacgctcaccattaatggacgcctgtttgcttgcccgcgagagcaattcgattcactgactcccttaccagaacaggaaggcccaactgttggaacagtgggaacttttgaactgatgagctccaaagatttagcataccagatgacaatttatgattgggaactcttcaactgcgtgcatgagctggagctaatctatcacacatttggaaggcataattttaaaaagaccacagcaaacttggatttgttcctgaggagatttaatgaaattcagttttgggtcgtcactgagatctgcctttgttctcagctcagcaagcgtgttcagctattaaaaaaatttattaagatagcagcccactgtaaggagtataaaaatctgaattccttttttgccatcgtcatgggactaagtaacgttgctgtgagccgcttggcactaacgtgggagaaactgccaagcaagttcaagaagttctatgcggagtttgaaagtttaatggacccttcaaggaaccacagggcctacaggctgacagtagctaagctggaacctcctctcatccccttcatgcctttgctcattaaagatatgacatttactcatgaggggaacaagacgttcattgacaatctagtaaactttgaaaaaatgcgcatgattgcaaatacggccagaacagtgagatactacaggagccaacccttcaatcctgatgcagctcaagctaataagaaccatcaggatgtccggagttatgtacggcaattaaatgtgattgacaaccagagaactttatcacagatgtcacacagattagagcctcgtcgacca

SEQ ID NO: 59 - DNA, 3776 bp, Artificial Sequence
  Synthetic
atggtcgctgcgcacgctgcccattcttcctcctctgccgagtggatcgcctgcctggataaaagaccactggagcgatccagcgaagatgtggatataatcttcactcgactgaaagaagttaaagcttttgagaaatttcacccaaatctccttcatcagatttgcttatgtggttattatgagaatctggaaaagggaataacattatttcgccagggtgatattggaacaaactggtatgctgtcctggcagggtctttggatgttaaagtatctgagaccagcagtcaccaggatgctgtgaccatctgtaccctgggaattgggacggcctttggagagtccattctggacaacacaccccgccatgcaaccatcgttaccagggagagcagtgaactgctccgcatcgagcagaaggacttcaaggcactatgggagaaatatcgacagtatatggcaggacttctggctcctccttatggtgttatggaaacgggctctaacaatgacaggattcctgacaaggagaacacacctctcattgaacctcacgttcctcttcgtcctgctaacaccattaccaaggtcccttcagagaagatcctcagagctggaaaaattttacgaaatgccattctctctcgagcacctcacatgataagagatagaaaataccacctaaagacatacagacaatgctgtgtgggaactgaactggtggactggatgatgcagcagacaccatgtgttcactcccggactcaagctgttggcatgtggcaagtcctgttagaagatggtgttctcaaccacgtggaccaggagcaccatttccaagacaaatatttattctatcgatttctggatgatgagcacgaggatgcccctttgcctactgaggaggagaagaaggagtgtgatgaggagctccaggacaccatgctgctgctgtcacagatgggccccgacgcccacatgaggatgatccttcgcaaaccacctggccagaggactgtggatgacctagagattatctatgaggagcttcttcatattaaagccttatcccatctttctaccacagtgaaacgagagttagcaggtgttctcatttttgagtctcacgccaaaggagggactgtgttgtttaaccagggggaagaaggtacctcctggtacattattctaaaaggatcagtgaatgtagtcatttacggcaagggtgtggtctgcaccctgcatgaaggagatgacttcggcaagttagcactagtgaatgatgccccacgagctgcctctatcgtcttacgagaagataactgccatttcttaagagtagacaaggaggatttcaaccggatcctaaggctcgagaacgtctatatcaaggccgacaagcagaagaacggcatcaaggcgaacttcaagatccgccacaacatcgaggacggcggcgtgcagctcgcctaccactaccagcagaacacccccatcggcgacggccccgtgctgctgcccgacaaccactacctgagcgtgcagtccatactttcgaaagaccccaacgagaagcgcgatcacatggtcctgctggagttcgtgaccgccgccgggatcactctcggcatggacgagctgtacaagggcggtaccggagggagcatggtgagcaagggcgaggagctgttcaccggggtggtgcccatccaggtcgagctggacggcgacgtaaacggccacaagttcagcgtgtccggcgagggtgagggcgatgccacctacggcaagctgaccctgaagttcatctgcaccaccggcaagctgcccgtgccctggcccaccctcgtgaccaccctgacctacggcgtgcagtgcttcagccgctaccccgaccacatgaagcagcacgacttcttcaagtccgccatgcccgaaggctacatccaggagcgcaccatcttcttcaaggacgacggcaactacaagacccgcgccgaggtgaagttcgagggcgacaccctggtgaaccgcatcgagctgaagggcatcgacttcaaggaggacggcaacatcctggggcacaagctggagtacaacacgcgtatcctaagggacgtggaggcgaatacagtcagacttaaagaacatgaccaagatgtcttggtgctggagaaggtcccagcagggaacagagcttctaatcaaggaaactcacagcctcagcaaaagtatactgtgatgtcaggaacacctgaaaaaattttagagcattttctagaaacaatacgccttgaggcaactttaaatgaagcaacagattctgttttaaatgactttattatgatgcactgtgtttttatgccaaatacccagctttgcccggcactggtggcccactaccacgcacagccttcacaaggtacagaacaggagaaaatggattatgccctcaacaataagaggcgagtcatccgcctggttctacagtgggctgccatgtatggagacctcctgcaagaggatgacgtgtctatggccttcctggaggagttttatgtatctgtatcagatgatgcccggatgattgctgccctcaaggagcaactgccagagttggagaagattgtcaagcaaatctcagaagatgcaaaggcaccacaaaagaagcacaaggttcttttgcaacagttcaatacgggcgatgagagagcccagaagcgccagcctatccgcggctctgatgaagttctgtttaaggtctattgcatggaccccacctacacaaccattcgggtgccagtggccacttcggtgaaggaagtcatcagtgcagttgccgacaagctgggctccggggagggcctgatcatagtcaagatgagttccggaggagaaaaggtggtgctcaaacctaatgatgtttcagtatttatgacgctcaccattaatggacgcctgtttgcttgcccgcgagagcaattcgattcactgactcccttaccagaacaggaaggcccaactgttggaacagtgggaacttttgaactgatgagctccaaagatttagcataccagatgacaatttatgattgggaactcttcaactgcgtgcatgagctggagctaatctatcacacatttggaaggcataattttaaaaagaccacagcaaacttggatttgttcctgaggagatttaatgaaattcagttttgggtcgtcactgagatctgcctttgttctcagctcagcaagcgtgttcagctattaaaaaaatttattaagatagcagcccactgtaaggagtataaaaatctgaattccttttttgccatcgtcatgggactaagtaacgttgctgtgagccgcttggcactaacgtgggagaaactgccaagcaagttcaagaagttctatgcggagtttgaaagtttaatggacccttcaaggaaccacagggcctacaggctgacagtagctaagctggaacctcctctcatccccttcatgcctttgctcattaaagatatgacatttactcatgaggggaacaagacgttcattgacaatctagtaaactttgaaaaaatgcgcatgattgcaaatacggccagaacagtgagatactacaggagccaacccttcaatcctgatgcagctcaagctaataagaaccatcaggatgtccggagttatgtacggcaattaaatgtgattgacaaccagagaactttatcacagatgtcacacagattagagcctcgtcgacc

SEQ ID NO: 60 - DNA, 3756 bp, Artificial Sequence
  Synthetic
atggtcgctgcgcacgctgcccattcttcctcctctgccgagtggatcgcctgcctggataaaagaccactggagcgatccagcgaagatgtggatataatcttcactcgactgaaagaagttaaagcttttgagaaatttcacccaaatctccttcatcagatttgcttatgtggttattatgagaatctggaaaagggaataacattatttcgccagggtgatattggaacaaactggtatgctgtcctggcagggtctttggatgttaaagtatctgagaccagcagtcaccaggatgctgtgaccatctgtaccctgggaattgggacggcctttggagagtccattctggacaacacaccccgccatgcaaccatcgttaccagggagagcagtgaactgctccgcatcgagcagaaggacttcaaggcactatgggagaaatatcgacagtatatggcaggacttctggctcctccttatggtgttatggaaacgggctctaacaatgacaggattcctgacaaggagaacacacctctcattgaacctcacgttcctcttcgtcctgctaacaccattaccaaggtcccttcagagaagatcctcagagctggaaaaattttacgaaatgccattctctctcgagcacctcacatgataagagatagaaaataccacctaaagacatacagacaatgctgtgtgggaactgaactggtggactggatgatgcagcagacaccatgtgttcactcccggactcaagctgttggcatgtggcaagtcctgttagaagatggtgttctcaaccacgtggaccaggagcaccatttccaagacaaatatttattctatcgatttctggatgatgagcacgaggatgcccctttgcctactgaggaggagaagaaggagtgtgatgaggagctccaggacaccatgctgctgctgtcacagatgggccccgacgcccacatgaggatgatccttcgcaaaccacctggccagaggactgtggatgacctagagattatctatgaggagcttcttcatattaaagccttatcccatctttctaccacagtgaaacgagagttagcaggtgttctcatttttgagtctcacgccaaaggagggactgtgttgtttaaccagggggaagaaggtacctcctggtacattattctaaaaggatcagtgaatgtagtcatttacggcaagggtgtggtctgcaccctgcatgaaggagatgacttcggcaagttagcactagtgaatgatgccccacgagctgcctctatcgtcttacgagaagataactgccatttcttaagagtagacaaggaggatttcaaccggatcctaaggctcgagaacgtctatatcaaggccgacaagcagaagaacggcatcaaggcgaacttcaagatccgccacaacatcgaggacggcggcgtgcagctcgcctaccactaccagcagaacacccccatcggcgacggccccgtgctgctgcccgacaaccactacctgagcgtgcagtccatactttcgaaagaccccaacgagaagcgcgatcacatggtcctgctggagttcgtgaccgccgccgggatcactctcggcatggacgagctgtacaagggcggtaccggagggagcatggtgagcaagggcgaggagctgttcaccggggtggtgcccatccaggtcgagctggacggcgacgtaaacggccacaagttcagcgtgtccggcgagggtgagggcgatgccacctacggcaagctgaccctgaagttcatctgcaccaccggcaagctgcccgtgccctggcccaccctcgtgaccaccctgacctacggcgtgcagtgcttcagccgctaccccgaccacatgaagcagcacgacttcttcaagtccgccatgcccgaaggctacatccaggagcgcaccatcttcttcaaggacgacggcaactacaagacccgcgccgaggtgaagttcgagggcgacaccctggtgaaccgcatcgagctgaagggcatcgacttcaaggaggacggcaacatcctggggcacaagctggagtacaacacgcgtaatacagtcagacttaaagaacatgaccaagatgtcttggtgctggagaaggtcccagcagggaacagagcttctaatcaaggaaactcacagcctcagcaaaagtatactgtgatgtcaggaacacctgaaaaaattttagagcattttctagaaacaatacgccttgaggcaactttaaatgaagcaacagattctgttttaaatgactttattatgatgcactgtgtttttatgccaaatacccagctttgcccggcactggtggcccactaccacgcacagccttcacaaggtacagaacaggagaaaatggattatgccctcaacaataagaggcgagtcatccgcctggttctacagtgggctgccatgtatggagacctcctgcaagaggatgacgtgtctatggccttcctggaggagttttatgtatctgtatcagatgatgcccggatgattgctgccctcaaggagcaactgccagagttggagaagattgtcaagcaaatctcagaagatgcaaaggcaccacaaaagaagcacaaggttcttttgcaacagttcaatacgggcgatgagagagcccagaagcgccagcctatccgcggctctgatgaagttctgtttaaggtctattgcatggaccccacctacacaaccattcgggtgccagtggccacttcggtgaaggaagtcatcagtgcagttgccgacaagctgggctccggggagggcctgatcatagtcaagatgagttccggaggagaaaaggtggtgctcaaacctaatgatgtttcagtatttatgacgctcaccattaatggacgcctgtttgcttgcccgcgagagcaattcgattcactgactcccttaccagaacaggaaggcccaactgttggaacagtgggaacttttgaactgatgagctccaaagatttagcataccagatgacaatttatgattgggaactcttcaactgcgtgcatgagctggagctaatctatcacacatttggaaggcataattttaaaaagaccacagcaaacttggatttgttcctgaggagatttaatgaaattcagttttgggtcgtcactgagatctgcctttgttctcagctcagcaagcgtgttcagctattaaaaaaatttattaagatagcagcccactgtaaggagtataaaaatctgaattccttttttgccatcgtcatgggactaagtaacgttgctgtgagccgcttggcactaacgtgggagaaactgccaagcaagttcaagaagttctatgcggagtttgaaagtttaatggacccttcaaggaaccacagggcctacaggctgacagtagctaagctggaacctcctctcatccccttcatgcctttgctcattaaagatatgacatttactcatgaggggaacaagacgttcattgacaatctagtaaactttgaaaaaatgcgcatgattgcaaatacggccagaacagtgagatactacaggagccaacccttcaatcctgatgcagctcaagctaataagaaccatcaggatgtccggagttatgtacggcaattaaatgtgattgacaaccagagaactttatcacagatgtcacacagattagagcctcgtcgacca

SEQ ID NO: 61 - DNA, 3783 bp, Artificial Sequence
  Synthetic
atggtcgctgcgcacgctgcccattcttcctcctctgccgagtggatcgcctgcctggataaaagaccactggagcgatccagcgaagatgtggatataatcttcactcgactgaaagaagttaaagcttttgagaaatttcacccaaatctccttcatcagatttgcttatgtggttattatgagaatctggaaaagggaataacattatttcgccagggtgatattggaacaaactggtatgctgtcctggcagggtctttggatgttaaagtatctgagaccagcagtcaccaggatgctgtgaccatctgtaccctgggaattgggacggcctttggagagtccattctggacaacacaccccgccatgcaaccatcgttaccagggagagcagtgaactgctccgcatcgagcagaaggacttcaaggcactatgggagaaatatcgacagtatatggcaggacttctggctcctccttatggtgttatggaaacgggctctaacaatgacaggattcctgacaaggagaacacacctctcattgaacctcacgttcctcttcgtcctgctaacaccattaccaaggtcccttcagagaagatcctcagagctggaaaaattttacgaaatgccattctctctcgagcacctcacatgataagagatagaaaataccacctaaagacatacagacaatgctgtgtgggaactgaactggtggactggatgatgcagcagacaccatgtgttcactcccggactcaagctgttggcatgtggcaagtcctgttagaagatggtgttctcaaccacgtggaccaggagcaccatttccaagacaaatatttattctatcgatttctggatgatgagcacgaggatgcccctttgcctactgaggaggagaagaaggagtgtgatgaggagctccaggacaccatgctgctgctgtcacagatgggccccgacgcccacatgaggatgatccttcgcaaaccacctggccagaggactgtggatgacctagagattatctatgaggagcttcttcatattaaagccttatcccatctttctaccacagtgaaacgagagttagcaggtgttctcatttttgagtctcacgccaaaggagggactgtgttgtttaaccagggggaagaaggtacctcctggtacattattctaaaaggatcagtgaatgtagtcatttacggcaagggtgtggtctgcaccctgcatgaaggagatgacttcggcaagttagcactagtgaatgatgccccacgagctgcctctatcgtcttacgagaagataactgccatttcttaagagtagacaaggaggatttcaaccggatcctaaggctcgagaacgtctatatcaaggccgacaagcagaagaacggcatcaaggcgaacttcaagatccgccacaacatcgaggacggcggcgtgcagctcgcctaccactaccagcagaacacccccatcggcgacggccccgtgctgctgcccgacaaccactacctgagcgtgcagtccatactttcgaaagaccccaacgagaagcgcgatcacatggtcctgctggagttcgtgaccgccgccgggatcactctcggcatggacgagctgtacaagggcggtaccggagggagcatggtgagcaagggcgaggagctgttcaccggggtggtgcccatccaggtcgagctggacggcgacgtaaacggccacaagttcagcgtgtccggcgagggtgagggcgatgccacctacggcaagctgaccctgaagttcatctgcaccaccggcaagctgcccgtgccctggcccaccctcgtgaccaccctgacctacggcgtgcagtgcttcagccgctaccccgaccacatgaagcagcacgacttcttcaagtccgccatgcccgaaggctacatccaggagcgcaccatcttcttcaaggacgacggcaactacaagacccgcgccgaggtgaagttcgagggcgacaccctggtgaaccgcatcgagctgaagggcatcgacttcaaggaggacggcaacatcctggggcacaagctggagtacaacacgcgtaaccggatcctaagggacgtggaggcgaatacagtcagacttaaagaacatgaccaagatgtcttggtgctggagaaggtcccagcagggaacagagcttctaatcaaggaaactcacagcctcagcaaaagtatactgtgatgtcaggaacacctgaaaaaattttagagcattttctagaaacaatacgccttgaggcaactttaaatgaagcaacagattctgttttaaatgactttattatgatgcactgtgtttttatgccaaatacccagctttgcccggcactggtggcccactaccacgcacagccttcacaaggtacagaacaggagaaaatggattatgccctcaacaataagaggcgagtcatccgcctggttctacagtgggctgccatgtatggagacctcctgcaagaggatgacgtgtctatggccttcctggaggagttttatgtatctgtatcagatgatgcccggatgattgctgccctcaaggagcaactgccagagttggagaagattgtcaagcaaatctcagaagatgcaaaggcaccacaaaagaagcacaaggttcttttgcaacagttcaatacgggcgatgagagagcccagaagcgccagcctatccgcggctctgatgaagttctgtttaaggtctattgcatggaccccacctacacaaccattcgggtgccagtggccacttcggtgaaggaagtcatcagtgcagttgccgacaagctgggctccggggagggcctgatcatagtcaagatgagttccggaggagaaaaggtggtgctcaaacctaatgatgtttcagtatttatgacgctcaccattaatggacgcctgtttgcttgcccgcgagagcaattcgattcactgactcccttaccagaacaggaaggcccaactgttggaacagtgggaacttttgaactgatgagctccaaagatttagcataccagatgacaatttatgattgggaactcttcaactgcgtgcatgagctggagctaatctatcacacatttggaaggcataattttaaaaagaccacagcaaacttggatttgttcctgaggagatttaatgaaattcagttttgggtcgtcactgagatctgcctttgttctcagctcagcaagcgtgttcagctattaaaaaaatttattaagatagcagcccactgtaaggagtataaaaatctgaattccttttttgccatcgtcatgggactaagtaacgttgctgtgagccgcttggcactaacgtgggagaaactgccaagcaagttcaagaagttctatgcggagtttgaaagtttaatggacccttcaaggaaccacagggcctacaggctgacagtagctaagctggaacctcctctcatccccttcatgcctttgctcattaaagatatgacatttactcatgaggggaacaagacgttcattgacaatctagtaaactttgaaaaaatgcgcatgattgcaaatacggccagaacagtgagatactacaggagccaacccttcaatcctgatgcagctcaagctaataagaaccatcaggatgtccggagttatgtacggcaattaaatgtgattgacaaccagagaactttatcacagatgtcacacagattagagcctcgtcgacca

SEQ ID NO: 62 - DNA, 3810 bp, Artificial Sequence
  Synthetic
atggtcgctgcgcacgctgcccattcttcctcctctgccgagtggatcgcctgcctggataaaagaccactggagcgatccagcgaagatgtggatataatcttcactcgactgaaagaagttaaagcttttgagaaatttcacccaaatctccttcatcagatttgcttatgtggttattatgagaatctggaaaagggaataacattatttcgccagggtgatattggaacaaactggtatgctgtcctggcagggtctttggatgttaaagtatctgagaccagcagtcaccaggatgctgtgaccatctgtaccctgggaattgggacggcctttggagagtccattctggacaacacaccccgccatgcaaccatcgttaccagggagagcagtgaactgctccgcatcgagcagaaggacttcaaggcactatgggagaaatatcgacagtatatggcaggacttctggctcctccttatggtgttatggaaacgggctctaacaatgacaggattcctgacaaggagaacacacctctcattgaacctcacgttcctcttcgtcctgctaacaccattaccaaggtcccttcagagaagatcctcagagctggaaaaattttacgaaatgccattctctctcgagcacctcacatgataagagatagaaaataccacctaaagacatacagacaatgctgtgtgggaactgaactggtggactggatgatgcagcagacaccatgtgttcactcccggactcaagctgttggcatgtggcaagtcctgttagaagatggtgttctcaaccacgtggaccaggagcaccatttccaagacaaatatttattctatcgatttctggatgatgagcacgaggatgcccctttgcctactgaggaggagaagaaggagtgtgatgaggagctccaggacaccatgctgctgctgtcacagatgggccccgacgcccacatgaggatgatccttcgcaaaccacctggccagaggactgtggatgacctagagattatctatgaggagcttcttcatattaaagccttatcccatctttctaccacagtgaaacgagagttagcaggtgttctcatttttgagtctcacgccaaaggagggactgtgttgtttaaccagggggaagaaggtacctcctggtacattattctaaaaggatcagtgaatgtagtcatttacggcaagggtgtggtctgcaccctgcatgaaggagatgacttcggcaagttagcactagtgaatgatgccccacgagctgcctctatcgtcttacgagaagataactgccatttcttaagagtagacaaggaggatttcaaccggatcctaagggacgtggaggcgaatctcgagaacgtctatatcaaggccgacaagcagaagaacggcatcaaggcgaacttcaagatccgccacaacatcgaggacggcggcgtgcagctcgcctaccactaccagcagaacacccccatcggcgacggccccgtgctgctgcccgacaaccactacctgagcgtgcagtccatactttcgaaagaccccaacgagaagcgcgatcacatggtcctgctggagttcgtgaccgccgccgggatcactctcggcatggacgagctgtacaagggcggtaccggagggagcatggtgagcaagggcgaggagctgttcaccggggtggtgcccatccaggtcgagctggacggcgacgtaaacggccacaagttcagcgtgtccggcgagggtgagggcgatgccacctacggcaagctgaccctgaagttcatctgcaccaccggcaagctgcccgtgccctggcccaccctcgtgaccaccctgacctacggcgtgcagtgcttcagccgctaccccgaccacatgaagcagcacgacttcttcaagtccgccatgcccgaaggctacatccaggagcgcaccatcttcttcaaggacgacggcaactacaagacccgcgccgaggtgaagttcgagggcgacaccctggtgaaccgcatcgagctgaagggcatcgacttcaaggaggacggcaacatcctggggcacaagctggagtacaacacgcgtaaggaggatttcaaccggatcctaagggacgtggaggcgaatacagtcagacttaaagaacatgaccaagatgtcttggtgctggagaaggtcccagcagggaacagagcttctaatcaaggaaactcacagcctcagcaaaagtatactgtgatgtcaggaacacctgaaaaaattttagagcattttctagaaacaatacgccttgaggcaactttaaatgaagcaacagattctgttttaaatgactttattatgatgcactgtgtttttatgccaaatacccagctttgcccggcactggtggcccactaccacgcacagccttcacaaggtacagaacaggagaaaatggattatgccctcaacaataagaggcgagtcatccgcctggttctacagtgggctgccatgtatggagacctcctgcaagaggatgacgtgtctatggccttcctggaggagttttatgtatctgtatcagatgatgcccggatgattgctgccctcaaggagcaactgccagagttggagaagattgtcaagcaaatctcagaagatgcaaaggcaccacaaaagaagcacaaggttcttttgcaacagttcaatacgggcgatgagagagcccagaagcgccagcctatccgcggctctgatgaagttctgtttaaggtctattgcatggaccccacctacacaaccattcgggtgccagtggccacttcggtgaaggaagtcatcagtgcagttgccgacaagctgggctccggggagggcctgatcatagtcaagatgagttccggaggagaaaaggtggtgctcaaacctaatgatgtttcagtatttatgacgctcaccattaatggacgcctgtttgcttgcccgcgagagcaattcgattcactgactcccttaccagaacaggaaggcccaactgttggaacagtgggaacttttgaactgatgagctccaaagatttagcataccagatgacaatttatgattgggaactcttcaactgcgtgcatgagctggagctaatctatcacacatttggaaggcataattttaaaaagaccacagcaaacttggatttgttcctgaggagatttaatgaaattcagttttgggtcgtcactgagatctgcctttgttctcagctcagcaagcgtgttcagctattaaaaaaatttattaagatagcagcccactgtaaggagtataaaaatctgaattccttttttgccatcgtcatgggactaagtaacgttgctgtgagccgcttggcactaacgtgggagaaactgccaagcaagttcaagaagttctatgcggagtttgaaagtttaatggacccttcaaggaaccacagggcctacaggctgacagtagctaagctggaacctcctctcatccccttcatgcctttgctcattaaagatatgacatttactcatgaggggaacaagacgttcattgacaatctagtaaactttgaaaaaatgcgcatgattgcaaatacggccagaacagtgagatactacaggagccaacccttcaatcctgatgcagctcaagctaataagaaccatcaggatgtccggagttatgtacggcaattaaatgtgattgacaaccagagaactttatcacagatgtcacacagattagagcctcgtcgacca

SEQ ID NO: 63 - DNA, 3759 bp, Artificial Sequence
  Synthetic
atggtcgctgcgcacgctgcccattcttcctcctctgccgagtggatcgcctgcctggataaaagaccactggagcgatccagcgaagatgtggatataatcttcactcgactgaaagaagttaaagcttttgagaaatttcacccaaatctccttcatcagatttgcttatgtggttattatgagaatctggaaaagggaataacattatttcgccagggtgatattggaacaaactggtatgctgtcctggcagggtctttggatgttaaagtatctgagaccagcagtcaccaggatgctgtgaccatctgtaccctgggaattgggacggcctttggagagtccattctggacaacacaccccgccatgcaaccatcgttaccagggagagcagtgaactgctccgcatcgagcagaaggacttcaaggcactatgggagaaatatcgacagtatatggcaggacttctggctcctccttatggtgttatggaaacgggctctaacaatgacaggattcctgacaaggagaacacacctctcattgaacctcacgttcctcttcgtcctgctaacaccattaccaaggtcccttcagagaagatcctcagagctggaaaaattttacgaaatgccattctctctcgagcacctcacatgataagagatagaaaataccacctaaagacatacagacaatgctgtgtgggaactgaactggtggactggatgatgcagcagacaccatgtgttcactcccggactcaagctgttggcatgtggcaagtcctgttagaagatggtgttctcaaccacgtggaccaggagcaccatttccaagacaaatatttattctatcgatttctggatgatgagcacgaggatgcccctttgcctactgaggaggagaagaaggagtgtgatgaggagctccaggacaccatgctgctgctgtcacagatgggccccgacgcccacatgaggatgatccttcgcaaaccacctggccagaggactgtggatgacctagagattatctatgaggagcttcttcatattaaagccttatcccatctttctaccacagtgaaacgagagttagcaggtgttctcatttttgagtctcacgccaaaggagggactgtgttgtttaaccagggggaagaaggtacctcctggtacattattctaaaaggatcagtgaatgtagtcatttacggcaagggtgtggtctgcaccctgcatgaaggagatgacttcggcaagttagcactagtgaatgatgccccacgagctgcctctatcgtcttacgagaagataactgccatttcttaagagtagacaaggaggatttcaaccggatcctaagggacgtgctcgagaacgtctatatcaaggccgacaagcagaagaacggcatcaaggcgaacttcaagatccgccacaacatcgaggacggcggcgtgcagctcgcctaccactaccagcagaacacccccatcggcgacggccccgtgctgctgcccgacaaccactacctgagcgtgcagtccatactttcgaaagaccccaacgagaagcgcgatcacatggtcctgctggagttcgtgaccgccgccgggatcactctcggcatggacgagctgtacaagggcggtaccggagggagcatggtgagcaagggcgaggagctgttcaccggggtggtgcccatccaggtcgagctggacggcgacgtaaacggccacaagttcagcgtgtccggcgagggtgagggcgatgccacctacggcaagctgaccctgaagttcatctgcaccaccggcaagctgcccgtgccctggcccaccctcgtgaccaccctgacctacggcgtgcagtgcttcagccgctaccccgaccacatgaagcagcacgacttcttcaagtccgccatgcccgaaggctacatccaggagcgcaccatcttcttcaaggacgacggcaactacaagacccgcgccgaggtgaagttcgagggcgacaccctggtgaaccgcatcgagctgaagggcatcgacttcaaggaggacggcaacatcctggggcacaagctggagtacaacacgcgtacagtcagacttaaagaacatgaccaagatgtcttggtgctggagaaggtcccagcagggaacagagcttctaatcaaggaaactcacagcctcagcaaaagtatactgtgatgtcaggaacacctgaaaaaattttagagcattttctagaaacaatacgccttgaggcaactttaaatgaagcaacagattctgttttaaatgactttattatgatgcactgtgtttttatgccaaatacccagctttgcccggcactggtggcccactaccacgcacagccttcacaaggtacagaacaggagaaaatggattatgccctcaacaataagaggcgagtcatccgcctggttctacagtgggctgccatgtatggagacctcctgcaagaggatgacgtgtctatggccttcctggaggagttttatgtatctgtatcagatgatgcccggatgattgctgccctcaaggagcaactgccagagttggagaagattgtcaagcaaatctcagaagatgcaaaggcaccacaaaagaagcacaaggttcttttgcaacagttcaatacgggcgatgagagagcccagaagcgccagcctatccgcggctctgatgaagttctgtttaaggtctattgcatggaccccacctacacaaccattcgggtgccagtggccacttcggtgaaggaagtcatcagtgcagttgccgacaagctgggctccggggagggcctgatcatagtcaagatgagttccggaggagaaaaggtggtgctcaaacctaatgatgtttcagtatttatgacgctcaccattaatggacgcctgtttgcttgcccgcgagagcaattcgattcactgactcccttaccagaacaggaaggcccaactgttggaacagtgggaacttttgaactgatgagctccaaagatttagcataccagatgacaatttatgattgggaactcttcaactgcgtgcatgagctggagctaatctatcacacatttggaaggcataattttaaaaagaccacagcaaacttggatttgttcctgaggagatttaatgaaattcagttttgggtcgtcactgagatctgcctttgttctcagctcagcaagcgtgttcagctattaaaaaaatttattaagatagcagcccactgtaaggagtataaaaatctgaattccttttttgccatcgtcatgggactaagtaacgttgctgtgagccgcttggcactaacgtgggagaaactgccaagcaagttcaagaagttctatgcggagtttgaaagtttaatggacccttcaaggaaccacagggcctacaggctgacagtagctaagctggaacctcctctcatccccttcatgcctttgctcattaaagatatgacatttactcatgaggggaacaagacgttcattgacaatctagtaaactttgaaaaaatgcgcatgattgcaaatacggccagaacagtgagatactacaggagccaacccttcaatcctgatgcagctcaagctaataagaaccatcaggatgtccggagttatgtacggcaattaaatgtgattgacaaccagagaactttatcacagatgtcacacagattagagcctcgtcgacca

SEQ ID NO: 64 - DNA, 3768 bp, Artificial Sequence
  Synthetic
atggtcgctgcgcacgctgcccattcttcctcctctgccgagtggatcgcctgcctggataaaagaccactggagcgatccagcgaagatgtggatataatcttcactcgactgaaagaagttaaagcttttgagaaatttcacccaaatctccttcatcagatttgcttatgtggttattatgagaatctggaaaagggaataacattatttcgccagggtgatattggaacaaactggtatgctgtcctggcagggtctttggatgttaaagtatctgagaccagcagtcaccaggatgctgtgaccatctgtaccctgggaattgggacggcctttggagagtccattctggacaacacaccccgccatgcaaccatcgttaccagggagagcagtgaactgctccgcatcgagcagaaggacttcaaggcactatgggagaaatatcgacagtatatggcaggacttctggctcctccttatggtgttatggaaacgggctctaacaatgacaggattcctgacaaggagaacacacctctcattgaacctcacgttcctcttcgtcctgctaacaccattaccaaggtcccttcagagaagatcctcagagctggaaaaattttacgaaatgccattctctctcgagcacctcacatgataagagatagaaaataccacctaaagacatacagacaatgctgtgtgggaactgaactggtggactggatgatgcagcagacaccatgtgttcactcccggactcaagctgttggcatgtggcaagtcctgttagaagatggtgttctcaaccacgtggaccaggagcaccatttccaagacaaatatttattctatcgatttctggatgatgagcacgaggatgcccctttgcctactgaggaggagaagaaggagtgtgatgaggagctccaggacaccatgctgctgctgtcacagatgggccccgacgcccacatgaggatgatccttcgcaaaccacctggccagaggactgtggatgacctagagattatctatgaggagcttcttcatattaaagccttatcccatctttctaccacagtgaaacgagagttagcaggtgttctcatttttgagtctcacgccaaaggagggactgtgttgtttaaccagggggaagaaggtacctcctggtacattattctaaaaggatcagtgaatgtagtcatttacggcaagggtgtggtctgcaccctgcatgaaggagatgacttcggcaagttagcactagtgaatgatgccccacgagctgcctctatcgtcttacgagaagataactgccatttcttaagagtagacaaggaggatttcaaccggatcctaaggatgtcgaacgtctatatcaaggccgacaagcagaagaacggcatcaaggcgaacttcaagatccgccacaacatcgaggacggcggcgtgcagctcgcctaccactaccagcagaacacccccatcggcgacggccccgtgctgctgcccgacaaccactacctgagcgtgcagtccatactttcgaaagaccccaacgagaagcgcgatcacatggtcctgctggagttcgtgaccgccgccgggatcactctcggcatggacgagctgtacaagggcggtaccggagggagcatggtgagcaagggcgaggagctgttcaccggggtggtgcccatccaggtcgagctggacggcgacgtaaacggccacaagttcagcgtgtccggcgagggtgagggcgatgccacctacggcaagctgaccctgaagttcatctgcaccaccggcaagctgcccgtgccctggcccaccctcgtgaccaccctgacctacggcgtgcagtgcttcagccgctaccccgaccacatgaagcagcacgacttcttcaagtccgccatgcccgaaggctacatccaggagcgcaccatcttcttcaaggacgacggcaactacaagacccgcgccgaggtgaagttcgagggcgacaccctggtgaaccgcatcgagctgaagggcatcgacttcaaggaggacggcaacatcctggggcacaagctggagtacaacgtatcagacgtggaggcgaatacagtcagacttaaagaacatgaccaagatgtcttggtgctggagaaggtcccagcagggaacagagcttctaatcaaggaaactcacagcctcagcaaaagtatactgtgatgtcaggaacacctgaaaaaattttagagcattttctagaaacaatacgccttgaggcaactttaaatgaagcaacagattctgttttaaatgactttattatgatgcactgtgtttttatgccaaatacccagctttgcccggcactggtggcccactaccacgcacagccttcacaaggtacagaacaggagaaaatggattatgccctcaacaataagaggcgagtcatccgcctggttctacagtgggctgccatgtatggagacctcctgcaagaggatgacgtgtctatggccttcctggaggagttttatgtatctgtatcagatgatgcccggatgattgctgccctcaaggagcaactgccagagttggagaagattgtcaagcaaatctcagaagatgcaaaggcaccacaaaagaagcacaaggttcttttgcaacagttcaatacgggcgatgagagagcccagaagcgccagcctatccgcggctctgatgaagttctgtttaaggtctattgcatggaccccacctacacaaccattcgggtgccagtggccacttcggtgaaggaagtcatcagtgcagttgccgacaagctgggctccggggagggcctgatcatagtcaagatgagttccggaggagaaaaggtggtgctcaaacctaatgatgtttcagtatttatgacgctcaccattaatggacgcctgtttgcttgcccgcgagagcaattcgattcactgactcccttaccagaacaggaaggcccaactgttggaacagtgggaacttttgaactgatgagctccaaagatttagcataccagatgacaatttatgattgggaactcttcaactgcgtgcatgagctggagctaatctatcacacatttggaaggcataattttaaaaagaccacagcaaacttggatttgttcctgaggagatttaatgaaattcagttttgggtcgtcactgagatctgcctttgttctcagctcagcaagcgtgttcagctattaaaaaaatttattaagatagcagcccactgtaaggagtataaaaatctgaattccttttttgccatcgtcatgggactaagtaacgttgctgtgagccgcttggcactaacgtgggagaaactgccaagcaagttcaagaagttctatgcggagtttgaaagtttaatggacccttcaaggaaccacagggcctacaggctgacagtagctaagctggaacctcctctcatccccttcatgcctttgctcattaaagatatgacatttactcatgaggggaacaagacgttcattgacaatctagtaaactttgaaaaaatgcgcatgattgcaaatacggccagaacagtgagatactacaggagccaacccttcaatcctgatgcagctcaagctaataagaaccatcaggatgtccggagttatgtacggcaattaaatgtgattgacaaccagagaactttatcacagatgtcacacagattagagcctcgtcgacca

SEQ ID NO: 65 - DNA, 3768 bp, Artificial Sequence
  Synthetic
atggtcgctgcgcacgctgcccattcttcctcctctgccgagtggatcgcctgcctggataaaagaccactggagcgatccagcgaagatgtggatataatcttcactcgactgaaagaagttaaagcttttgagaaatttcacccaaatctccttcatcagatttgcttatgtggttattatgagaatctggaaaagggaataacattatttcgccagggtgatattggaacaaactggtatgctgtcctggcagggtctttggatgttaaagtatctgagaccagcagtcaccaggatgctgtgaccatctgtaccctgggaattgggacggcctttggagagtccattctggacaacacaccccgccatgcaaccatcgttaccagggagagcagtgaactgctccgcatcgagcagaaggacttcaaggcactatgggagaaatatcgacagtatatggcaggacttctggctcctccttatggtgttatggaaacgggctctaacaatgacaggattcctgacaaggagaacacacctctcattgaacctcacgttcctcttcgtcctgctaacaccattaccaaggtcccttcagagaagatcctcagagctggaaaaattttacgaaatgccattctctctcgagcacctcacatgataagagatagaaaataccacctaaagacatacagacaatgctgtgtgggaactgaactggtggactggatgatgcagcagacaccatgtgttcactcccggactcaagctgttggcatgtggcaagtcctgttagaagatggtgttctcaaccacgtggaccaggagcaccatttccaagacaaatatttattctatcgatttctggatgatgagcacgaggatgcccctttgcctactgaggaggagaagaaggagtgtgatgaggagctccaggacaccatgctgctgctgtcacagatgggccccgacgcccacatgaggatgatccttcgcaaaccacctggccagaggactgtggatgacctagagattatctatgaggagcttcttcatattaaagccttatcccatctttctaccacagtgaaacgagagttagcaggtgttctcatttttgagtctcacgccaaaggagggactgtgttgtttaaccagggggaagaaggtacctcctggtacattattctaaaaggatcagtgaatgtagtcatttacggcaagggtgtggtctgcaccctgcatgaaggagatgacttcggcaagttagcactagtgaatgatgccccacgagctgcctctatcgtcttacgagaagataactgccatttcttaagagtagacaaggaggatttcaaccggatcctaaggctcgagaacgtctatatcaaggccgacaagcagaagaacggcatcaaggcgaacttcaagatccgccacaacatcgaggacggcggcgtgcagctcgcctaccactaccagcagaacacccccatcggcgacggccccgtgctgctgcccgacaaccactacctgagcgtgcagtccatactttcgaaagaccccaacgagaagcgcgatcacatggtcctgctggagttcgtgaccgccgccgggatcactctcggcatggacgagctgtacaagggcggtaccggagggagcatggtgagcaagggcgaggagctgttcaccggggtggtgcccatccaggtcgagctggacggcgacgtaaacggccacaagttcagcgtgtccggcgagggtgagggcgatgccacctacggcaagctgaccctgaagttcatctgcaccaccggcaagctgcccgtgccctggcccaccctcgtgaccaccctgacctacggcgtgcagtgcttcagccgctaccccgaccacatgaagcagcacgacttcttcaagtccgccatgcccgaaggctacatccaggagcgcaccatcttcttcaaggacgacggcaactacaagacccgcgccgaggtgaagttcgagggcgacaccctggtgaaccgcatcgagctgaagggcatcgacttcaaggaggacggcaacatcctggggcacaagctggagtacaacacgcgtgacgtggaggcgaatacagtcagacttaaagaacatgaccaagatgtcttggtgctggagaaggtcccagcagggaacagagcttctaatcaaggaaactcacagcctcagcaaaagtatactgtgatgtcaggaacacctgaaaaaattttagagcattttctagaaacaatacgccttgaggcaactttaaatgaagcaacagattctgttttaaatgactttattatgatgcactgtgtttttatgccaaatacccagctttgcccggcactggtggcccactaccacgcacagccttcacaaggtacagaacaggagaaaatggattatgccctcaacaataagaggcgagtcatccgcctggttctacagtgggctgccatgtatggagacctcctgcaagaggatgacgtgtctatggccttcctggaggagttttatgtatctgtatcagatgatgcccggatgattgctgccctcaaggagcaactgccagagttggagaagattgtcaagcaaatctcagaagatgcaaaggcaccacaaaagaagcacaaggttcttttgcaacagttcaatacgggcgatgagagagcccagaagcgccagcctatccgcggctctgatgaagttctgtttaaggtctattgcatggaccccacctacacaaccattcgggtgccagtggccacttcggtgaaggaagtcatcagtgcagttgccgacaagctgggctccggggagggcctgatcatagtcaagatgagttccggaggagaaaaggtggtgctcaaacctaatgatgtttcagtatttatgacgctcaccattaatggacgcctgtttgcttgcccgcgagagcaattcgattcactgactcccttaccagaacaggaaggcccaactgttggaacagtgggaacttttgaactgatgagctccaaagatttagcataccagatgacaatttatgattgggaactcttcaactgcgtgcatgagctggagctaatctatcacacatttggaaggcataattttaaaaagaccacagcaaacttggatttgttcctgaggagatttaatgaaattcagttttgggtcgtcactgagatctgcctttgttctcagctcagcaagcgtgttcagctattaaaaaaatttattaagatagcagcccactgtaaggagtataaaaatctgaattccttttttgccatcgtcatgggactaagtaacgttgctgtgagccgcttggcactaacgtgggagaaactgccaagcaagttcaagaagttctatgcggagtttgaaagtttaatggacccttcaaggaaccacagggcctacaggctgacagtagctaagctggaacctcctctcatccccttcatgcctttgctcattaaagatatgacatttactcatgaggggaacaagacgttcattgacaatctagtaaactttgaaaaaatgcgcatgattgcaaatacggccagaacagtgagatactacaggagccaacccttcaatcctgatgcagctcaagctaataagaaccatcaggatgtccggagttatgtacggcaattaaatgtgattgacaaccagagaactttatcacagatgtcacacagattagagcctcgtcgacca

SEQ ID NO: 66 - DNA, 3774 bp, Artificial Sequence
  Synthetic
atggtcgctgcgcacgctgcccattcttcctcctctgccgagtggatcgcctgcctggataaaagaccactggagcgatccagcgaagatgtggatataatcttcactcgactgaaagaagttaaagcttttgagaaatttcacccaaatctccttcatcagatttgcttatgtggttattatgagaatctggaaaagggaataacattatttcgccagggtgatattggaacaaactggtatgctgtcctggcagggtctttggatgttaaagtatctgagaccagcagtcaccaggatgctgtgaccatctgtaccctgggaattgggacggcctttggagagtccattctggacaacacaccccgccatgcaaccatcgttaccagggagagcagtgaactgctccgcatcgagcagaaggacttcaaggcactatgggagaaatatcgacagtatatggcaggacttctggctcctccttatggtgttatggaaacgggctctaacaatgacaggattcctgacaaggagaacacacctctcattgaacctcacgttcctcttcgtcctgctaacaccattaccaaggtcccttcagagaagatcctcagagctggaaaaattttacgaaatgccattctctctcgagcacctcacatgataagagatagaaaataccacctaaagacatacagacaatgctgtgtgggaactgaactggtggactggatgatgcagcagacaccatgtgttcactcccggactcaagctgttggcatgtggcaagtcctgttagaagatggtgttctcaaccacgtggaccaggagcaccatttccaagacaaatatttattctatcgatttctggatgatgagcacgaggatgcccctttgcctactgaggaggagaagaaggagtgtgatgaggagctccaggacaccatgctgctgctgtcacagatgggccccgacgcccacatgaggatgatccttcgcaaaccacctggccagaggactgtggatgacctagagattatctatgaggagcttcttcatattaaagccttatcccatctttctaccacagtgaaacgagagttagcaggtgttctcatttttgagtctcacgccaaaggagggactgtgttgtttaaccagggggaagaaggtacctcctggtacattattctaaaaggatcagtgaatgtagtcatttacggcaagggtgtggtctgcaccctgcatgaaggagatgacttcggcaagttagcactagtgaatgatgccccacgagctgcctctatcgtcttacgagaagataactgccatttcttaagagtagacaaggaggatttcaaccggatcctaaggctggtgtcgcacaacgtctatatcaaggccgacaagcagaagaacggcatcaaggcgaacttcaagatccgccacaacatcgaggacggcggcgtgcagctcgcctaccactaccagcagaacacccccatcggcgacggccccgtgctgctgcccgacaaccactacctgagcgtgcagtccatactttcgaaagaccccaacgagaagcgcgatcacatggtcctgctggagttcgtgaccgccgccgggatcactctcggcatggacgagctgtacaagggcggtaccggagggagcatggtgagcaagggcgaggagctgttcaccggggtggtgcccatccaggtcgagctggacggcgacgtaaacggccacaagttcagcgtgtccggcgagggtgagggcgatgccacctacggcaagctgaccctgaagttcatctgcaccaccggcaagctgcccgtgccctggcccaccctcgtgaccaccctgacctacggcgtgcagtgcttcagccgctaccccgaccacatgaagcagcacgacttcttcaagtccgccatgcccgaaggctacatccaggagcgcaccatcttcttcaaggacgacggcaactacaagacccgcgccgaggtgaagttcgagggcgacaccctggtgaaccgcatcgagctgaagggcatcgacttcaaggaggacggcaacatcctggggcacaagctggagtacaacttcaacgacgtggaggcgaatacagtcagacttaaagaacatgaccaagatgtcttggtgctggagaaggtcccagcagggaacagagcttctaatcaaggaaactcacagcctcagcaaaagtatactgtgatgtcaggaacacctgaaaaaattttagagcattttctagaaacaatacgccttgaggcaactttaaatgaagcaacagattctgttttaaatgactttattatgatgcactgtgtttttatgccaaatacccagctttgcccggcactggtggcccactaccacgcacagccttcacaaggtacagaacaggagaaaatggattatgccctcaacaataagaggcgagtcatccgcctggttctacagtgggctgccatgtatggagacctcctgcaagaggatgacgtgtctatggccttcctggaggagttttatgtatctgtatcagatgatgcccggatgattgctgccctcaaggagcaactgccagagttggagaagattgtcaagcaaatctcagaagatgcaaaggcaccacaaaagaagcacaaggttcttttgcaacagttcaatacgggcgatgagagagcccagaagcgccagcctatccgcggctctgatgaagttctgtttaaggtctattgcatggaccccacctacacaaccattcgggtgccagtggccacttcggtgaaggaagtcatcagtgcagttgccgacaagctgggctccggggagggcctgatcatagtcaagatgagttccggaggagaaaaggtggtgctcaaacctaatgatgtttcagtatttatgacgctcaccattaatggacgcctgtttgcttgcccgcgagagcaattcgattcactgactcccttaccagaacaggaaggcccaactgttggaacagtgggaacttttgaactgatgagctccaaagatttagcataccagatgacaatttatgattgggaactcttcaactgcgtgcatgagctggagctaatctatcacacatttggaaggcataattttaaaaagaccacagcaaacttggatttgttcctgaggagatttaatgaaattcagttttgggtcgtcactgagatctgcctttgttctcagctcagcaagcgtgttcagctattaaaaaaatttattaagatagcagcccactgtaaggagtataaaaatctgaattccttttttgccatcgtcatgggactaagtaacgttgctgtgagccgcttggcactaacgtgggagaaactgccaagcaagttcaagaagttctatgcggagtttgaaagtttaatggacccttcaaggaaccacagggcctacaggctgacagtagctaagctggaacctcctctcatccccttcatgcctttgctcattaaagatatgacatttactcatgaggggaacaagacgttcattgacaatctagtaaactttgaaaaaatgcgcatgattgcaaatacggccagaacagtgagatactacaggagccaacccttcaatcctgatgcagctcaagctaataagaaccatcaggatgtccggagttatgtacggcaattaaatgtgattgacaaccagagaactttatcacagatgtcacacagattagagcctcgtcgacca

SEQ ID NO: 67 - DNA, 4317 bp, Artificial Sequence
  Synthetic
atggtcgctgcgcacgctgcccattcttcctcctctgccgagtggatcgcctgcctggataaaagaccactggagcgatccagcgaagatgtggatataatcttcactcgactgaaagaagttaaagcttttgagaaatttcacccaaatctccttcatcagatttgcttatgtggttattatgagaatctggaaaagggaataacattatttcgccagggtgatattggaacaaactggtatgctgtcctggcagggtctttggatgttaaagtatctgagaccagcagtcaccaggatgctgtgaccatctgtaccctgggaattgggacggcctttggagagtccattctggacaacacaccccgccatgcaaccatcgttaccagggagagcagtgaactgctccgcatcgagcagaaggacttcaaggcactatgggagaaatatcgacagtatatggcaggacttctggctcctccttatggtgttatggaaacgggctctaacaatgacaggattcctgacaaggagaacacacctctcattgaacctcacgttcctcttcgtcctgctaacaccattaccaaggtcccttcagagaagatcctcagagctggaaaaattttacgaaatgccattctctctcgagcacctcacatgataagagatagaaaataccacctaaagacatacagacaatgctgtgtgggaactgaactggtggactggatgatgcagcagacaccatgtgttcactcccggactcaagctgttggcatgtggcaagtcctgttagaagatggtgttctcaaccacgtggaccaggagcaccatttccaagacaaatatttattctatcgatttctggatgatgagcacgaggatgcccctttgcctactgaggaggagaagaaggagtgtgatgaggagctccaggacaccatgctgctgctgtcacagatgggccccgacgcccacatgaggatgatccttcgcaaaccacctggccagaggactgtggatgacctagagattatctatgaggagcttcttcatattaaagccttatcccatctttctaccacagtgaaacgagagttagcaggtgttctcatttttgagtctcacgccaaaggagggactgtgttgtttaaccagggggaagaaggtacctcctggtacattattctaaaaggatcagtgaatgtagtcatttacggcaagggtgtggtctgcaccctgcatgaaggagatgacttcggcaagttagcactagtgaatgatgccccacgagctgcctctatcgtcttacgagaagataactgccatttcttaagagtagacaaggaggatttcaaccggatcctaagggacgtggaggcgaatacagtcagacttaaagaacatgaccaagatgtcttggtgctggagaaggtcccagcagggaacagagcttctaatcaaggaaactcacagcctcagcaaaagtatactgtgatgtcaggaacacctgaaaaaattttagagcattttctagaaacaatacgccttgaggcaactttaaatgaagcaacagattctgttttaaatgactttattatgatgcactgtgtttttatgccaaatacccagctttgcccggcactggtggcccactaccacgcacagccttcacaaggtacagaacaggagaaaatggattatgccctcaacaataagaggcgagtcatccgcctggttctacagtgggctgccatgtatggagacctcctgcaagaggatgacgtgtctatggccttcctggaggagttttatgtatctgtatcagatgatgcccggatgattgctgccctcaaggagcaactgccagagttggagaagattgtcaagcaaatctcagaagatgcaaaggcaccacaaaagaagcacaaggttcttttgcaacagttcaatacgggcgatgagagagcccagaagcgccagcctatccgcggctctgatgaagttctgtttaaggtctattgcatggaccccacctacacaaccattcgggtgccagtggccacttcggtgaaggaagtcatcagtgcagttgccgacaagctgggctccggggagggcctgatcatagtcaagatgagttccggaggagaaaaggtggtgctcaaacctaatgatgtttcagtatttatgacgctcaccattaatggacgcctgtttgcttgcccgcgagagcaattcgattcactgactcccttaccagaacaggaaggcccaactgttggaacagtgggaacttttgaactgatgagctccaaagatttagcataccagatgacaatttatgattgggaactcttcaactgcgtgcatgagctggagctaatctatcacacatttggaaggcataattttaaaaagaccacagcaaacttggatttgttcctgaggagatttaatgaaattcagttttgggtcgtcactgagatctgcctttgttctcagctcagcaagcgtgttcagctattaaaaaaatttattaagatagcagcccactgtaaggagtataaaaatctgaattccttttttgccatcgtcatgggactaagtaacgttgctgtgagccgcttggcactaacgtgggagaaactgccaagcaagttcaagaagttctatgcggagtttgaaagtttaatggacccttcaaggaaccacagggcctacaggctgacagtagctaagctggaacctcctctcatccccttcatgcctttgctcattaaagatatgacatttactcatgaggggaacaagacgttcattgacaatctagtaaactttgaaaaaatgcgcatgattgcaaatacggccagaacagtgagatactacaggagccaacccttcaatcctgatgcagctcaagctaataagaaccatcaggatgtccggagttatgtacggcaattaaatgtgattgacaaccagagaactttatcacagatgtcacacagattagagcctcgtcgaccactcgagaacgtctatatcaaggccgacaagcagaagaacggcatcaaggcgaacttcaagatccgccacaacatcgaggacggcggcgtgcagctcgcctaccactaccagcagaacacccccatcggcgacggccccgtgctgctgcccgacaaccactacctgagcgtgcagtccatactttcgaaagaccccaacgagaagcgcgatcacatggtcctgctggagttcgtgaccgccgccgggatcactctcggcatggacgagctgtacaagggcggtaccggagggagcatggtgagcaagggcgaggagctgttcaccggggtggtgcccatccaggtcgagctggacggcgacgtaaacggccacaagttcagcgtgtccggcgagggtgagggcgatgccacctacggcaagctgaccctgaagttcatctgcaccaccggcaagctgcccgtgccctggcccaccctcgtgaccaccctgacctacggcgtgcagtgcttcagccgctaccccgaccacatgaagcagcacgacttcttcaagtccgccatgcccgaaggctacatccaggagcgcaccatcttcttcaaggacgacggcaactacaagacccgcgccgaggtgaagttcgagggcgacaccctggtgaaccgcatcgagctgaagggcatcgacttcaaggaggacggcaacatcctggggcacaagctggagtacaacacgcgtcgtgagtataagctagtcgttcttggctcaggaggcgttggaaagtctgctttgactgtacaatttgttcaaggaatttttgtagaaaaatacgatcctacgatagaagattcttatagaaagcaagttgaagtagatgcacaacagtgtatgcttgaaatcttggatactgcaggaacggagcaatttacagcaatgagggatttatacatgaaaaatggacaaggatttgcattagtttattccatcacagcacagtccacatttaacgatttacaagacctgagagaacagattcttcgagttaaagacactgatgatgttccaatgattcttgttggtaataagtgtgacttggaagatgaaagagttgtagggaaggaacaaggtcaaaatctagcaagacaatggaacaactgtgcattcttagaatcttctgcaaaatcaaaaataaatgttaatgagatcttttatgacctagtgcggcaaattaacagaaaaactccagtgcctgggaaggctcgcaaaaagtcatcatgtcagctgctt

SEQ ID NO: 68 - DNA, 3768 bp, Artificial Sequence
  Synthetic
atggtcgctgcgcacgctgcccattcttcctcctctgccgagtggatcgcctgcctggataaaagaccactggagcgatccagcgaagatgtggatataatcttcactcgactgaaagaagttaaagcttttgagaaatttcacccaaatctccttcatcagatttgcttatgtggttattatgagaatctggaaaagggaataacattatttcgccagggtgatattggaacaaactggtatgctgtcctggcagggtctttggatgttaaagtatctgagaccagcagtcaccaggatgctgtgaccatctgtaccctgggaattgggacggcctttggagagtccattctggacaacacaccccgccatgcaaccatcgttaccagggagagcagtgaactgctccgcatcgagcagaaggacttcaaggcactatgggagaaatatcgacagtatatggcaggacttctggctcctccttatggtgttatggaaacgggctctaacaatgacaggattcctgacaaggagaacacacctctcattgaacctcacgttcctcttcgtcctgctaacaccattaccaaggtcccttcagagaagatcctcagagctggaaaaattttacgaaatgccattctctctcgagcacctcacatgataagagatagaaaataccacctaaagacatacagacaatgctgtgtgggaactgaactggtggactggatgatgcagcagacaccatgtgttcactcccggactcaagctgttggcatgtggcaagtcctgttagaagatggtgttctcaaccacgtggaccaggagcaccatttccaagacaaatatttattctatcgatttctggatgatgagcacgaggatgcccctttgcctactgaggaggagaagaaggagtgtgatgaggagctccaggacaccatgctgctgctgtcacagatgggccccgacgcccacatgaggatgatccttcgcaaaccacctggccagaggactgtggatgacctagagattatctatgaggagcttcttcatattaaagccttatcccatctttctaccacagtgaaacgagagttagcaggtgttctcatttttgagtctcacgccaaaggagggactgtgttgtttaaccagggggaagaaggtacctcctggtacattattctaaaaggatcagtgaatgtagtcatttacggcaagggtgtggtctgcaccctgcatgaaggagatgacttcggcaagttagcactagtgaatgatgccccacgagctgcctctatcgtcttacgagaagataactgccatttcttaagagtagacaaggaggatttcaaccggatcctaagggacgtggagctcgagaacgtctatatcaaggccgacaagcagaagaacggcatcaaggcgaacttcaagatccgccacaacatcgaggacggcggcgtgcagctcgcctaccactaccagcagaacacccccatcggcgacggccccgtgctgctgcccgacaaccactacctgagcgtgcagtccatactttcgaaagaccccaacgagaagcgcgatcacatggtcctgctggagttcgtgaccgccgccgggatcactctcggcatggacgagctgtacaagggcggtaccggagggagcatggtgagcaagggcgaggagctgttcaccggggtggtgcccatccaggtcgagctggacggcgacgtaaacggccacaagttcagcgtgtccggcgagggtgagggcgatgccacctacggcaagctgaccctgaagttcatctgcaccaccggcaagctgcccgtgccctggcccaccctcgtgaccaccctgacctacggcgtgcagtgcttcagccgctaccccgaccacatgaagcagcacgacttcttcaagtccgccatgcccgaaggctacatccaggagcgcaccatcttcttcaaggacgacggcaactacaagacccgcgccgaggtgaagttcgagggcgacaccctggtgaaccgcatcgagctgaagggcatcgacttcaaggaggacggcaacatcctggggcacaagctggagtacaacacgcgtgcgaatacagtcagacttaaagaacatgaccaagatgtcttggtgctggagaaggtcccagcagggaacagagcttctaatcaaggaaactcacagcctcagcaaaagtatactgtgatgtcaggaacacctgaaaaaattttagagcattttctagaaacaatacgccttgaggcaactttaaatgaagcaacagattctgttttaaatgactttattatgatgcactgtgtttttatgccaaatacccagctttgcccggcactggtggcccactaccacgcacagccttcacaaggtacagaacaggagaaaatggattatgccctcaacaataagaggcgagtcatccgcctggttctacagtgggctgccatgtatggagacctcctgcaagaggatgacgtgtctatggccttcctggaggagttttatgtatctgtatcagatgatgcccggatgattgctgccctcaaggagcaactgccagagttggagaagattgtcaagcaaatctcagaagatgcaaaggcaccacaaaagaagcacaaggttcttttgcaacagttcaatacgggcgatgagagagcccagaagcgccagcctatccgcggctctgatgaagttctgtttaaggtctattgcatggaccccacctacacaaccattcgggtgccagtggccacttcggtgaaggaagtcatcagtgcagttgccgacaagctgggctccggggagggcctgatcatagtcaagatgagttccggaggagaaaaggtggtgctcaaacctaatgatgtttcagtatttatgacgctcaccattaatggacgcctgtttgcttgcccgcgagagcaattcgattcactgactcccttaccagaacaggaaggcccaactgttggaacagtgggaacttttgaactgatgagctccaaagatttagcataccagatgacaatttatgattgggaactcttcaactgcgtgcatgagctggagctaatctatcacacatttggaaggcataattttaaaaagaccacagcaaacttggatttgttcctgaggagatttaatgaaattcagttttgggtcgtcactgagatctgcctttgttctcagctcagcaagcgtgttcagctattaaaaaaatttattaagatagcagcccactgtaaggagtataaaaatctgaattccttttttgccatcgtcatgggactaagtaacgttgctgtgagccgcttggcactaacgtgggagaaactgccaagcaagttcaagaagttctatgcggagtttgaaagtttaatggacccttcaaggaaccacagggcctacaggctgacagtagctaagctggaacctcctctcatccccttcatgcctttgctcattaaagatatgacatttactcatgaggggaacaagacgttcattgacaatctagtaaactttgaaaaaatgcgcatgattgcaaatacggccagaacagtgagatactacaggagccaacccttcaatcctgatgcagctcaagctaataagaaccatcaggatgtccggagttatgtacggcaattaaatgtgattgacaaccagagaactttatcacagatgtcacacagattagagcctcgtcgacca

SEQ ID NO: 69 - DNA, 3768 bp, Artificial Sequence
  Synthetic
atggtcgctgcgcacgctgcccattcttcctcctctgccgagtggatcgcctgcctggataaaagaccactggagcgatccagcgaagatgtggatataatcttcactcgactgaaagaagttaaagcttttgagaaatttcacccaaatctccttcatcagatttgcttatgtggttattatgagaatctggaaaagggaataacattatttcgccagggtgatattggaacaaactggtatgctgtcctggcagggtctttggatgttaaagtatctgagaccagcagtcaccaggatgctgtgaccatctgtaccctgggaattgggacggcctttggagagtccattctggacaacacaccccgccatgcaaccatcgttaccagggagagcagtgaactgctccgcatcgagcagaaggacttcaaggcactatgggagaaatatcgacagtatatggcaggacttctggctcctccttatggtgttatggaaacgggctctaacaatgacaggattcctgacaaggagaacacacctctcattgaacctcacgttcctcttcgtcctgctaacaccattaccaaggtcccttcagagaagatcctcagagctggaaaaattttacgaaatgccattctctctcgagcacctcacatgataagagatagaaaataccacctaaagacatacagacaatgctgtgtgggaactgaactggtggactggatgatgcagcagacaccatgtgttcactcccggactcaagctgttggcatgtggcaagtcctgttagaagatggtgttctcaaccacgtggaccaggagcaccatttccaagacaaatatttattctatcgatttctggatgatgagcacgaggatgcccctttgcctactgaggaggagaagaaggagtgtgatgaggagctccaggacaccatgctgctgctgtcacagatgggccccgacgcccacatgaggatgatccttcgcaaaccacctggccagaggactgtggatgacctagagattatctatgaggagcttcttcatattaaagccttatcccatctttctaccacagtgaaacgagagttagcaggtgttctcatttttgagtctcacgccaaaggagggactgtgttgtttaaccagggggaagaaggtacctcctggtacattattctaaaaggatcagtgaatgtagtcatttacggcaagggtgtggtctgcaccctgcatgaaggagatgacttcggcaagttagcactagtgaatgatgccccacgagctgcctctatcgtcttacgagaagataactgccatttcttaagagtagacaaggaggatttcaaccggatcctaagggacgtggaggcgaatacagtcagacttaaagaacatgaccaagatgtcttggtgctggagaaggtcccagcagggaacagagcttctaatcaaggaaactcacagcctcagcaaaagtatactgtgatgtcaggaacacctgaaaaaattttagagcattttctagaaacaatacgccttctcgagaacgtctatatcaaggccgacaagcagaagaacggcatcaaggcgaacttcaagatccgccacaacatcgaggacggcggcgtgcagctcgcctaccactaccagcagaacacccccatcggcgacggccccgtgctgctgcccgacaaccactacctgagcgtgcagtccatactttcgaaagaccccaacgagaagcgcgatcacatggtcctgctggagttcgtgaccgccgccgggatcactctcggcatggacgagctgtacaagggcggtaccggagggagcatggtgagcaagggcgaggagctgttcaccggggtggtgcccatccaggtcgagctggacggcgacgtaaacggccacaagttcagcgtgtccggcgagggtgagggcgatgccacctacggcaagctgaccctgaagttcatctgcaccaccggcaagctgcccgtgccctggcccaccctcgtgaccaccctgacctacggcgtgcagtgcttcagccgctaccccgaccacatgaagcagcacgacttcttcaagtccgccatgcccgaaggctacatccaggagcgcaccatcttcttcaaggacgacggcaactacaagacccgcgccgaggtgaagttcgagggcgacaccctggtgaaccgcatcgagctgaagggcatcgacttcaaggaggacggcaacatcctggggcacaagctggagtacaacacgcgtgaggcaactttaaatgaagcaacagattctgttttaaatgactttattatgatgcactgtgtttttatgccaaatacccagctttgcccggcactggtggcccactaccacgcacagccttcacaaggtacagaacaggagaaaatggattatgccctcaacaataagaggcgagtcatccgcctggttctacagtgggctgccatgtatggagacctcctgcaagaggatgacgtgtctatggccttcctggaggagttttatgtatctgtatcagatgatgcccggatgattgctgccctcaaggagcaactgccagagttggagaagattgtcaagcaaatctcagaagatgcaaaggcaccacaaaagaagcacaaggttcttttgcaacagttcaatacgggcgatgagagagcccagaagcgccagcctatccgcggctctgatgaagttctgtttaaggtctattgcatggaccccacctacacaaccattcgggtgccagtggccacttcggtgaaggaagtcatcagtgcagttgccgacaagctgggctccggggagggcctgatcatagtcaagatgagttccggaggagaaaaggtggtgctcaaacctaatgatgtttcagtatttatgacgctcaccattaatggacgcctgtttgcttgcccgcgagagcaattcgattcactgactcccttaccagaacaggaaggcccaactgttggaacagtgggaacttttgaactgatgagctccaaagatttagcataccagatgacaatttatgattgggaactcttcaactgcgtgcatgagctggagctaatctatcacacatttggaaggcataattttaaaaagaccacagcaaacttggatttgttcctgaggagatttaatgaaattcagttttgggtcgtcactgagatctgcctttgttctcagctcagcaagcgtgttcagctattaaaaaaatttattaagatagcagcccactgtaaggagtataaaaatctgaattccttttttgccatcgtcatgggactaagtaacgttgctgtgagccgcttggcactaacgtgggagaaactgccaagcaagttcaagaagttctatgcggagtttgaaagtttaatggacccttcaaggaaccacagggcctacaggctgacagtagctaagctggaacctcctctcatccccttcatgcctttgctcattaaagatatgacatttactcatgaggggaacaagacgttcattgacaatctagtaaactttgaaaaaatgcgcatgattgcaaatacggccagaacagtgagatactacaggagccaacccttcaatcctgatgcagctcaagctaataagaaccatcaggatgtccggagttatgtacggcaattaaatgtgattgacaaccagagaactttatcacagatgtcacacagattagagcctcgtcgacca

SEQ ID NO: 70 - DNA, 3768 bp, Artificial Sequence
  Synthetic
atggtcgctgcgcacgctgcccattcttcctcctctgccgagtggatcgcctgcctggataaaagaccactggagcgatccagcgaagatgtggatataatcttcactcgactgaaagaagttaaagcttttgagaaatttcacccaaatctccttcatcagatttgcttatgtggttattatgagaatctggaaaagggaataacattatttcgccagggtgatattggaacaaactggtatgctgtcctggcagggtctttggatgttaaagtatctgagaccagcagtcaccaggatgctgtgaccatctgtaccctgggaattgggacggcctttggagagtccattctggacaacacaccccgccatgcaaccatcgttaccagggagagcagtgaactgctccgcatcgagcagaaggacttcaaggcactatgggagaaatatcgacagtatatggcaggacttctggctcctccttatggtgttatggaaacgggctctaacaatgacaggattcctgacaaggagaacacacctctcattgaacctcacgttcctcttcgtcctgctaacaccattaccaaggtcccttcagagaagatcctcagagctggaaaaattttacgaaatgccattctctctcgagcacctcacatgataagagatagaaaataccacctaaagacatacagacaatgctgtgtgggaactgaactggtggactggatgatgcagcagacaccatgtgttcactcccggactcaagctgttggcatgtggcaagtcctgttagaagatggtgttctcaaccacgtggaccaggagcaccatttccaagacaaatatttattctatcgatttctggatgatgagcacgaggatgcccctttgcctactgaggaggagaagaaggagtgtgatgaggagctccaggacaccatgctgctgctgtcacagatgggccccgacgcccacatgaggatgatccttcgcaaaccacctggccagaggactgtggatgacctagagattatctatgaggagcttcttcatattaaagccttatcccatctttctaccacagtgaaacgagagttagcaggtgttctcatttttgagtctcacgccaaaggagggactgtgttgtttaaccagggggaagaaggtacctcctggtacattattctaaaaggatcagtgaatgtagtcatttacggcaagggtgtggtctgcaccctgcatgaaggagatgacttcggcaagttagcactagtgaatgatgccccacgagctgcctctatcgtcttacgagaagataactgccatttcttaagagtagacaaggaggatttcaaccggatcctactcgagaacgtctatatcaaggccgacaagcagaagaacggcatcaaggcgaacttcaagatccgccacaacatcgaggacggcggcgtgcagctcgcctaccactaccagcagaacacccccatcggcgacggccccgtgctgctgcccgacaaccactacctgagcgtgcagtccatactttcgaaagaccccaacgagaagcgcgatcacatggtcctgctggagttcgtgaccgccgccgggatcactctcggcatggacgagctgtacaagggcggtaccggagggagcatggtgagcaagggcgaggagctgttcaccggggtggtgcccatccaggtcgagctggacggcgacgtaaacggccacaagttcagcgtgtccggcgagggtgagggcgatgccacctacggcaagctgaccctgaagttcatctgcaccaccggcaagctgcccgtgccctggcccaccctcgtgaccaccctgacctacggcgtgcagtgcttcagccgctaccccgaccacatgaagcagcacgacttcttcaagtccgccatgcccgaaggctacatccaggagcgcaccatcttcttcaaggacgacggcaactacaagacccgcgccgaggtgaagttcgagggcgacaccctggtgaaccgcatcgagctgaagggcatcgacttcaaggaggacggcaacatcctggggcacaagctggagtacaacacgcgtagggacgtggaggcgaatacagtcagacttaaagaacatgaccaagatgtcttggtgctggagaaggtcccagcagggaacagagcttctaatcaaggaaactcacagcctcagcaaaagtatactgtgatgtcaggaacacctgaaaaaattttagagcattttctagaaacaatacgccttgaggcaactttaaatgaagcaacagattctgttttaaatgactttattatgatgcactgtgtttttatgccaaatacccagctttgcccggcactggtggcccactaccacgcacagccttcacaaggtacagaacaggagaaaatggattatgccctcaacaataagaggcgagtcatccgcctggttctacagtgggctgccatgtatggagacctcctgcaagaggatgacgtgtctatggccttcctggaggagttttatgtatctgtatcagatgatgcccggatgattgctgccctcaaggagcaactgccagagttggagaagattgtcaagcaaatctcagaagatgcaaaggcaccacaaaagaagcacaaggttcttttgcaacagttcaatacgggcgatgagagagcccagaagcgccagcctatccgcggctctgatgaagttctgtttaaggtctattgcatggaccccacctacacaaccattcgggtgccagtggccacttcggtgaaggaagtcatcagtgcagttgccgacaagctgggctccggggagggcctgatcatagtcaagatgagttccggaggagaaaaggtggtgctcaaacctaatgatgtttcagtatttatgacgctcaccattaatggacgcctgtttgcttgcccgcgagagcaattcgattcactgactcccttaccagaacaggaaggcccaactgttggaacagtgggaacttttgaactgatgagctccaaagatttagcataccagatgacaatttatgattgggaactcttcaactgcgtgcatgagctggagctaatctatcacacatttggaaggcataattttaaaaagaccacagcaaacttggatttgttcctgaggagatttaatgaaattcagttttgggtcgtcactgagatctgcctttgttctcagctcagcaagcgtgttcagctattaaaaaaatttattaagatagcagcccactgtaaggagtataaaaatctgaattccttttttgccatcgtcatgggactaagtaacgttgctgtgagccgcttggcactaacgtgggagaaactgccaagcaagttcaagaagttctatgcggagtttgaaagtttaatggacccttcaaggaaccacagggcctacaggctgacagtagctaagctggaacctcctctcatccccttcatgcctttgctcattaaagatatgacatttactcatgaggggaacaagacgttcattgacaatctagtaaactttgaaaaaatgcgcatgattgcaaatacggccagaacagtgagatactacaggagccaacccttcaatcctgatgcagctcaagctaataagaaccatcaggatgtccggagttatgtacggcaattaaatgtgattgacaaccagagaactttatcacagatgtcacacagattagagcctcgtcgacca

SEQ ID NO: 71 - DNA, 3768 bp, Artificial Sequence
  Synthetic
atggtcgctgcgcacgctgcccattcttcctcctctgccgagtggatcgcctgcctggataaaagaccactggagcgatccagcgaagatgtggatataatcttcactcgactgaaagaagttaaagcttttgagaaatttcacccaaatctccttcatcagatttgcttatgtggttattatgagaatctggaaaagggaataacattatttcgccagggtgatattggaacaaactggtatgctgtcctggcagggtctttggatgttaaagtatctgagaccagcagtcaccaggatgctgtgaccatctgtaccctgggaattgggacggcctttggagagtccattctggacaacacaccccgccatgcaaccatcgttaccagggagagcagtgaactgctccgcatcgagcagaaggacttcaaggcactatgggagaaatatcgacagtatatggcaggacttctggctcctccttatggtgttatggaaacgggctctaacaatgacaggattcctgacaaggagaacacacctctcattgaacctcacgttcctcttcgtcctgctaacaccattaccaaggtcccttcagagaagatcctcagagctggaaaaattttacgaaatgccattctctctcgagcacctcacatgataagagatagaaaataccacctaaagacatacagacaatgctgtgtgggaactgaactggtggactggatgatgcagcagacaccatgtgttcactcccggactcaagctgttggcatgtggcaagtcctgttagaagatggtgttctcaaccacgtggaccaggagcaccatttccaagacaaatatttattctatcgatttctggatgatgagcacgaggatgcccctttgcctactgaggaggagaagaaggagtgtgatgaggagctccaggacaccatgctgctgctgtcacagatgggccccgacgcccacatgaggatgatccttcgcaaaccacctggccagaggactgtgctcgagaacgtctatatcaaggccgacaagcagaagaacggcatcaaggcgaacttcaagatccgccacaacatcgaggacggcggcgtgcagctcgcctaccactaccagcagaacacccccatcggcgacggccccgtgctgctgcccgacaaccactacctgagcgtgcagtccatactttcgaaagaccccaacgagaagcgcgatcacatggtcctgctggagttcgtgaccgccgccgggatcactctcggcatggacgagctgtacaagggcggtaccggagggagcatggtgagcaagggcgaggagctgttcaccggggtggtgcccatccaggtcgagctggacggcgacgtaaacggccacaagttcagcgtgtccggcgagggtgagggcgatgccacctacggcaagctgaccctgaagttcatctgcaccaccggcaagctgcccgtgccctggcccaccctcgtgaccaccctgacctacggcgtgcagtgcttcagccgctaccccgaccacatgaagcagcacgacttcttcaagtccgccatgcccgaaggctacatccaggagcgcaccatcttcttcaaggacgacggcaactacaagacccgcgccgaggtgaagttcgagggcgacaccctggtgaaccgcatcgagctgaagggcatcgacttcaaggaggacggcaacatcctggggcacaagctggagtacaacacgcgtgatgacctagagattatctatgaggagcttcttcatattaaagccttatcccatctttctaccacagtgaaacgagagttagcaggtgttctcatttttgagtctcacgccaaaggagggactgtgttgtttaaccagggggaagaaggtacctcctggtacattattctaaaaggatcagtgaatgtagtcatttacggcaagggtgtggtctgcaccctgcatgaaggagatgacttcggcaagttagcactagtgaatgatgccccacgagctgcctctatcgtcttacgagaagataactgccatttcttaagagtagacaaggaggatttcaaccggatcctaagggacgtggaggcgaatacagtcagacttaaagaacatgaccaagatgtcttggtgctggagaaggtcccagcagggaacagagcttctaatcaaggaaactcacagcctcagcaaaagtatactgtgatgtcaggaacacctgaaaaaattttagagcattttctagaaacaatacgccttgaggcaactttaaatgaagcaacagattctgttttaaatgactttattatgatgcactgtgtttttatgccaaatacccagctttgcccggcactggtggcccactaccacgcacagccttcacaaggtacagaacaggagaaaatggattatgccctcaacaataagaggcgagtcatccgcctggttctacagtgggctgccatgtatggagacctcctgcaagaggatgacgtgtctatggccttcctggaggagttttatgtatctgtatcagatgatgcccggatgattgctgccctcaaggagcaactgccagagttggagaagattgtcaagcaaatctcagaagatgcaaaggcaccacaaaagaagcacaaggttcttttgcaacagttcaatacgggcgatgagagagcccagaagcgccagcctatccgcggctctgatgaagttctgtttaaggtctattgcatggaccccacctacacaaccattcgggtgccagtggccacttcggtgaaggaagtcatcagtgcagttgccgacaagctgggctccggggagggcctgatcatagtcaagatgagttccggaggagaaaaggtggtgctcaaacctaatgatgtttcagtatttatgacgctcaccattaatggacgcctgtttgcttgcccgcgagagcaattcgattcactgactcccttaccagaacaggaaggcccaactgttggaacagtgggaacttttgaactgatgagctccaaagatttagcataccagatgacaatttatgattgggaactcttcaactgcgtgcatgagctggagctaatctatcacacatttggaaggcataattttaaaaagaccacagcaaacttggatttgttcctgaggagatttaatgaaattcagttttgggtcgtcactgagatctgcctttgttctcagctcagcaagcgtgttcagctattaaaaaaatttattaagatagcagcccactgtaaggagtataaaaatctgaattccttttttgccatcgtcatgggactaagtaacgttgctgtgagccgcttggcactaacgtgggagaaactgccaagcaagttcaagaagttctatgcggagtttgaaagtttaatggacccttcaaggaaccacagggcctacaggctgacagtagctaagctggaacctcctctcatccccttcatgcctttgctcattaaagatatgacatttactcatgaggggaacaagacgttcattgacaatctagtaaactttgaaaaaatgcgcatgattgcaaatacggccagaacagtgagatactacaggagccaacccttcaatcctgatgcagctcaagctaataagaaccatcaggatgtccggagttatgtacggcaattaaatgtgattgacaaccagagaactttatcacagatgtcacacagattagagcctcgtcgacca

SEQ ID NO: 72 - DNA, 3768 bp, Artificial Sequence
  Synthetic
atggtcgctgcgcacgctgcccattcttcctcctctgccgagtggatcgcctgcctggataaaagaccactggagcgatccagcgaagatgtggatataatcttcactcgactgaaagaagttaaagcttttgagaaatttcacccaaatctccttcatcagatttgcttatgtggttattatgagaatctggaaaagggaataacattatttcgccagggtgatattggaacaaactggtatgctgtcctggcagggtctttggatgttaaagtatctgagaccagcagtcaccaggatgctgtgaccatctgtaccctgggaattgggacggcctttggagagtccattctggacaacacaccccgccatgcaaccatcgttaccagggagagcagtgaactgctccgcatcgagcagaaggacttcaaggcactatgggagaaatatcgacagtatatggcaggacttctggctcctccttatggtgttatggaaacgggctctaacaatgacaggattcctgacaaggagaacacacctctcattgaacctcacgttcctcttcgtcctgctaacaccattaccaaggtcccttcagagaagatcctcagagctggaaaaattttacgaaatgccattctctctcgagcacctcacatgataagagatagaaaataccacctaaagacatacagacaatgctgtgtgggaactgaactggtggactggatgatgcagcagacaccatgtgttcactcccggactcaagctgttggcatgtggcaagtcctgttagaagatggtgttctcaaccacgtggaccaggagcaccatttccaagacaaatatttattctatcgatttctggatgatgagcacgaggatgcccctttgcctactgaggaggagaagaaggagtgtgatgaggagctccaggacaccatgctgctgctgtcacagatgggccccgacgcccacatgaggatgatccttcgcaaaccacctggccagaggactgtggatgacctagagattatctatgaggagcttcttcatattaaagccttatcccatctttctaccacagtgaaacgagagttagcaggtgttctcatttttgagtctcacgccaaaggagggactgtgttgtttaaccagggggaagaaggtacctcctggtacattattctaaaaggatcagtgaatgtagtcatttacggcaagggtgtggtctgcaccctgcatgaaggagatgacttcggcaagttagcactagtgaatgatgccccacgagctgcctctatcgtcttacgagaagataactgccatttcttaagagtagacaaggaggatttcaaccggatcctaagggacgtggaggcgaatacagtcagacttaaagaacatgaccaagatgtcttggtgctggagaaggtcccagcagggaacagagctctcgagaacgtctatatcaaggccgacaagcagaagaacggcatcaaggcgaacttcaagatccgccacaacatcgaggacggcggcgtgcagctcgcctaccactaccagcagaacacccccatcggcgacggccccgtgctgctgcccgacaaccactacctgagcgtgcagtccatactttcgaaagaccccaacgagaagcgcgatcacatggtcctgctggagttcgtgaccgccgccgggatcactctcggcatggacgagctgtacaagggcggtaccggagggagcatggtgagcaagggcgaggagctgttcaccggggtggtgcccatccaggtcgagctggacggcgacgtaaacggccacaagttcagcgtgtccggcgagggtgagggcgatgccacctacggcaagctgaccctgaagttcatctgcaccaccggcaagctgcccgtgccctggcccaccctcgtgaccaccctgacctacggcgtgcagtgcttcagccgctaccccgaccacatgaagcagcacgacttcttcaagtccgccatgcccgaaggctacatccaggagcgcaccatcttcttcaaggacgacggcaactacaagacccgcgccgaggtgaagttcgagggcgacaccctggtgaaccgcatcgagctgaagggcatcgacttcaaggaggacggcaacatcctggggcacaagctggagtacaacacgcgttctaatcaaggaaactcacagcctcagcaaaagtatactgtgatgtcaggaacacctgaaaaaattttagagcattttctagaaacaatacgccttgaggcaactttaaatgaagcaacagattctgttttaaatgactttattatgatgcactgtgtttttatgccaaatacccagctttgcccggcactggtggcccactaccacgcacagccttcacaaggtacagaacaggagaaaatggattatgccctcaacaataagaggcgagtcatccgcctggttctacagtgggctgccatgtatggagacctcctgcaagaggatgacgtgtctatggccttcctggaggagttttatgtatctgtatcagatgatgcccggatgattgctgccctcaaggagcaactgccagagttggagaagattgtcaagcaaatctcagaagatgcaaaggcaccacaaaagaagcacaaggttcttttgcaacagttcaatacgggcgatgagagagcccagaagcgccagcctatccgcggctctgatgaagttctgtttaaggtctattgcatggaccccacctacacaaccattcgggtgccagtggccacttcggtgaaggaagtcatcagtgcagttgccgacaagctgggctccggggagggcctgatcatagtcaagatgagttccggaggagaaaaggtggtgctcaaacctaatgatgtttcagtatttatgacgctcaccattaatggacgcctgtttgcttgcccgcgagagcaattcgattcactgactcccttaccagaacaggaaggcccaactgttggaacagtgggaacttttgaactgatgagctccaaagatttagcataccagatgacaatttatgattgggaactcttcaactgcgtgcatgagctggagctaatctatcacacatttggaaggcataattttaaaaagaccacagcaaacttggatttgttcctgaggagatttaatgaaattcagttttgggtcgtcactgagatctgcctttgttctcagctcagcaagcgtgttcagctattaaaaaaatttattaagatagcagcccactgtaaggagtataaaaatctgaattccttttttgccatcgtcatgggactaagtaacgttgctgtgagccgcttggcactaacgtgggagaaactgccaagcaagttcaagaagttctatgcggagtttgaaagtttaatggacccttcaaggaaccacagggcctacaggctgacagtagctaagctggaacctcctctcatccccttcatgcctttgctcattaaagatatgacatttactcatgaggggaacaagacgttcattgacaatctagtaaactttgaaaaaatgcgcatgattgcaaatacggccagaacagtgagatactacaggagccaacccttcaatcctgatgcagctcaagctaataagaaccatcaggatgtccggagttatgtacggcaattaaatgtgattgacaaccagagaactttatcacagatgtcacacagattagagcctcgtcgacca

SEQ ID NO: 73 - DNA, 3768 bp, Artificial Sequence
  Synthetic
atggtcgctgcgcacgctgcccattcttcctcctctgccgagtggatcgcctgcctggataaaagaccactggagcgatccagcgaagatgtggatataatcttcactcgactgaaagaagttaaagcttttgagaaatttcacccaaatctccttcatcagatttgcttatgtggttattatgagaatctggaaaagggaataacattatttcgccagggtgatattggaacaaactggtatgctgtcctggcagggtctttggatgttaaagtatctgagaccagcagtcaccaggatgctgtgaccatctgtaccctgggaattgggacggcctttggagagtccattctggacaacacaccccgccatgcaaccatcgttaccagggagagcagtgaactgctccgcatcgagcagaaggacttcaaggcactatgggagaaatatcgacagtatatggcaggacttctggctcctccttatggtgttatggaaacgggctctaacaatgacaggattcctgacaaggagaacacacctctcattgaacctcacgttcctcttcgtcctgctaacaccattaccaaggtcccttcagagaagatcctcagagctggaaaaattttacgaaatgccattctctctcgagcacctcacatgataagagatagaaaataccacctaaagacatacagacaatgctgtgtgggaactgaactggtggactggatgatgcagcagacaccatgtgttcactcccggactcaagctgttggcatgtggcaagtcctgttagaagatggtgttctcaaccacgtggaccaggagcaccatttccaagacaaatatttattctatcgatttctggatgatgagcacgaggatgcccctttgcctactgaggaggagaagaaggagtgtgatgaggagctccaggacaccatgctgctgctgtcacagatgggccccgacgcccacatgaggatgatccttcgcaaaccacctggccagaggactgtggatgacctagagattatctatgaggagcttcttcatattaaagccttatcccatctttctaccacagtgaaacgagagttagcaggtgttctcatttttgagtctcacgccaaaggagggactgtgttgtttaaccagggggaagaaggtacctcctggtacattattctaaaaggatcagtgaatgtagtcatttacggcaagggtgtggtctgcaccctgcatgaaggagatgacttcggcaagttagcactagtgaatgatgccccacgagctgcctctatcgtcttacgagaagataactgccatttcttaagagtagacaaggaggatttcaaccggatcctaagggacgtggaggcgaatacagtcagacttaaagaacatgaccaagatgtcttggtgctggagaaggtcccagcagggaacagagcttctaatcaaggaaactcacagcctcagcaaaagtatactgtgatgtcaggaacacctgaaaaaattttagagcattttctagaaacaatacgccttgaggcactcgagaacgtctatatcaaggccgacaagcagaagaacggcatcaaggcgaacttcaagatccgccacaacatcgaggacggcggcgtgcagctcgcctaccactaccagcagaacacccccatcggcgacggccccgtgctgctgcccgacaaccactacctgagcgtgcagtccatactttcgaaagaccccaacgagaagcgcgatcacatggtcctgctggagttcgtgaccgccgccgggatcactctcggcatggacgagctgtacaagggcggtaccggagggagcatggtgagcaagggcgaggagctgttcaccggggtggtgcccatccaggtcgagctggacggcgacgtaaacggccacaagttcagcgtgtccggcgagggtgagggcgatgccacctacggcaagctgaccctgaagttcatctgcaccaccggcaagctgcccgtgccctggcccaccctcgtgaccaccctgacctacggcgtgcagtgcttcagccgctaccccgaccacatgaagcagcacgacttcttcaagtccgccatgcccgaaggctacatccaggagcgcaccatcttcttcaaggacgacggcaactacaagacccgcgccgaggtgaagttcgagggcgacaccctggtgaaccgcatcgagctgaagggcatcgacttcaaggaggacggcaacatcctggggcacaagctggagtacaacacgcgtactttaaatgaagcaacagattctgttttaaatgactttattatgatgcactgtgtttttatgccaaatacccagctttgcccggcactggtggcccactaccacgcacagccttcacaaggtacagaacaggagaaaatggattatgccctcaacaataagaggcgagtcatccgcctggttctacagtgggctgccatgtatggagacctcctgcaagaggatgacgtgtctatggccttcctggaggagttttatgtatctgtatcagatgatgcccggatgattgctgccctcaaggagcaactgccagagttggagaagattgtcaagcaaatctcagaagatgcaaaggcaccacaaaagaagcacaaggttcttttgcaacagttcaatacgggcgatgagagagcccagaagcgccagcctatccgcggctctgatgaagttctgtttaaggtctattgcatggaccccacctacacaaccattcgggtgccagtggccacttcggtgaaggaagtcatcagtgcagttgccgacaagctgggctccggggagggcctgatcatagtcaagatgagttccggaggagaaaaggtggtgctcaaacctaatgatgtttcagtatttatgacgctcaccattaatggacgcctgtttgcttgcccgcgagagcaattcgattcactgactcccttaccagaacaggaaggcccaactgttggaacagtgggaacttttgaactgatgagctccaaagatttagcataccagatgacaatttatgattgggaactcttcaactgcgtgcatgagctggagctaatctatcacacatttggaaggcataattttaaaaagaccacagcaaacttggatttgttcctgaggagatttaatgaaattcagttttgggtcgtcactgagatctgcctttgttctcagctcagcaagcgtgttcagctattaaaaaaatttattaagatagcagcccactgtaaggagtataaaaatctgaattccttttttgccatcgtcatgggactaagtaacgttgctgtgagccgcttggcactaacgtgggagaaactgccaagcaagttcaagaagttctatgcggagtttgaaagtttaatggacccttcaaggaaccacagggcctacaggctgacagtagctaagctggaacctcctctcatccccttcatgcctttgctcattaaagatatgacatttactcatgaggggaacaagacgttcattgacaatctagtaaactttgaaaaaatgcgcatgattgcaaatacggccagaacagtgagatactacaggagccaacccttcaatcctgatgcagctcaagctaataagaaccatcaggatgtccggagttatgtacggcaattaaatgtgattgacaaccagagaactttatcacagatgtcacacagattagagcctcgtcgacca

SEQ ID NO: 74 - protein, 881 aa, Homo sapiens
MVLRRMHRPRSCSYQLLLEHQRPSCIQGLRWTPLTNSEESLDFSESLEQASTERVLRAGRQLHRHLLATCPNLIRDRKYHLRLYRQCCSGRELVDGILALGLGVHSRSQVVGICQVLLDEGALCHVKHDWAFQDRDAQFYRFPGPEPEPVGTHEMEEELAEAVALLSQRGPDALLTVALRKPPGQRTDEELDLIFEELLHIKAVAHLSNSVKRELAAVLLFEPHSKAGTVLFSQGDKGTSWYIIWKGSVNVVTHGKGLVTTLHEGDDFGQLALVNDAPRAATIILREDNCHFLRVDKQDFNRIIKDVEAKTMRLEEHGKVVLVLERASQGAGPSRPPTPGRNRYTVMSGTPEKILELLLEAMGPDSSAHDPTETFLSDFLLTHRVFMPSAQLCAALLHHFHVEPAGGSEQERSTYVCNKRQQILRLVSQWVALYGSMLHTDPVATSFLQKLSDLVGRDTRLSNLLREQWPERRRCHRLENGCGNASPQMKARNLPVWLPNQDEPLPGSSCAIQVGDKVPYDICRPDHSVLTLQLPVTASVREVMAALAQEDGWTKGQVLVKVNSAGDAIGLQPDARGVATSLGLNERLFVVNPQEVHELIPHPDQLGPTVGSAEGLDLVSAKDLAGQLTDHDWSLFNSIHQVELIHYVLGPQHLRDVTTANLERFMRRFNELQYWVATELCLCPVPGPRAQLLRKFIKLAAHLKEQKNLNSFFAVMFGLSNSAISRLAHTWERLPHKVRKLYSALERLLDPSWNHRVYRLALAKLSPPVIPFMPLLLKDMTFIHEGNHTLVENLINFEKMRMMARAARMLHHCRSHNPVPLSPLRSRVSHLHEDSQVARISTCSEQSLSTRSPASTWAYVQQLKVIDNQRELSRLSRELEP

SEQ ID NO: 75 - protein, 381 aa, Homo sapiens
MESGSTAASEEARSLRECELYVQKHNIQALLKDSIVQLCTARPERPMAFLREYFERLEKEEAKQIQNLQKAGTRTDSREDEISPPPPNPVVKGRRRRGAISAEVYTEEDAASYVRKVIPKDYKTMAALAKAIEKNVLFSHLDDNERSDIFDAMFSVSFIAGETVIQQGDEGDNFYVIDQGETDVYVNNEWATSVGEGGSFGELALIYGTPRAATVKAKTNVKLWGIDRDSYRRILMGSTLRKRKMYEEFLSKVSILESLDKWERLTVADALEPVQFEDGQKIVVQGEPGDEFFIILEGSAAVLQRRSENEEFVEVGRLGPSDYFGEIALLMNRPRAATVVARGPLKCVKLDRPRFERVLGPCSDILKRNIQQYNSFVSLSV

SEQ ID NO: 76 - protein, 184 aa, Homo sapiens [sequence omitted]

SEQ ID NO: 77 - protein, 239 aa, Artificial Sequence
  Synthetic
MVSKGEELFTGVVPILVELDGDVNGHKFSVSGEGEGDATYGKLTLKFICTTGKLPVPWPTLVTTLTYGVQCFSRYPDHMKQHDFFKSAMPEGYVQERTIFFKDDGNYKTRAEVKFEGDTLVNRIELKGIDFKEDGNILGHKLEYNYNSHNVYIMADKQKNGIKVNFKIRHNIEDGSVQLADHYQQNTPIGDGPVLLPDNHYLSTQSALSKDPNEKRDHMVLLEFVTAAGITLGMDELYK